European Patent Application EP 4 700 042 A1, published February 25, 2026. Title: A microorganism for producing purine nucleotides and method for producing purine nucleotides using the same. Applicant: CJ CheilJedang Corporation. The sequence listing filed with the application follows.

SEQUENCE LISTING (260 sequences)

SEQ ID NO: 1 - protein, 413 aa, Corynebacterium glutamicum
  source 1..413: note = Corynebacterium stationis MFS transporter AA
MHTTEEVKLFTPTFIMGWVANFLQFLVFYFLITTMALYATKEFSASETEAGFAASAIVIGAVFSRLVSGYIIDRFGRRKIVVVSVIATTIACALYIPIDSLGLLYADRFFHGVAYAFACTAIMAMVQELIPSARRSEGTGYLALGTTVSAAIGPALALFLLGSFNYEVLFVVVLGISIVSLIASLVIYFRTSDPEPELDENGNAAEPIKFSFKSIINPKVLPIGLFMLLVAFAYSGVIAHINAFAENRDVVTGAGLFFIAYAISMFVMRSYLGKLQDRRGDNSVIYFGLVFFVISFIVLSLSTANWHVVVAGVLAGLGYGTLMPAAQAVSVGVVDKSEFGSAFSTLFLFVDLGFGFGPVILGAVVSAIGYGSMYAVLVGVGVIAGIYYLFTHARTERAKHGVVKHVETMVLAQ

SEQ ID NO: 2 - DNA, 1242 bp, Corynebacterium glutamicum
  source 1..1242: mol_type = genomic DNA; note = Corynebacterium stationis MFS transporter NT
gtgcacacaaccgaagaggtcaaactctttacgccgacgtttatcatggggtgggtcgccaacttcctgcagttcttggtgttctacttcctcatcaccacgatggcgctctacgcaaccaaggaattcagcgcatcggaaaccgaagcaggctttgccgccagtgcgattgttatcggtgcggtcttttcccgtttggtttccggatacattattgaccgcttcggtcgccgcaaaattgtggtggtctccgtcatcgcgaccactattgcgtgcgcgctatatatcccgatcgattctttggggctgctctacgctgaccgcttcttccacggtgtagcttatgcctttgcgtgcaccgcgattatggcgatggtccaggaactcattccttctgcacgccgctccgaaggcactggctacctggctttgggtaccaccgtttcggctgctatcggaccagcgctagcgctatttttgctgggttctttcaactacgaagtcctcttcgttgtcgtcctcggcatttcgattgtctctttgatcgcttcgctagtcatctatttccgcacctccgacccagagccagagctggatgaaaacggcaatgctgctgagcccattaagttcagcttcaagtccatcattaaccctaaagtcttgccgattggcctcttcatgctgctggtagcctttgcctactccggcgtgatcgcacatatcaacgcttttgctgaaaaccgcgacgttgttactggcgcaggcctattctttatcgcttacgccatctccatgttcgtgatgcgctcctaccttggtaaattgcaagaccgccggggcgataacagcgttatctactttggtctcgtattctttgttatctcatttatcgtgctctcgctttctaccgccaactggcatgtcgttgtcgctggcgtgctagcaggtctgggctacggcaccttgatgccagctgctcaagcagtatctgttggtgttgtcgacaagagcgagttcggctcagcattttccaccttgttccttttcgttgacctcggcttcggcttcggcccagtcatccttggtgcagtggtttccgcgattggctacggttcgatgtatgcagtgctcgtcggcgtcggcgttattgctggcatctactacctgttcacccacgcacgcaccgagcgcgcaaagcacggcgtagtcaagcatgtagaaaccatggttctggctcaataa

SEQ ID NO: 3 - protein, 406 aa, Corynebacterium glutamicum
  source 1..406: note = Corynebacterium glutamicum ATCC13032 MFS transporter AA
MSVAEEGKLFTPTFVMGWFANLFQFLVFYFLITTMALYAIKEFQASEVEAGFASSSIVIGAVFSRFFSGYIIDRFGRRKIVLISVLVTTIACALYLPIESLPLLYANRFLHGVGYAFAATAIMAMVQELIPASRRSEGTGYLALGTTVSAALGPALALFVLGTFDYDMLFIVVLATSVISLIAVVFMYFKTSDPEPSGEPAKFSFKSIMNPKIIPIGIFILLICFAYSGVIAYINAFAEERDLITGAGLFFIAYAVSMFVMRSFLGKLQDRRGDNVVIYFGLFFFVISLTILSFATSNWHVVLSGVIAGLGYGTLMPAVQSIAVGVVDKTEFGTAFSTLFLFVDLGFGFGPIILGAVSAAIGFGPMYAALAGVGVIAGIFYLFTHARTDRAKNGFVKHPEPVALVS

SEQ ID NO: 4 - DNA, 1221 bp, Corynebacterium glutamicum
  source 1..1221: mol_type = genomic DNA; note = Corynebacterium glutamicum ATCC13032 MFS transporter NT
atgtccgtagctgaagaagggaaactttttacaccaacgtttgtcatgggatggtttgccaaccttttccagttcctggtgttctacttcctcatcaccaccatggctttgtacgccatcaaggaatttcaagcctctgaagtagaagctggcttcgcatccagctcaattgttatcggcgcagtcttttccaggtttttctccggctatattattgaccgttttggtcgacgcaagattgtgctcatctcagtcctagtcactaccattgcgtgtgccttgtaccttcccatcgaatcattgccattgctatacgcaaacaggttcctccacggtgttggatacgcttttgctgccaccgcgatcatggcaatggtccaggagctcattccagcgtcacgacgttccgaaggtactggttacctggcattgggcactaccgtttctgcagcacttggaccagccctagcactttttgtcctaggaacatttgattacgacatgctgtttatcgtggtcttggcaacctcggtcatctctttgatcgccgtcgtgttcatgtactttaagaccagcgaccctgagccttctggggaaccagccaagttcagcttcaaatctattatgaacccaaagatcatccccatcggcatctttatcttgcttatttgctttgcttactctggcgtcattgcctacatcaacgcatttgctgaagaacgcgatctgattacgggtgctggattgttcttcattgcctacgcagtatcaatgtttgtgatgcgcagcttccttggcaaactgcaggaccgtcgcggagacaacgtcgttatttactttggattgttcttcttcgttatttccttgacgattttgtcctttgccacttccaactggcacgttgtgttgtccggagtcattgcaggtctgggatacggcactttgatgccagcagtgcagtccatcgctgttggtgtagtagacaaaaccgaattcggtacggccttctccactttgttcctgtttgtggacttaggttttggctttggacctattatcctgggagcagtttctgcggcaattggtttcggacctatgtatgcagcactggcaggtgtgggtgtgattgccggaatcttctacctgttcacacacgctcgcaccgatcgagctaagaatggctttgttaaacacccagagcctgtcgctttagttagctag

SEQ ID NO: 5 - protein, 391 aa, Corynebacterium glutamicum
  source 1..391: note = Corynebacterium glutamicum ATCC13869 MFS transporter AA
MGWFANLFQFLVFYFLITTMALYAIKEFQASEVEAGFASSSIVIGAVFSRFFSGYIIDRFGRRKIVLISVLVTTIACALYLPIESLPLLYANRFLHGVGYAFAATAIMAMVQELIPASRRSEGTGYLALGTTVSAALGPALALFVLGTFDYDMLFIVVLATSIISLIAVVFMYFKTSDPEPSGEPAKFSFKSIMNPKIIPIGIFILLICFAYSGVIAYINAFAEERDLITGAGLFFIAYAVSMFVMRSFLGKLQDRRGDNVVIYFGLFFFVISLVILSFATSNWHVVLSGVIAGLGYGTLMPAVQSIAVGVVDKTEFGTAFSTLFLFVDLGFGFGPIILGAVSAAIGFGPMYAALAGVGVIAGIFYLFTHARTDRAKNGFVKHPEPVALVS

SEQ ID NO: 6 - DNA, 1176 bp, Corynebacterium glutamicum
  source 1..1176: mol_type = genomic DNA; note = Corynebacterium glutamicum ATCC13869 MFS transporter NT
atgggatggtttgccaacctgttccaattcttggtgttctacttcctcatcaccaccatggctttgtatgccatcaaggaatttcaggcctctgaagtagaagcaggatttgcatccagctcaattgttatcggcgcagtcttttccaggtttttctccggctatattattgaccgttttggtcgacgcaagattgtgctcatctcagtcctcgtcactaccattgcgtgtgccttgtaccttcccatcgaatcattgccattgctatacgcaaacaggttcctccacggtgttggatacgcttttgctgccaccgcgatcatggcaatggtccaggagctcattccagcgtcacgacgttccgaaggtactggttacctggcattgggcaccaccgtttctgcagcacttggaccagccctagcactttttgtcctaggaacatttgattacgacatgctgtttatcgtggtcttggcaacctccatcatctctttgattgccgtcgtattcatgtactttaagaccagcgaccctgagccttctggggaaccagccaagttcagcttcaaatctattatgaacccaaagatcatccccatcggcatctttatcttgcttatttgctttgcttactctggcgtcattgcctacatcaacgcatttgctgaagaacgcgatctgattacgggtgctggattgttcttcattgcctacgcagtatcaatgtttgtgatgcgcagcttccttggcaaactgcaggaccgtcgcggagacaacgtcgttatttactttggattgttcttcttcgttatttccttggtgattttgtcctttgccacttccaactggcacgttgtgttgtccggggtcattgcaggtctgggatacggcactttgatgccagcagtgcagtccatcgctgttggtgtagtagacaaaaccgaattcggtacggccttctccactttgttcctgtttgtggacttaggttttggctttggacctattatcctgggagcggtttctgcggcaattggtttcggacctatgtatgcagcactggcaggtgtgggtgtgattgccggaatcttctacctgttcacacacgctcgcaccgatcgagctaagaatggctttgttaaacacccagagcctgtcgctttagttagctag

SEQ ID NO: 7 - protein, 413 aa, synthetic construct
  source 1..413: note = C. st L185Q AA
MHTTEEVKLFTPTFIMGWVANFLQFLVFYFLITTMALYATKEFSASETEAGFAASAIVIGAVFSRLVSGYIIDRFGRRKIVVVSVIATTIACALYIPIDSLGLLYADRFFHGVAYAFACTAIMAMVQELIPSARRSEGTGYLALGTTVSAAIGPALALFLLGSFNYEVLFVVVLGISIVSLIASQVIYFRTSDPEPELDENGNAAEPIKFSFKSIINPKVLPIGLFMLLVAFAYSGVIAHINAFAENRDVVTGAGLFFIAYAISMFVMRSYLGKLQDRRGDNSVIYFGLVFFVISFIVLSLSTANWHVVVAGVLAGLGYGTLMPAAQAVSVGVVDKSEFGSAFSTLFLFVDLGSGFGPVILGAVVSAIGYGSMYAVLVGVGVIAGIYYLFTHARTERAKHGVVKHVETMVLAQ

SEQ ID NO: 8 - DNA, 1242 bp, synthetic construct
  source 1..1242: mol_type = other DNA; note = C. st L185Q NT
gtgcacacaaccgaagaggtcaaactctttacgccgacgtttatcatggggtgggtcgccaacttcctgcagttcttggtgttctacttcctcatcaccacgatggcgctctacgcaaccaaggaattcagcgcatcggaaaccgaagcaggctttgccgccagtgcgattgttatcggtgcggtcttttcccgtttggtttccggatacattattgaccgcttcggtcgccgcaaaattgtggtggtctccgtcatcgcgaccactattgcgtgcgcgctatatatcccgatcgattctttggggctgctctacgctgaccgcttcttccacggtgtagcttatgcctttgcgtgcaccgcgattatggcgatggtccaggaactcattccttctgcacgccgctccgaaggcactggctacctggctttgggtaccaccgtttcggctgctatcggaccagcgctagcgctatttttgctgggttctttcaactacgaagtcctcttcgttgtcgtcctcggcatttcgattgtctctttgatcgcttcgcaggtcatctatttccgcacctccgacccagagccagagctggatgaaaacggcaatgctgctgagcccattaagttcagcttcaagtccatcattaaccctaaagtcttgccgattggcctcttcatgctgctggtagcctttgcctactccggcgtgatcgcacatatcaacgcttttgctgaaaaccgcgacgttgttactggcgcaggcctattctttatcgcttacgccatctccatgttcgtgatgcgctcctaccttggtaaattgcaagaccgccggggcgataacagcgttatctactttggtctcgtattctttgttatctcatttatcgtgctctcgctttctaccgccaactggcatgtcgttgtcgctggcgtgctagcaggtctgggctacggcaccttgatgccagctgctcaagcagtatctgttggtgttgtcgacaagagcgagttcggctcagcattttccaccttgttccttttcgttgacctcggcttcggcttcggcccagtcatccttggtgcagtggtttccgcgattggctacggttcgatgtatgcagtgctcgtcggcgtcggcgttattgctggcatctactacctgttcacccacgcacgcaccgagcgcgcaaagcacggcgtagtcaagcatgtagaaaccatggttctggctcaataa

SEQ ID NO: 9 - protein, 413 aa, synthetic construct
  source 1..413: note = C. st V378A AA
MHTTEEVKLFTPTFIMGWVANFLQFLVFYFLITTMALYATKEFSASETEAGFAASAIVIGAVFSRLVSGYIIDRFGRRKIVVVSVIATTIACALYIPIDSLGLLYADRFFHGVAYAFACTAIMAMVQELIPSARRSEGTGYLALGTTVSAAIGPALALFLLGSFNYEVLFVVVLGISIVSLIASLVIYFRTSDPEPELDENGNAAEPIKFSFKSIINPKVLPIGLFMLLVAFAYSGVIAHINAFAENRDVVTGAGLFFIAYAISMFVMRSYLGKLQDRRGDNSVIYFGLVFFVISFIVLSLSTANWHVVVAGVLAGLGYGTLMPAAQAVSVGVVDKSEFGSAFSTLFLFVDLGFGFGPVILGAVVSAIGYGSMYAVLAGVGVIAGIYYLFTHARTERAKHGVVKHVETMVLAQ

SEQ ID NO: 10 - DNA, 1242 bp, synthetic construct
  source 1..1242: mol_type = other DNA; note = C. st V378A NT
gtgcacacaaccgaagaggtcaaactctttacgccgacgtttatcatggggtgggtcgccaacttcctgcagttcttggtgttctacttcctcatcaccacgatggcgctctacgcaaccaaggaattcagcgcatcggaaaccgaagcaggctttgccgccagtgcgattgttatcggtgcggtcttttcccgtttggtttccggatacattattgaccgcttcggtcgccgcaaaattgtggtggtctccgtcatcgcgaccactattgcgtgcgcgctatatatcccgatcgattctttggggctgctctacgctgaccgcttcttccacggtgtagcttatgcctttgcgtgcaccgcgattatggcgatggtccaggaactcattccttctgcacgccgctccgaaggcactggctacctggctttgggtaccaccgtttcggctgctatcggaccagcgctagcgctatttttgctgggttctttcaactacgaagtcctcttcgttgtcgtcctcggcatttcgattgtctctttgatcgcttcgctagtcatctatttccgcacctccgacccagagccagagctggatgaaaacggcaatgctgctgagcccattaagttcagcttcaagtccatcattaaccctaaagtcttgccgattggcctcttcatgctgctggtagcctttgcctactccggcgtgatcgcacatatcaacgcttttgctgaaaaccgcgacgttgttactggcgcaggcctattctttatcgcttacgccatctccatgttcgtgatgcgctcctaccttggtaaattgcaagaccgccggggcgataacagcgttatctactttggtctcgtattctttgttatctcatttatcgtgctctcgctttctaccgccaactggcatgtcgttgtcgctggcgtgctagcaggtctgggctacggcaccttgatgccagctgctcaagcagtatctgttggtgttgtcgacaagagcgagttcggctcagcattttccaccttgttccttttcgttgacctcggcttcggcttcggcccagtcatccttggtgcagtggtttccgcgattggctacggttcgatgtatgcagtgctcgcaggcgtcggcgttattgctggcatctactacctgttcacccacgcacgcaccgagcgcgcaaagcacggcgtagtcaagcatgtagaaaccatggttctggctcaataa

SEQ ID NO: 11 - protein, 413 aa, synthetic construct
  source 1..413: note = C. st I383L AA
MHTTEEVKLFTPTFIMGWVANFLQFLVFYFLITTMALYATKEFSASETEAGFAASAIVIGAVFSRLVSGYIIDRFGRRKIVVVSVIATTIACALYIPIDSLGLLYADRFFHGVAYAFACTAIMAMVQELIPSARRSEGTGYLALGTTVSAAIGPALALFLLGSFNYEVLFVVVLGISIVSLIASLVIYFRTSDPEPELDENGNAAEPIKFSFKSIINPKVLPIGLFMLLVAFAYSGVIAHINAFAENRDVVTGAGLFFIAYAISMFVMRSYLGKLQDRRGDNSVIYFGLVFFVISFIVLSLSTANWHVVVAGVLAGLGYGTLMPAAQAVSVGVVDKSEFGSAFSTLFLFVDLGFGFGPVILGAVVSAIGYGSMYAVLAGVGVLAGIYYLFTHARTERAKHGVVKHVETMVLAQ

SEQ ID NO: 12 - DNA, 1242 bp, synthetic construct
  source 1..1242: mol_type = other DNA; note = C. st I383L NT
gtgcacacaaccgaagaggtcaaactctttacgccgacgtttatcatggggtgggtcgccaacttcctgcagttcttggtgttctacttcctcatcaccacgatggcgctctacgcaaccaaggaattcagcgcatcggaaaccgaagcaggctttgccgccagtgcgattgttatcggtgcggtcttttcccgtttggtttccggatacattattgaccgcttcggtcgccgcaaaattgtggtggtctccgtcatcgcgaccactattgcgtgcgcgctatatatcccgatcgattctttggggctgctctacgctgaccgcttcttccacggtgtagcttatgcctttgcgtgcaccgcgattatggcgatggtccaggaactcattccttctgcacgccgctccgaaggcactggctacctggctttgggtaccaccgtttcggctgctatcggaccagcgctagcgctatttttgctgggttctttcaactacgaagtcctcttcgttgtcgtcctcggcatttcgattgtctctttgatcgcttcgctagtcatctatttccgcacctccgacccagagccagagctggatgaaaacggcaatgctgctgagcccattaagttcagcttcaagtccatcattaaccctaaagtcttgccgattggcctcttcatgctgctggtagcctttgcctactccggcgtgatcgcacatatcaacgcttttgctgaaaaccgcgacgttgttactggcgcaggcctattctttatcgcttacgccatctccatgttcgtgatgcgctcctaccttggtaaattgcaagaccgccggggcgataacagcgttatctactttggtctcgtattctttgttatctcatttatcgtgctctcgctttctaccgccaactggcatgtcgttgtcgctggcgtgctagcaggtctgggctacggcaccttgatgccagctgctcaagcagtatctgttggtgttgtcgacaagagcgagttcggctcagcattttccaccttgttccttttcgttgacctcggcttcggcttcggcccagtcatccttggtgcagtggtttccgcgattggctacggttcgatgtatgcagtgctcgtcggcgtcggcgttctggctggcatctactacctgttcacccacgcacgcaccgagcgcgcaaagcacggcgtagtcaagcatgtagaaaccatggttctggctcaataa

SEQ ID NO: 13 - protein, 413 aa, synthetic construct
  source 1..413: note = C. st V403A AA
MHTTEEVKLFTPTFIMGWVANFLQFLVFYFLITTMALYATKEFSASETEAGFAASAIVIGAVFSRLVSGYIIDRFGRRKIVVVSVIATTIACALYIPIDSLGLLYADRFFHGVAYAFACTAIMAMVQELIPSARRSEGTGYLALGTTVSAAIGPALALFLLGSFNYEVLFVVVLGISIVSLIASLVIYFRTSDPEPELDENGNAAEPIKFSFKSIINPKVLPIGLFMLLVAFAYSGVIAHINAFAENRDVVTGAGLFFIAYAISMFVMRSYLGKLQDRRGDNSVIYFGLVFFVISFIVLSLSTANWHVVVAGVLAGLGYGTLMPAAQAVSVGVVDKSEFGSAFSTLFLFVDLGFGFGPVILGAVVSAIGYGSMYAVLVGVGVIAGIYYLFTHARTERAKHGVAKHVETMVLAQ

SEQ ID NO: 14 - DNA, 1242 bp, synthetic construct
  source 1..1242: mol_type = other DNA; note = C. st V403A NT
gtgcacacaaccgaagaggtcaaactctttacgccgacgtttatcatggggtgggtcgccaacttcctgcagttcttggtgttctacttcctcatcaccacgatggcgctctacgcaaccaaggaattcagcgcatcggaaaccgaagcaggctttgccgccagtgcgattgttatcggtgcggtcttttcccgtttggtttccggatacattattgaccgcttcggtcgccgcaaaattgtggtggtctccgtcatcgcgaccactattgcgtgcgcgctatatatcccgatcgattctttggggctgctctacgctgaccgcttcttccacggtgtagcttatgcctttgcgtgcaccgcgattatggcgatggtccaggaactcattccttctgcacgccgctccgaaggcactggctacctggctttgggtaccaccgtttcggctgctatcggaccagcgctagcgctatttttgctgggttctttcaactacgaagtcctcttcgttgtcgtcctcggcatttcgattgtctctttgatcgcttcgctagtcatctatttccgcacctccgacccagagccagagctggatgaaaacggcaatgctgctgagcccattaagttcagcttcaagtccatcattaaccctaaagtcttgccgattggcctcttcatgctgctggtagcctttgcctactccggcgtgatcgcacatatcaacgcttttgctgaaaaccgcgacgttgttactggcgcaggcctattctttatcgcttacgccatctccatgttcgtgatgcgctcctaccttggtaaattgcaagaccgccggggcgataacagcgttatctactttggtctcgtattctttgttatctcatttatcgtgctctcgctttctaccgccaactggcatgtcgttgtcgctggcgtgctagcaggtctgggctacggcaccttgatgccagctgctcaagcagtatctgttggtgttgtcgacaagagcgagttcggctcagcattttccaccttgttccttttcgttgacctcggcttcggcttcggcccagtcatccttggtgcagtggtttccgcgattggctacggttcgatgtatgcagtgctcgtcggcgtcggcgttattgctggcatctactacctgttcacccacgcacgcaccgagcgcgcaaagcacggcgtagcaaagcatgtagaaaccatggttctggctcaataa

SEQ ID NO: 15 - protein, 413 aa, synthetic construct
  source 1..413: note = C. st S283G AA
MHTTEEVKLFTPTFIMGWVANFLQFLVFYFLITTMALYATKEFSASETEAGFAASAIVIGAVFSRLVSGYIIDRFGRRKIVVVSVIATTIACALYIPIDSLGLLYADRFFHGVAYAFACTAIMAMVQELIPSARRSEGTGYLALGTTVSAAIGPALALFLLGSFNYEVLFVVVLGISIVSLIASLVIYFRTSDPEPELDENGNAAEPIKFSFKSIINPKVLPIGLFMLLVAFAYSGVIAHINAFAENRDVVTGAGLFFIAYAISMFVMRSYLGKLQDRRGDNGVIYFGLVFFVISFIVLSLSTANWHVVVAGVLAGLGYGTLMPAAQAVSVGVVDKSEFGSAFSTLFLFVDLGFGFGPVILGAVVSAIGYGSMYAVLVGVGVIAGIYYLFTHARTERAKHGVVKHVETMVLAQ

SEQ ID NO: 16 - DNA, 1242 bp, synthetic construct
  source 1..1242: mol_type = other DNA; note = C. st S283G NT
gtgcacacaaccgaagaggtcaaactctttacgccgacgtttatcatggggtgggtcgccaacttcctgcagttcttggtgttctacttcctcatcaccacgatggcgctctacgcaaccaaggaattcagcgcatcggaaaccgaagcaggctttgccgccagtgcgattgttatcggtgcggtcttttcccgtttggtttccggatacattattgaccgcttcggtcgccgcaaaattgtggtggtctccgtcatcgcgaccactattgcgtgcgcgctatatatcccgatcgattctttggggctgctctacgctgaccgcttcttccacggtgtagcttatgcctttgcgtgcaccgcgattatggcgatggtccaggaactcattccttctgcacgccgctccgaaggcactggctacctggctttgggtaccaccgtttcggctgctatcggaccagcgctagcgctatttttgctgggttctttcaactacgaagtcctcttcgttgtcgtcctcggcatttcgattgtctctttgatcgcttcgctagtcatctatttccgcacctccgacccagagccagagctggatgaaaacggcaatgctgctgagcccattaagttcagcttcaagtccatcattaaccctaaagtcttgccgattggcctcttcatgctgctggtagcctttgcctactccggcgtgatcgcacatatcaacgcttttgctgaaaaccgcgacgttgttactggcgcaggcctattctttatcgcttacgccatctccatgttcgtgatgcgctcctaccttggtaaattgcaagaccgccggggcgataacggcgttatctactttggtctcgtattctttgttatctcatttatcgtgctctcgctttctaccgccaactggcatgtcgttgtcgctggcgtgctagcaggtctgggctacggcaccttgatgccagctgctcaagcagtatctgttggtgttgtcgacaagagcgagttcggctcagcattttccaccttgttccttttcgttgacctcggcttcggcttcggcccagtcatccttggtgcagtggtttccgcgattggctacggttcgatgtatgcagtgctcgtcggcgtcggcgttattgctggcatctactacctgttcacccacgcacgcaccgagcgcgcaaagcacggcgtagtcaagcatgtagaaaccatggttctggctcaataa

SEQ ID NO: 17 - protein, 413 aa, synthetic construct
  source 1..413: note = C. st F354S AA
MHTTEEVKLFTPTFIMGWVANFLQFLVFYFLITTMALYATKEFSASETEAGFAASAIVIGAVFSRLVSGYIIDRFGRRKIVVVSVIATTIACALYIPIDSLGLLYADRFFHGVAYAFACTAIMAMVQELIPSARRSEGTGYLALGTTVSAAIGPALALFLLGSFNYEVLFVVVLGISIVSLIASLVIYFRTSDPEPELDENGNAAEPIKFSFKSIINPKVLPIGLFMLLVAFAYSGVIAHINAFAENRDVVTGAGLFFIAYAISMFVMRSYLGKLQDRRGDNSVIYFGLVFFVISFIVLSLSTANWHVVVAGVLAGLGYGTLMPAAQAVSVGVVDKSEFGSAFSTLFLFVDLGSGFGPVILGAVVSAIGYGSMYAVLVGVGVIAGIYYLFTHARTERAKHGVVKHVETMVLAQ

SEQ ID NO: 18 - DNA, 1242 bp, synthetic construct
  source 1..1242: mol_type = other DNA; note = C. st F354S NT
gtgcacacaaccgaagaggtcaaactctttacgccgacgtttatcatggggtgggtcgccaacttcctgcagttcttggtgttctacttcctcatcaccacgatggcgctctacgcaaccaaggaattcagcgcatcggaaaccgaagcaggctttgccgccagtgcgattgttatcggtgcggtcttttcccgtttggtttccggatacattattgaccgcttcggtcgccgcaaaattgtggtggtctccgtcatcgcgaccactattgcgtgcgcgctatatatcccgatcgattctttggggctgctctacgctgaccgcttcttccacggtgtagcttatgcctttgcgtgcaccgcgattatggcgatggtccaggaactcattccttctgcacgccgctccgaaggcactggctacctggctttgggtaccaccgtttcggctgctatcggaccagcgctagcgctatttttgctgggttctttcaactacgaagtcctcttcgttgtcgtcctcggcatttcgattgtctctttgatcgcttcgctagtcatctatttccgcacctccgacccagagccagagctggatgaaaacggcaatgctgctgagcccattaagttcagcttcaagtccatcattaaccctaaagtcttgccgattggcctcttcatgctgctggtagcctttgcctactccggcgtgatcgcacatatcaacgcttttgctgaaaaccgcgacgttgttactggcgcaggcctattctttatcgcttacgccatctccatgttcgtgatgcgctcctaccttggtaaattgcaagaccgccggggcgataacagcgttatctactttggtctcgtattctttgttatctcatttatcgtgctctcgctttctaccgccaactggcatgtcgttgtcgctggcgtgctagcaggtctgggctacggcaccttgatgccagctgctcaagcagtatctgttggtgttgtcgacaagagcgagttcggctcagcattttccaccttgttccttttcgttgacctcggctccggcttcggcccagtcatccttggtgcagtggtttccgcgattggctacggttcgatgtatgcagtgctcgtcggcgtcggcgttattgctggcatctactacctgttcacccacgcacgcaccgagcgcgcaaagcacggcgtagtcaagcatgtagaaaccatggttctggctcaataa

SEQ ID NO: 19 - protein, 413 aa, synthetic construct
  source 1..413: note = C. st F354Y AA
MHTTEEVKLFTPTFIMGWVANFLQFLVFYFLITTMALYATKEFSASETEAGFAASAIVIGAVFSRLVSGYIIDRFGRRKIVVVSVIATTIACALYIPIDSLGLLYADRFFHGVAYAFACTAIMAMVQELIPSARRSEGTGYLALGTTVSAAIGPALALFLLGSFNYEVLFVVVLGISIVSLIASLVIYFRTSDPEPELDENGNAAEPIKFSFKSIINPKVLPIGLFMLLVAFAYSGVIAHINAFAENRDVVTGAGLFFIAYAISMFVMRSYLGKLQDRRGDNSVIYFGLVFFVISFIVLSLSTANWHVVVAGVLAGLGYGTLMPAAQAVSVGVVDKSEFGSAFSTLFLFVDLGYGFGPVILGAVVSAIGYGSMYAVLVGVGVIAGIYYLFTHARTERAKHGVVKHVETMVLAQ

SEQ ID NO: 20 - DNA, 1242 bp, synthetic construct
  source 1..1242: mol_type = other DNA; note = C. st F354Y NT
gtgcacacaaccgaagaggtcaaactctttacgccgacgtttatcatggggtgggtcgccaacttcctgcagttcttggtgttctacttcctcatcaccacgatggcgctctacgcaaccaaggaattcagcgcatcggaaaccgaagcaggctttgccgccagtgcgattgttatcggtgcggtcttttcccgtttggtttccggatacattattgaccgcttcggtcgccgcaaaattgtggtggtctccgtcatcgcgaccactattgcgtgcgcgctatatatcccgatcgattctttggggctgctctacgctgaccgcttcttccacggtgtagcttatgcctttgcgtgcaccgcgattatggcgatggtccaggaactcattccttctgcacgccgctccgaaggcactggctacctggctttgggtaccaccgtttcggctgctatcggaccagcgctagcgctatttttgctgggttctttcaactacgaagtcctcttcgttgtcgtcctcggcatttcgattgtctctttgatcgcttcgctagtcatctatttccgcacctccgacccagagccagagctggatgaaaacggcaatgctgctgagcccattaagttcagcttcaagtccatcattaaccctaaagtcttgccgattggcctcttcatgctgctggtagcctttgcctactccggcgtgatcgcacatatcaacgcttttgctgaaaaccgcgacgttgttactggcgcaggcctattctttatcgcttacgccatctccatgttcgtgatgcgctcctaccttggtaaattgcaagaccgccggggcgataacagcgttatctactttggtctcgtattctttgttatctcatttatcgtgctctcgctttctaccgccaactggcatgtcgttgtcgctggcgtgctagcaggtctgggctacggcaccttgatgccagctgctcaagcagtatctgttggtgttgtcgacaagagcgagttcggctcagcattttccaccttgttccttttcgttgacctcggctacggcttcggcccagtcatccttggtgcagtggtttccgcgattggctacggttcgatgtatgcagtgctcgtcggcgtcggcgttattgctggcatctactacctgttcacccacgcacgcaccgagcgcgcaaagcacggcgtagtcaagcatgtagaaaccatggttctggctcaataa

SEQ ID NO: 21 - protein, 413 aa, synthetic construct
  source 1..413: note = C. st F354N AA
MHTTEEVKLFTPTFIMGWVANFLQFLVFYFLITTMALYATKEFSASETEAGFAASAIVIGAVFSRLVSGYIIDRFGRRKIVVVSVIATTIACALYIPIDSLGLLYADRFFHGVAYAFACTAIMAMVQELIPSARRSEGTGYLALGTTVSAAIGPALALFLLGSFNYEVLFVVVLGISIVSLIASLVIYFRTSDPEPELDENGNAAEPIKFSFKSIINPKVLPIGLFMLLVAFAYSGVIAHINAFAENRDVVTGAGLFFIAYAISMFVMRSYLGKLQDRRGDNSVIYFGLVFFVISFIVLSLSTANWHVVVAGVLAGLGYGTLMPAAQAVSVGVVDKSEFGSAFSTLFLFVDLGNGFGPVILGAVVSAIGYGSMYAVLVGVGVIAGIYYLFTHARTERAKHGVVKHVETMVLAQ

SEQ ID NO: 22 - DNA, 1242 bp, synthetic construct
  source 1..1242: mol_type = other DNA; note = C. st F354N NT
gtgcacacaaccgaagaggtcaaactctttacgccgacgtttatcatggggtgggtcgccaacttcctgcagttcttggtgttctacttcctcatcaccacgatggcgctctacgcaaccaaggaattcagcgcatcggaaaccgaagcaggctttgccgccagtgcgattgttatcggtgcggtcttttcccgtttggtttccggatacattattgaccgcttcggtcgccgcaaaattgtggtggtctccgtcatcgcgaccactattgcgtgcgcgctatatatcccgatcgattctttggggctgctctacgctgaccgcttcttccacggtgtagcttatgcctttgcgtgcaccgcgattatggcgatggtccaggaactcattccttctgcacgccgctccgaaggcactggctacctggctttgggtaccaccgtttcggctgctatcggaccagcgctagcgctatttttgctgggttctttcaactacgaagtcctcttcgttgtcgtcctcggcatttcgattgtctctttgatcgcttcgctagtcatctatttccgcacctccgacccagagccagagctggatgaaaacggcaatgctgctgagcccattaagttcagcttcaagtccatcattaaccctaaagtcttgccgattggcctcttcatgctgctggtagcctttgcctactccggcgtgatcgcacatatcaacgcttttgctgaaaaccgcgacgttgttactggcgcaggcctattctttatcgcttacgccatctccatgttcgtgatgcgctcctaccttggtaaattgcaagaccgccggggcgataacagcgttatctactttggtctcgtattctttgttatctcatttatcgtgctctcgctttctaccgccaactggcatgtcgttgtcgctggcgtgctagcaggtctgggctacggcaccttgatgccagctgctcaagcagtatctgttggtgttgtcgacaagagcgagttcggctcagcattttccaccttgttccttttcgttgacctcggcaacggcttcggcccagtcatccttggtgcagtggtttccgcgattggctacggttcgatgtatgcagtgctcgtcggcgtcggcgttattgctggcatctactacctgttcacccacgcacgcaccgagcgcgcaaagcacggcgtagtcaagcatgtagaaaccatggttctggctcaataa

SEQ ID NO: 23 - protein, 413 aa, synthetic construct
  source 1..413: note = C. st F354C AA
MHTTEEVKLFTPTFIMGWVANFLQFLVFYFLITTMALYATKEFSASETEAGFAASAIVIGAVFSRLVSGYIIDRFGRRKIVVVSVIATTIACALYIPIDSLGLLYADRFFHGVAYAFACTAIMAMVQELIPSARRSEGTGYLALGTTVSAAIGPALALFLLGSFNYEVLFVVVLGISIVSLIASLVIYFRTSDPEPELDENGNAAEPIKFSFKSIINPKVLPIGLFMLLVAFAYSGVIAHINAFAENRDVVTGAGLFFIAYAISMFVMRSYLGKLQDRRGDNSVIYFGLVFFVISFIVLSLSTANWHVVVAGVLAGLGYGTLMPAAQAVSVGVVDKSEFGSAFSTLFLFVDLGCGFGPVILGAVVSAIGYGSMYAVLVGVGVIAGIYYLFTHARTERAKHGVVKHVETMVLAQ

SEQ ID NO: 24 - DNA, 1242 bp, synthetic construct
  source 1..1242: mol_type = other DNA; note = C. st F354C NT
gtgcacacaaccgaagaggtcaaactctttacgccgacgtttatcatggggtgggtcgccaacttcctgcagttcttggtgttctacttcctcatcaccacgatggcgctctacgcaaccaaggaattcagcgcatcggaaaccgaagcaggctttgccgccagtgcgattgttatcggtgcggtcttttcccgtttggtttccggatacattattgaccgcttcggtcgccgcaaaattgtggtggtctccgtcatcgcgaccactattgcgtgcgcgctatatatcccgatcgattctttggggctgctctacgctgaccgcttcttccacggtgtagcttatgcctttgcgtgcaccgcgattatggcgatggtccaggaactcattccttctgcacgccgctccgaaggcactggctacctggctttgggtaccaccgtttcggctgctatcggaccagcgctagcgctatttttgctgggttctttcaactacgaagtcctcttcgttgtcgtcctcggcatttcgattgtctctttgatcgcttcgctagtcatctatttccgcacctccgacccagagccagagctggatgaaaacggcaatgctgctgagcccattaagttcagcttcaagtccatcattaaccctaaagtcttgccgattggcctcttcatgctgctggtagcctttgcctactccggcgtgatcgcacatatcaacgcttttgctgaaaaccgcgacgttgttactggcgcaggcctattctttatcgcttacgccatctccatgttcgtgatgcgctcctaccttggtaaattgcaagaccgccggggcgataacagcgttatctactttggtctcgtattctttgttatctcatttatcgtgctctcgctttctaccgccaactggcatgtcgttgtcgctggcgtgctagcaggtctgggctacggcaccttgatgccagctgctcaagcagtatctgttggtgttgtcgacaagagcgagttcggctcagcattttccaccttgttccttttcgttgacctcggctgcggcttcggcccagtcatccttggtgcagtggtttccgcgattggctacggttcgatgtatgcagtgctcgtcggcgtcggcgttattgctggcatctactacctgttcacccacgcacgcaccgagcgcgcaaagcacggcgtagtcaagcatgtagaaaccatggttctggctcaataa

SEQ ID NO: 25 - protein, 413 aa, synthetic construct
  source 1..413: note = C. st F354R AA
MHTTEEVKLFTPTFIMGWVANFLQFLVFYFLITTMALYATKEFSASETEAGFAASAIVIGAVFSRLVSGYIIDRFGRRKIVVVSVIATTIACALYIPIDSLGLLYADRFFHGVAYAFACTAIMAMVQELIPSARRSEGTGYLALGTTVSAAIGPALALFLLGSFNYEVLFVVVLGISIVSLIASLVIYFRTSDPEPELDENGNAAEPIKFSFKSIINPKVLPIGLFMLLVAFAYSGVIAHINAFAENRDVVTGAGLFFIAYAISMFVMRSYLGKLQDRRGDNSVIYFGLVFFVISFIVLSLSTANWHVVVAGVLAGLGYGTLMPAAQAVSVGVVDKSEFGSAFSTLFLFVDLGRGFGPVILGAVVSAIGYGSMYAVLVGVGVIAGIYYLFTHARTERAKHGVVKHVETMVLAQ

SEQ ID NO: 26 - DNA, 1242 bp, synthetic construct
  source 1..1242: mol_type = other DNA; note = C. st F354R NT
gtgcacacaaccgaagaggtcaaactctttacgccgacgtttatcatggggtgggtcgccaacttcctgcagttcttggtgttctacttcctcatcaccacgatggcgctctacgcaaccaaggaattcagcgcatcggaaaccgaagcaggctttgccgccagtgcgattgttatcggtgcggtcttttcccgtttggtttccggatacattattgaccgcttcggtcgccgcaaaattgtggtggtctccgtcatcgcgaccactattgcgtgcgcgctatatatcccgatcgattctttggggctgctctacgctgaccgcttcttccacggtgtagcttatgcctttgcgtgcaccgcgattatggcgatggtccaggaactcattccttctgcacgccgctccgaaggcactggctacctggctttgggtaccaccgtttcggctgctatcggaccagcgctagcgctatttttgctgggttctttcaactacgaagtcctcttcgttgtcgtcctcggcatttcgattgtctctttgatcgcttcgctagtcatctatttccgcacctccgacccagagccagagctggatgaaaacggcaatgctgctgagcccattaagttcagcttcaagtccatcattaaccctaaagtcttgccgattggcctcttcatgctgctggtagcctttgcctactccggcgtgatcgcacatatcaacgcttttgctgaaaaccgcgacgttgttactggcgcaggcctattctttatcgcttacgccatctccatgttcgtgatgcgctcctaccttggtaaattgcaagaccgccggggcgataacagcgttatctactttggtctcgtattctttgttatctcatttatcgtgctctcgctttctaccgccaactggcatgtcgttgtcgctggcgtgctagcaggtctgggctacggcaccttgatgccagctgctcaagcagtatctgttggtgttgtcgacaagagcgagttcggctcagcattttccaccttgttccttttcgttgacctcggcagaggcttcggcccagtcatccttggtgcagtggtttccgcgattggctacggttcgatgtatgcagtgctcgtcggcgtcggcgttattgctggcatctactacctgttcacccacgcacgcaccgagcgcgcaaagcacggcgtagtcaagcatgtagaaaccatggttctggctcaataa

SEQ ID NO: 27 - protein, 413 aa, synthetic construct
  source 1..413: note = C. st F354I AA
MHTTEEVKLFTPTFIMGWVANFLQFLVFYFLITTMALYATKEFSASETEAGFAASAIVIGAVFSRLVSGYIIDRFGRRKIVVVSVIATTIACALYIPIDSLGLLYADRFFHGVAYAFACTAIMAMVQELIPSARRSEGTGYLALGTTVSAAIGPALALFLLGSFNYEVLFVVVLGISIVSLIASLVIYFRTSDPEPELDENGNAAEPIKFSFKSIINPKVLPIGLFMLLVAFAYSGVIAHINAFAENRDVVTGAGLFFIAYAISMFVMRSYLGKLQDRRGDNSVIYFGLVFFVISFIVLSLSTANWHVVVAGVLAGLGYGTLMPAAQAVSVGVVDKSEFGSAFSTLFLFVDLGIGFGPVILGAVVSAIGYGSMYAVLVGVGVIAGIYYLFTHARTERAKHGVVKHVETMVLAQ

SEQ ID NO: 28 - DNA, 1242 bp, synthetic construct
  source 1..1242: mol_type = other DNA; note = C. st F354I NT
gtgcacacaaccgaagaggtcaaactctttacgccgacgtttatcatggggtgggtcgccaacttcctgcagttcttggtgttctacttcctcatcaccacgatggcgctctacgcaaccaaggaattcagcgcatcggaaaccgaagcaggctttgccgccagtgcgattgttatcggtgcggtcttttcccgtttggtttccggatacattattgaccgcttcggtcgccgcaaaattgtggtggtctccgtcatcgcgaccactattgcgtgcgcgctatatatcccgatcgattctttggggctgctctacgctgaccgcttcttccacggtgtagcttatgcctttgcgtgcaccgcgattatggcgatggtccaggaactcattccttctgcacgccgctccgaaggcactggctacctggctttgggtaccaccgtttcggctgctatcggaccagcgctagcgctatttttgctgggttctttcaactacgaagtcctcttcgttgtcgtcctcggcatttcgattgtctctttgatcgcttcgctagtcatctatttccgcacctccgacccagagccagagctggatgaaaacggcaatgctgctgagcccattaagttcagcttcaagtccatcattaaccctaaagtcttgccgattggcctcttcatgctgctggtagcctttgcctactccggcgtgatcgcacatatcaacgcttttgctgaaaaccgcgacgttgttactggcgcaggcctattctttatcgcttacgccatctccatgttcgtgatgcgctcctaccttggtaaattgcaagaccgccggggcgataacagcgttatctactttggtctcgtattctttgttatctcatttatcgtgctctcgctttctaccgccaactggcatgtcgttgtcgctggcgtgctagcaggtctgggctacggcaccttgatgccagctgctcaagcagtatctgttggtgttgtcgacaagagcgagttcggctcagcattttccaccttgttccttttcgttgacctcggcatcggcttcggcccagtcatccttggtgcagtggtttccgcgattggctacggttcgatgtatgcagtgctcgtcggcgtcggcgttattgctggcatctactacctgttcacccacgcacgcaccgagcgcgcaaagcacggcgtagtcaagcatgtagaaaccatggttctggctcaataa

SEQ ID NO: 29 - protein, 413 aa, synthetic construct
  source 1..413: note = C. st F354V AA
MHTTEEVKLFTPTFIMGWVANFLQFLVFYFLITTMALYATKEFSASETEAGFAASAIVIGAVFSRLVSGYIIDRFGRRKIVVVSVIATTIACALYIPIDSLGLLYADRFFHGVAYAFACTAIMAMVQELIPSARRSEGTGYLALGTTVSAAIGPALALFLLGSFNYEVLFVVVLGISIVSLIASLVIYFRTSDPEPELDENGNAAEPIKFSFKSIINPKVLPIGLFMLLVAFAYSGVIAHINAFAENRDVVTGAGLFFIAYAISMFVMRSYLGKLQDRRGDNSVIYFGLVFFVISFIVLSLSTANWHVVVAGVLAGLGYGTLMPAAQAVSVGVVDKSEFGSAFSTLFLFVDLGVGFGPVILGAVVSAIGYGSMYAVLVGVGVIAGIYYLFTHARTERAKHGVVKHVETMVLAQ

SEQ ID NO: 30 - DNA, 1242 bp, synthetic construct
  source 1..1242: mol_type = other DNA; note = C. st F354V NT
gtgcacacaaccgaagaggtcaaactctttacgccgacgtttatcatggggtgggtcgccaacttcctgcagttcttggtgttctacttcctcatcaccacgatggcgctctacgcaaccaaggaattcagcgcatcggaaaccgaagcaggctttgccgccagtgcgattgttatcggtgcggtcttttcccgtttggtttccggatacattattgaccgcttcggtcgccgcaaaattgtggtggtctccgtcatcgcgaccactattgcgtgcgcgctatatatcccgatcgattctttggggctgctctacgctgaccgcttcttccacggtgtagcttatgcctttgcgtgcaccgcgattatggcgatggtccaggaactcattccttctgcacgccgctccgaaggcactggctacctggctttgggtaccaccgtttcggctgctatcggaccagcgctagcgctatttttgctgggttctttcaactacgaagtcctcttcgttgtcgtcctcggcatttcgattgtctctttgatcgcttcgctagtcatctatttccgcacctccgacccagagccagagctggatgaaaacggcaatgctgctgagcccattaagttcagcttcaagtccatcattaaccctaaagtcttgccgattggcctcttcatgctgctggtagcctttgcctactccggcgtgatcgcacatatcaacgcttttgctgaaaaccgcgacgttgttactggcgcaggcctattctttatcgcttacgccatctccatgttcgtgatgcgctcctaccttggtaaattgcaagaccgccggggcgataacagcgttatctactttggtctcgtattctttgttatctcatttatcgtgctctcgctttctaccgccaactggcatgtcgttgtcgctggcgtgctagcaggtctgggctacggcaccttgatgccagctgctcaagcagtatctgttggtgttgtcgacaagagcgagttcggctcagcattttccaccttgttccttttcgttgacctcggcgtgggcttcggcccagtcatccttggtgcagtggtttccgcgattggctacggttcgatgtatgcagtgctcgtcggcgtcggcgttattgctggcatctactacctgttcacccacgcacgcaccgagcgcgcaaagcacggcgtagtcaagcatgtagaaaccatggttctggctcaataa

SEQ ID NO: 31 - protein, 413 aa, synthetic construct
  source 1..413: note = C. st F354D AA
MHTTEEVKLFTPTFIMGWVANFLQFLVFYFLITTMALYATKEFSASETEAGFAASAIVIGAVFSRLVSGYIIDRFGRRKIVVVSVIATTIACALYIPIDSLGLLYADRFFHGVAYAFACTAIMAMVQELIPSARRSEGTGYLALGTTVSAAIGPALALFLLGSFNYEVLFVVVLGISIVSLIASLVIYFRTSDPEPELDENGNAAEPIKFSFKSIINPKVLPIGLFMLLVAFAYSGVIAHINAFAENRDVVTGAGLFFIAYAISMFVMRSYLGKLQDRRGDNSVIYFGLVFFVISFIVLSLSTANWHVVVAGVLAGLGYGTLMPAAQAVSVGVVDKSEFGSAFSTLFLFVDLGDGFGPVILGAVVSAIGYGSMYAVLVGVGVIAGIYYLFTHARTERAKHGVVKHVETMVLAQ

SEQ ID NO: 32 - DNA, 1242 bp, synthetic construct
  source 1..1242: mol_type = other DNA; note = C. st F354D NT
gtgcacacaaccgaagaggtcaaactctttacgccgacgtttatcatggggtgggtcgccaacttcctgcagttcttggtgttctacttcctcatcaccacgatggcgctctacgcaaccaaggaattcagcgcatcggaaaccgaagcaggctttgccgccagtgcgattgttatcggtgcggtcttttcccgtttggtttccggatacattattgaccgcttcggtcgccgcaaaattgtggtggtctccgtcatcgcgaccactattgcgtgcgcgctatatatcccgatcgattctttggggctgctctacgctgaccgcttcttccacggtgtagcttatgcctttgcgtgcaccgcgattatggcgatggtccaggaactcattccttctgcacgccgctccgaaggcactggctacctggctttgggtaccaccgtttcggctgctatcggaccagcgctagcgctatttttgctgggttctttcaactacgaagtcctcttcgttgtcgtcctcggcatttcgattgtctctttgatcgcttcgctagtcatctatttccgcacctccgacccagagccagagctggatgaaaacggcaatgctgctgagcccattaagttcagcttcaagtccatcattaaccctaaagtcttgccgattggcctcttcatgctgctggtagcctttgcctactccggcgtgatcgcacatatcaacgcttttgctgaaaaccgcgacgttgttactggcgcaggcctattctttatcgcttacgccatctccatgttcgtgatgcgctcctaccttggtaaattgcaagaccgccggggcgataacagcgttatctactttggtctcgtattctttgttatctcatttatcgtgctctcgctttctaccgccaactggcatgtcgttgtcgctggcgtgctagcaggtctgggctacggcaccttgatgccagctgctcaagcagtatctgttggtgttgtcgacaagagcgagttcggctcagcattttccaccttgttccttttcgttgacctcggcgatggcttcggcccagtcatccttggtgcagtggtttccgcgattggctacggttcgatgtatgcagtgctcgtcggcgtcggcgttattgctggcatctactacctgttcacccacgcacgcaccgagcgcgcaaagcacggcgtagtcaagcatgtagaaaccatggttctggctcaataa

SEQ ID NO: 33 - protein, 413 aa, synthetic construct
  source 1..413: note = C. st F354G AA
MHTTEEVKLFTPTFIMGWVANFLQFLVFYFLITTMALYATKEFSASETEAGFAASAIVIGAVFSRLVSGYIIDRFGRRKIVVVSVIATTIACALYIPIDSLGLLYADRFFHGVAYAFACTAIMAMVQELIPSARRSEGTGYLALGTTVSAAIGPALALFLLGSFNYEVLFVVVLGISIVSLIASLVIYFRTSDPEPELDENGNAAEPIKFSFKSIINPKVLPIGLFMLLVAFAYSGVIAHINAFAENRDVVTGAGLFFIAYAISMFVMRSYLGKLQDRRGDNSVIYFGLVFFVISFIVLSLSTANWHVVVAGVLAGLGYGTLMPAAQAVSVGVVDKSEFGSAFSTLFLFVDLGGGFGPVILGAVVSAIGYGSMYAVLVGVGVIAGIYYLFTHARTERAKHGVVKHVETMVLAQ

SEQ ID NO: 34 - DNA, 1242 bp, synthetic construct
  source 1..1242: mol_type = other DNA; note = C. st F354G NT
gtgcacacaaccgaagaggtcaaactctttacgccgacgtttatcatggggtgggtcgccaacttcctgcagttcttggtgttctacttcctcatcaccacgatggcgctctacgcaaccaaggaattcagcgcatcggaaaccgaagcaggctttgccgccagtgcgattgttatcggtgcggtcttttcccgtttggtttccggatacattattgaccgcttcggtcgccgcaaaattgtggtggtctccgtcatcgcgaccactattgcgtgcgcgctatatatcccgatcgattctttggggctgctctacgctgaccgcttcttccacggtgtagcttatgcctttgcgtgcaccgcgattatggcgatggtccaggaactcattccttctgcacgccgctccgaaggcactggctacctggctttgggtaccaccgtttcggctgctatcggaccagcgctagcgctatttttgctgggttctttcaactacgaagtcctcttcgttgtcgtcctcggcatttcgattgtctctttgatcgcttcgctagtcatctatttccgcacctccgacccagagccagagctggatgaaaacggcaatgctgctgagcccattaagttcagcttcaagtccatcattaaccctaaagtcttgccgattggcctcttcatgctgctggtagcctttgcctactccggcgtgatcgcacatatcaacgcttttgctgaaaaccgcgacgttgttactggcgcaggcctattctttatcgcttacgccatctccatgttcgtgatgcgctcctaccttggtaaattgcaagaccgccggggcgataacagcgttatctactttggtctcgtattctttgttatctcatttatcgtgctctcgctttctaccgccaactggcatgtcgttgtcgctggcgtgctagcaggtctgggctacggcaccttgatgccagctgctcaagcagtatctgttggtgttgtcgacaagagcgagttcggctcagcattttccaccttgttccttttcgttgacctcggcggcggcttcggcccagtcatccttggtgcagtggtttccgcgattggctacggttcgatgtatgcagtgctcgtcggcgtcggcgttattgctggcatctactacctgttcacccacgcacgcaccgagcgcgcaaagcacggcgtagtcaagcatgtagaaaccatggttctggctcaataa

SEQ ID NO: 35 - protein, 413 aa, synthetic construct
  source 1..413: note = C. st F354P AA
MHTTEEVKLFTPTFIMGWVANFLQFLVFYFLITTMALYATKEFSASETEAGFAASAIVIGAVFSRLVSGYIIDRFGRRKIVVVSVIATTIACALYIPIDSLGLLYADRFFHGVAYAFACTAIMAMVQELIPSARRSEGTGYLALGTTVSAAIGPALALFLLGSFNYEVLFVVVLGISIVSLIASLVIYFRTSDPEPELDENGNAAEPIKFSFKSIINPKVLPIGLFMLLVAFAYSGVIAHINAFAENRDVVTGAGLFFIAYAISMFVMRSYLGKLQDRRGDNSVIYFGLVFFVISFIVLSLSTANWHVVVAGVLAGLGYGTLMPAAQAVSVGVVDKSEFGSAFSTLFLFVDLGPGFGPVILGAVVSAIGYGSMYAVLVGVGVIAGIYYLFTHARTERAKHGVVKHVETMVLAQ

SEQ ID NO: 36 - DNA, 1242 bp, synthetic construct
  source 1..1242: mol_type = other DNA; note = C. st F354P NT
gtgcacacaaccgaagaggtcaaactctttacgccgacgtttatcatggggtgggtcgccaacttcctgcagttcttggtgttctacttcctcatcaccacgatggcgctctacgcaaccaaggaattcagcgcatcggaaaccgaagcaggctttgccgccagtgcgattgttatcggtgcggtcttttcccgtttggtttccggatacattattgaccgcttcggtcgccgcaaaattgtggtggtctccgtcatcgcgaccactattgcgtgcgcgctatatatcccgatcgattctttggggctgctctacgctgaccgcttcttccacggtgtagcttatgcctttgcgtgcaccgcgattatggcgatggtccaggaactcattccttctgcacgccgctccgaaggcactggctacctggctttgggtaccaccgtttcggctgctatcggaccagcgctagcgctatttttgctgggttctttcaactacgaagtcctcttcgttgtcgtcctcggcatttcgattgtctctttgatcgcttcgctagtcatctatttccgcacctccgacccagagccagagctggatgaaaacggcaatgctgctgagcccattaagttcagcttcaagtccatcattaaccctaaagtcttgccgattggcctcttcatgctgctggtagcctttgcctactccggcgtgatcgcacatatcaacgcttttgctgaaaaccgcgacgttgttactggcgcaggcctattctttatcgcttacgccatctccatgttcgtgatgcgctcctaccttggtaaattgcaagaccgccggggcgataacagcgttatctactttggtctcgtattctttgttatctcatttatcgtgctctcgctttctaccgccaactggcatgtcgttgtcgctggcgtgctagcaggtctgggctacggcaccttgatgccagctgctcaagcagtatctgttggtgttgtcgacaagagcgagttcggctcagcattttccaccttgttccttttcgttgacctcggcccaggcttcggcccagtcatccttggtgcagtggtttccgcgattggctacggttcgatgtatgcagtgctcgtcggcgtcggcgttattgctggcatctactacctgttcacccacgcacgcaccgagcgcgcaaagcacggcgtagtcaagcatgtagaaaccatggttctggctcaataa

SEQ ID NO: 37 - protein, 413 aa, synthetic construct
  source 1..413: note = C. st F354A AA
MHTTEEVKLFTPTFIMGWVANFLQFLVFYFLITTMALYATKEFSASETEAGFAASAIVIGAVFSRLVSGYIIDRFGRRKIVVVSVIATTIACALYIPIDSLGLLYADRFFHGVAYAFACTAIMAMVQELIPSARRSEGTGYLALGTTVSAAIGPALALFLLGSFNYEVLFVVVLGISIVSLIASLVIYFRTSDPEPELDENGNAAEPIKFSFKSIINPKVLPIGLFMLLVAFAYSGVIAHINAFAENRDVVTGAGLFFIAYAISMFVMRSYLGKLQDRRGDNSVIYFGLVFFVISFIVLSLSTANWHVVVAGVLAGLGYGTLMPAAQAVSVGVVDKSEFGSAFSTLFLFVDLGAGFGPVILGAVVSAIGYGSMYAVLVGVGVIAGIYYLFTHARTERAKHGVVKHVETMVLAQ

SEQ ID NO: 38 - DNA, 1242 bp, synthetic construct
  source 1..1242: mol_type = other DNA; note = C. st F354A NT
gtgcacacaaccgaagaggtcaaactctttacgccgacgtttatcatggggtgggtcgccaacttcctgcagttcttggtgttctacttcctcatcaccacgatggcgctctacgcaaccaaggaattcagcgcatcggaaaccgaagcaggctttgccgccagtgcgattgttatcggtgcggtcttttcccgtttggtttccggatacattattgaccgcttcggtcgccgcaaaattgtggtggtctccgtcatcgcgaccactattgcgtgcgcgctatatatcccgatcgattctttggggctgctctacgctgaccgcttcttccacggtgtagcttatgcctttgcgtgcaccgcgattatggcgatggtccaggaactcattccttctgcacgccgctccgaaggcactggctacctggctttgggtaccaccgtttcggctgctatcggaccagcgctagcgctatttttgctgggttctttcaactacgaagtcctcttcgttgtcgtcctcggcatttcgattgtctctttgatcgcttcgctagtcatctatttccgcacctccgacccagagccagagctggatgaaaacggcaatgctgctgagcccattaagttcagcttcaagtccatcattaaccctaaagtcttgccgattggcctcttcatgctgctggtagcctttgcctactccggcgtgatcgcacatatcaacgcttttgctgaaaaccgcgacgttgttactggcgcaggcctattctttatcgcttacgccatctccatgttcgtgatgcgctcctaccttggtaaattgcaagaccgccggggcgataacagcgttatctactttggtctcgtattctttgttatctcatttatcgtgctctcgctttctaccgccaactggcatgtcgttgtcgctggcgtgctagcaggtctgggctacggcaccttgatgccagctgctcaagcagtatctgttggtgttgtcgacaagagcgagttcggctcagcattttccaccttgttccttttcgttgacctcggcgcaggcttcggcccagtcatccttggtgcagtggtttccgcgattggctacggttcgatgtatgcagtgctcgtcggcgtcggcgttattgctggcatctactacctgttcacccacgcacgcaccgagcgcgcaaagcacggcgtagtcaagcatgtagaaaccatggttctggctcaataa

SEQ ID NO: 39 - protein, 413 aa, synthetic construct
  source 1..413: note = C. st F354E AA
MHTTEEVKLFTPTFIMGWVANFLQFLVFYFLITTMALYATKEFSASETEAGFAASAIVIGAVFSRLVSGYIIDRFGRRKIVVVSVIATTIACALYIPIDSLGLLYADRFFHGVAYAFACTAIMAMVQELIPSARRSEGTGYLALGTTVSAAIGPALALFLLGSFNYEVLFVVVLGISIVSLIASLVIYFRTSDPEPELDENGNAAEPIKFSFKSIINPKVLPIGLFMLLVAFAYSGVIAHINAFAENRDVVTGAGLFFIAYAISMFVMRSYLGKLQDRRGDNSVIYFGLVFFVISFIVLSLSTANWHVVVAGVLAGLGYGTLMPAAQAVSVGVVDKSEFGSAFSTLFLFVDLGEGFGPVILGAVVSAIGYGSMYAVLVGVGVIAGIYYLFTHARTERAKHGVVKHVETMVLAQ

SEQ ID NO: 40 - DNA, 1242 bp, synthetic construct
  source 1..1242: mol_type = other DNA; note = C. st F354E NT
gtgcacacaaccgaagaggtcaaactctttacgccgacgtttatcatggggtgggtcgccaacttcctgcagttcttggtgttctacttcctcatcaccacgatggcgctctacgcaaccaaggaattcagcgcatcggaaaccgaagcaggctttgccgccagtgcgattgttatcggtgcggtcttttcccgtttggtttccggatacattattgaccgcttcggtcgccgcaaaattgtggtggtctccgtcatcgcgaccactattgcgtgcgcgctatatatcccgatcgattctttggggctgctctacgctgaccgcttcttccacggtgtagcttatgcctttgcgtgcaccgcgattatggcgatggtccaggaactcattccttctgcacgccgctccgaaggcactggctacctggctttgggtaccaccgtttcggctgctatcggaccagcgctagcgctatttttgctgggttctttcaactacgaagtcctcttcgttgtcgtcctcggcatttcgattgtctctttgatcgcttcgctagtcatctatttccgcacctccgacccagagccagagctggatgaaaacggcaatgctgctgagcccattaagttcagcttcaagtccatcattaaccctaaagtcttgccgattggcctcttcatgctgctggtagcctttgcctactccggcgtgatcgcacatatcaacgcttttgctgaaaaccgcgacgttgttactggcgcaggcctattctttatcgcttacgccatctccatgttcgtgatgcgctcctaccttggtaaattgcaagaccgccggggcgataacagcgttatctactttggtctcgtattctttgttatctcatttatcgtgctctcgctttctaccgccaactggcatgtcgttgtcgctggcgtgctagcaggtctgggctacggcaccttgatgccagctgctcaagcagtatctgttggtgttgtcgacaagagcgagttcggctcagcattttccaccttgttccttttcgttgacctcggcgaaggcttcggcccagtcatccttggtgcagtggtttccgcgattggctacggttcgatgtatgcagtgctcgtcggcgtcggcgttattgctggcatctactacctgttcacccacgcacgcaccgagcgcgcaaagcacggcgtagtcaagcatgtagaaaccatggttctggctcaataa

SEQ ID NO: 41 - protein, 413 aa, synthetic construct
  source 1..413: note = C. st F354M AA
MHTTEEVKLFTPTFIMGWVANFLQFLVFYFLITTMALYATKEFSASETEAGFAASAIVIGAVFSRLVSGYIIDRFGRRKIVVVSVIATTIACALYIPIDSLGLLYADRFFHGVAYAFACTAIMAMVQELIPSARRSEGTGYLALGTTVSAAIGPALALFLLGSFNYEVLFVVVLGISIVSLIASLVIYFRTSDPEPELDENGNAAEPIKFSFKSIINPKVLPIGLFMLLVAFAYSGVIAHINAFAENRDVVTGAGLFFIAYAISMFVMRSYLGKLQDRRGDNSVIYFGLVFFVISFIVLSLSTANWHVVVAGVLAGLGYGTLMPAAQAVSVGVVDKSEFGSAFSTLFLFVDLGMGFGPVILGAVVSAIGYGSMYAVLVGVGVIAGIYYLFTHARTERAKHGVVKHVETMVLAQ

SEQ ID NO: 42 - DNA, 1242 bp, synthetic construct
  source 1..1242: mol_type = other DNA; note = C. st F354M NT
gtgcacacaaccgaagaggtcaaactctttacgccgacgtttatcatggggtgggtcgccaacttcctgcagttcttggtgttctacttcctcatcaccacgatggcgctctacgcaaccaaggaattcagcgcatcggaaaccgaagcaggctttgccgccagtgcgattgttatcggtgcggtcttttcccgtttggtttccggatacattattgaccgcttcggtcgccgcaaaattgtggtggtctccgtcatcgcgaccactattgcgtgcgcgctatatatcccgatcgattctttggggctgctctacgctgaccgcttcttccacggtgtagcttatgcctttgcgtgcaccgcgattatggcgatggtccaggaactcattccttctgcacgccgctccgaaggcactggctacctggctttgggtaccaccgtttcggctgctatcggaccagcgctagcgctatttttgctgggttctttcaactacgaagtcctcttcgttgtcgtcctcggcatttcgattgtctctttgatcgcttcgctagtcatctatttccgcacctccgacccagagccagagctggatgaaaacggcaatgctgctgagcccattaagttcagcttcaagtccatcattaaccctaaagtcttgccgattggcctcttcatgctgctggtagcctttgcctactccggcgtgatcgcacatatcaacgcttttgctgaaaaccgcgacgttgttactggcgcaggcctattctttatcgcttacgccatctccatgttcgtgatgcgctcctaccttggtaaattgcaagaccgccggggcgataacagcgttatctactttggtctcgtattctttgttatctcatttatcgtgctctcgctttctaccgccaactggcatgtcgttgtcgctggcgtgctagcaggtctgggctacggcaccttgatgccagctgctcaagcagtatctgttggtgttgtcgacaagagcgagttcggctcagcattttccaccttgttccttttcgttgacctcggcatgggcttcggcccagtcatccttggtgcagtggtttccgcgattggctacggttcgatgtatgcagtgctcgtcggcgtcggcgttattgctggcatctactacctgttcacccacgcacgcaccgagcgcgcaaagcacggcgtagtcaagcatgtagaaaccatggttctggctcaataa

SEQ ID NO: 43 - protein, 413 aa, synthetic construct
  source 1..413: note = C. st F354W AA
MHTTEEVKLFTPTFIMGWVANFLQFLVFYFLITTMALYATKEFSASETEAGFAASAIVIGAVFSRLVSGYIIDRFGRRKIVVVSVIATTIACALYIPIDSLGLLYADRFFHGVAYAFACTAIMAMVQELIPSARRSEGTGYLALGTTVSAAIGPALALFLLGSFNYEVLFVVVLGISIVSLIASLVIYFRTSDPEPELDENGNAAEPIKFSFKSIINPKVLPIGLFMLLVAFAYSGVIAHINAFAENRDVVTGAGLFFIAYAISMFVMRSYLGKLQDRRGDNSVIYFGLVFFVISFIVLSLSTANWHVVVAGVLAGLGYGTLMPAAQAVSVGVVDKSEFGSAFSTLFLFVDLGWGFGPVILGAVVSAIGYGSMYAVLVGVGVIAGIYYLFTHARTERAKHGVVKHVETMVLAQ

SEQ ID NO: 44 - DNA, 1242 bp, synthetic construct
  source 1..1242: mol_type = other DNA; note = C. st F354W NT
gtgcacacaaccgaagaggtcaaactctttacgccgacgtttatcatggggtgggtcgccaacttcctgcagttcttggtgttctacttcctcatcaccacgatggcgctctacgcaaccaaggaattcagcgcatcggaaaccgaagcaggctttgccgccagtgcgattgttatcggtgcggtcttttcccgtttggtttccggatacattattgaccgcttcggtcgccgcaaaattgtggtggtctccgtcatcgcgaccactattgcgtgcgcgctatatatcccgatcgattctttggggctgctctacgctgaccgcttcttccacggtgtagcttatgcctttgcgtgcaccgcgattatggcgatggtccaggaactcattccttctgcacgccgctccgaaggcactggctacctggctttgggtaccaccgtttcggctgctatcggaccagcgctagcgctatttttgctgggttctttcaactacgaagtcctcttcgttgtcgtcctcggcatttcgattgtctctttgatcgcttcgctagtcatctatttccgcacctccgacccagagccagagctggatgaaaacggcaatgctgctgagcccattaagttcagcttcaagtccatcattaaccctaaagtcttgccgattggcctcttcatgctgctggtagcctttgcctactccggcgtgatcgcacatatcaacgcttttgctgaaaaccgcgacgttgttactggcgcaggcctattctttatcgcttacgccatctccatgttcgtgatgcgctcctaccttggtaaattgcaagaccgccggggcgataacagcgttatctactttggtctcgtattctttgttatctcatttatcgtgctctcgctttctaccgccaactggcatgtcgttgtcgctggcgtgctagcaggtctgggctacggcaccttgatgccagctgctcaagcagtatctgttggtgttgtcgacaagagcgagttcggctcagcattttccaccttgttccttttcgttgacctcggctggggcttcggcccagtcatccttggtgcagtggtttccgcgattggctacggttcgatgtatgcagtgctcgtcggcgtcggcgttattgctggcatctactacctgttcacccacgcacgcaccgagcgcgcaaagcacggcgtagtcaagcatgtagaaaccatggttctggctcaataa

SEQ ID NO: 45 - protein, 413 aa, synthetic construct
  source 1..413: note = C. st F354T AA
MHTTEEVKLFTPTFIMGWVANFLQFLVFYFLITTMALYATKEFSASETEAGFAASAIVIGAVFSRLVSGYIIDRFGRRKIVVVSVIATTIACALYIPIDSLGLLYADRFFHGVAYAFACTAIMAMVQELIPSARRSEGTGYLALGTTVSAAIGPALALFLLGSFNYEVLFVVVLGISIVSLIASLVIYFRTSDPEPELDENGNAAEPIKFSFKSIINPKVLPIGLFMLLVAFAYSGVIAHINAFAENRDVVTGAGLFFIAYAISMFVMRSYLGKLQDRRGDNSVIYFGLVFFVISFIVLSLSTANWHVVVAGVLAGLGYGTLMPAAQAVSVGVVDKSEFGSAFSTLFLFVDLGTGFGPVILGAVVSAIGYGSMYAVLVGVGVIAGIYYLFTHARTERAKHGVVKHVETMVLAQ

SEQ ID NO: 46 - DNA, 1242 bp, synthetic construct
  source 1..1242: mol_type = other DNA; note = C. st F354T NT
gtgcacacaaccgaagaggtcaaactctttacgccgacgtttatcatggggtgggtcgccaacttcctgcagttcttggtgttctacttcctcatcaccacgatggcgctctacgcaaccaaggaattcagcgcatcggaaaccgaagcaggctttgccgccagtgcgattgttatcggtgcggtcttttcccgtttggtttccggatacattattgaccgcttcggtcgccgcaaaattgtggtggtctccgtcatcgcgaccactattgcgtgcgcgctatatatcccgatcgattctttggggctgctctacgctgaccgcttcttccacggtgtagcttatgcctttgcgtgcaccgcgattatggcgatggtccaggaactcattccttctgcacgccgctccgaaggcactggctacctggctttgggtaccaccgtttcggctgctatcggaccagcgctagcgctatttttgctgggttctttcaactacgaagtcctcttcgttgtcgtcctcggcatttcgattgtctctttgatcgcttcgctagtcatctatttccgcacctccgacccagagccagagctggatgaaaacggcaatgctgctgagcccattaagttcagcttcaagtccatcattaaccctaaagtcttgccgattggcctcttcatgctgctggtagcctttgcctactccggcgtgatcgcacatatcaacgcttttgctgaaaaccgcgacgttgttactggcgcaggcctattctttatcgcttacgccatctccatgttcgtgatgcgctcctaccttggtaaattgcaagaccgccggggcgataacagcgttatctactttggtctcgtattctttgttatctcatttatcgtgctctcgctttctaccgccaactggcatgtcgttgtcgctggcgtgctagcaggtctgggctacggcaccttgatgccagctgctcaagcagtatctgttggtgttgtcgacaagagcgagttcggctcagcattttccaccttgttccttttcgttgacctcggcaccggcttcggcccagtcatccttggtgcagtggtttccgcgattggctacggttcgatgtatgcagtgctcgtcggcgtcggcgttattgctggcatctactacctgttcacccacgcacgcaccgagcgcgcaaagcacggcgtagtcaagcatgtagaaaccatggttctggctcaataa

SEQ ID NO: 47 - protein, 413 aa, synthetic construct
  source 1..413: note = C. st F354Q AA
MHTTEEVKLFTPTFIMGWVANFLQFLVFYFLITTMALYATKEFSASETEAGFAASAIVIGAVFSRLVSGYIIDRFGRRKIVVVSVIATTIACALYIPIDSLGLLYADRFFHGVAYAFACTAIMAMVQELIPSARRSEGTGYLALGTTVSAAIGPALALFLLGSFNYEVLFVVVLGISIVSLIASLVIYFRTSDPEPELDENGNAAEPIKFSFKSIINPKVLPIGLFMLLVAFAYSGVIAHINAFAENRDVVTGAGLFFIAYAISMFVMRSYLGKLQDRRGDNSVIYFGLVFFVISFIVLSLSTANWHVVVAGVLAGLGYGTLMPAAQAVSVGVVDKSEFGSAFSTLFLFVDLGQGFGPVILGAVVSAIGYGSMYAVLVGVGVIAGIYYLFTHARTERAKHGVVKHVETMVLAQ

SEQ ID NO: 48 - DNA, 1242 bp, synthetic construct
  source 1..1242: mol_type = other DNA; note = C. st F354Q NT
gtgcacacaaccgaagaggtcaaactctttacgccgacgtttatcatggggtgggtcgccaacttcctgcagttcttggtgttctacttcctcatcaccacgatggcgctctacgcaaccaaggaattcagcgcatcggaaaccgaagcaggctttgccgccagtgcgattgttatcggtgcggtcttttcccgtttggtttccggatacattattgaccgcttcggtcgccgcaaaattgtggtggtctccgtcatcgcgaccactattgcgtgcgcgctatatatcccgatcgattctttggggctgctctacgctgaccgcttcttccacggtgtagcttatgcctttgcgtgcaccgcgattatggcgatggtccaggaactcattccttctgcacgccgctccgaaggcactggctacctggctttgggtaccaccgtttcggctgctatcggaccagcgctagcgctatttttgctgggttctttcaactacgaagtcctcttcgttgtcgtcctcggcatttcgattgtctctttgatcgcttcgctagtcatctatttccgcacctccgacccagagccagagctggatgaaaacggcaatgctgctgagcccattaagttcagcttcaagtccatcattaaccctaaagtcttgccgattggcctcttcatgctgctggtagcctttgcctactccggcgtgatcgcacatatcaacgcttttgctgaaaaccgcgacgttgttactggcgcaggcctattctttatcgcttacgccatctccatgttcgtgatgcgctcctaccttggtaaattgcaagaccgccggggcgataacagcgttatctactttggtctcgtattctttgttatctcatttatcgtgctctcgctttctaccgccaactggcatgtcgttgtcgctggcgtgctagcaggtctgggctacggcaccttgatgccagctgctcaagcagtatctgttggtgttgtcgacaagagcgagttcggctcagcattttccaccttgttccttttcgttgacctcggccagggcttcggcccagtcatccttggtgcagtggtttccgcgattggctacggttcgatgtatgcagtgctcgtcggcgtcggcgttattgctggcatctactacctgttcacccacgcacgcaccgagcgcgcaaagcacggcgtagtcaagcatgtagaaaccatggttctggctcaataa

SEQ ID NO: 49 - protein, 413 aa, synthetic construct
  source 1..413: note = C. st F354K AA
MHTTEEVKLFTPTFIMGWVANFLQFLVFYFLITTMALYATKEFSASETEAGFAASAIVIGAVFSRLVSGYIIDRFGRRKIVVVSVIATTIACALYIPIDSLGLLYADRFFHGVAYAFACTAIMAMVQELIPSARRSEGTGYLALGTTVSAAIGPALALFLLGSFNYEVLFVVVLGISIVSLIASLVIYFRTSDPEPELDENGNAAEPIKFSFKSIINPKVLPIGLFMLLVAFAYSGVIAHINAFAENRDVVTGAGLFFIAYAISMFVMRSYLGKLQDRRGDNSVIYFGLVFFVISFIVLSLSTANWHVVVAGVLAGLGYGTLMPAAQAVSVGVVDKSEFGSAFSTLFLFVDLGKGFGPVILGAVVSAIGYGSMYAVLVGVGVIAGIYYLFTHARTERAKHGVVKHVETMVLAQ

SEQ ID NO: 50 - DNA, 1242 bp, synthetic construct
  source 1..1242: mol_type = other DNA; note = C. st F354K NT
gtgcacacaaccgaagaggtcaaactctttacgccgacgtttatcatggggtgggtcgccaacttcctgcagttcttggtgttctacttcctcatcaccacgatggcgctctacgcaaccaaggaattcagcgcatcggaaaccgaagcaggctttgccgccagtgcgattgttatcggtgcggtcttttcccgtttggtttccggatacattattgaccgcttcggtcgccgcaaaattgtggtggtctccgtcatcgcgaccactattgcgtgcgcgctatatatcccgatcgattctttggggctgctctacgctgaccgcttcttccacggtgtagcttatgcctttgcgtgcaccgcgattatggcgatggtccaggaactcattccttctgcacgccgctccgaaggcactggctacctggctttgggtaccaccgtttcggctgctatcggaccagcgctagcgctatttttgctgggttctttcaactacgaagtcctcttcgttgtcgtcctcggcatttcgattgtctctttgatcgcttcgctagtcatctatttccgcacctccgacccagagccagagctggatgaaaacggcaatgctgctgagcccattaagttcagcttcaagtccatcattaaccctaaagtcttgccgattggcctcttcatgctgctggtagcctttgcctactccggcgtgatcgcacatatcaacgcttttgctgaaaaccgcgacgttgttactggcgcaggcctattctttatcgcttacgccatctccatgttcgtgatgcgctcctaccttggtaaattgcaagaccgccggggcgataacagcgttatctactttggtctcgtattctttgttatctcatttatcgtgctctcgctttctaccgccaactggcatgtcgttgtcgctggcgtgctagcaggtctgggctacggcaccttgatgccagctgctcaagcagtatctgttggtgttgtcgacaagagcgagttcggctcagcattttccaccttgttccttttcgttgacctcggcaagggcttcggcccagtcatccttggtgcagtggtttccgcgattggctacggttcgatgtatgcagtgctcgtcggcgtcggcgttattgctggcatctactacctgttcacccacgcacgcaccgagcgcgcaaagcacggcgtagtcaagcatgtagaaaccatggttctggctcaataa

SEQ ID NO: 51 - protein, 413 aa, synthetic construct
  source 1..413: note = C. st F354L AA
MHTTEEVKLFTPTFIMGWVANFLQFLVFYFLITTMALYATKEFSASETEAGFAASAIVIGAVFSRLVSGYIIDRFGRRKIVVVSVIATTIACALYIPIDSLGLLYADRFFHGVAYAFACTAIMAMVQELIPSARRSEGTGYLALGTTVSAAIGPALALFLLGSFNYEVLFVVVLGISIVSLIASLVIYFRTSDPEPELDENGNAAEPIKFSFKSIINPKVLPIGLFMLLVAFAYSGVIAHINAFAENRDVVTGAGLFFIAYAISMFVMRSYLGKLQDRRGDNSVIYFGLVFFVISFIVLSLSTANWHVVVAGVLAGLGYGTLMPAAQAVSVGVVDKSEFGSAFSTLFLFVDLGLGFGPVILGAVVSAIGYGSMYAVLVGVGVIAGIYYLFTHARTERAKHGVVKHVETMVLAQ

SEQ ID NO: 52 - DNA, 1242 bp, synthetic construct
  source 1..1242: mol_type = other DNA; note = C. st F354L NT
gtgcacacaaccgaagaggtcaaactctttacgccgacgtttatcatggggtgggtcgccaacttcctgcagttcttggtgttctacttcctcatcaccacgatggcgctctacgcaaccaaggaattcagcgcatcggaaaccgaagcaggctttgccgccagtgcgattgttatcggtgcggtcttttcccgtttggtttccggatacattattgaccgcttcggtcgccgcaaaattgtggtggtctccgtcatcgcgaccactattgcgtgcgcgctatatatcccgatcgattctttggggctgctctacgctgaccgcttcttccacggtgtagcttatgcctttgcgtgcaccgcgattatggcgatggtccaggaactcattccttctgcacgccgctccgaaggcactggctacctggctttgggtaccaccgtttcggctgctatcggaccagcgctagcgctatttttgctgggttctttcaactacgaagtcctcttcgttgtcgtcctcggcatttcgattgtctctttgatcgcttcgctagtcatctatttccgcacctccgacccagagccagagctggatgaaaacggcaatgctgctgagcccattaagttcagcttcaagtccatcattaaccctaaagtcttgccgattggcctcttcatgctgctggtagcctttgcctactccggcgtgatcgcacatatcaacgcttttgctgaaaaccgcgacgttgttactggcgcaggcctattctttatcgcttacgccatctccatgttcgtgatgcgctcctaccttggtaaattgcaagaccgccggggcgataacagcgttatctactttggtctcgtattctttgttatctcatttatcgtgctctcgctttctaccgccaactggcatgtcgttgtcgctggcgtgctagcaggtctgggctacggcaccttgatgccagctgctcaagcagtatctgttggtgttgtcgacaagagcgagttcggctcagcattttccaccttgttccttttcgttgacctcggcctgggcttcggcccagtcatccttggtgcagtggtttccgcgattggctacggttcgatgtatgcagtgctcgtcggcgtcggcgttattgctggcatctactacctgttcacccacgcacgcaccgagcgcgcaaagcacggcgtagtcaagcatgtagaaaccatggttctggctcaataa

SEQ ID NO: 53 - protein, 413 aa, synthetic construct
  source 1..413: note = C. st F354H AA
MHTTEEVKLFTPTFIMGWVANFLQFLVFYFLITTMALYATKEFSASETEAGFAASAIVIGAVFSRLVSGYIIDRFGRRKIVVVSVIATTIACALYIPIDSLGLLYADRFFHGVAYAFACTAIMAMVQELIPSARRSEGTGYLALGTTVSAAIGPALALFLLGSFNYEVLFVVVLGISIVSLIASLVIYFRTSDPEPELDENGNAAEPIKFSFKSIINPKVLPIGLFMLLVAFAYSGVIAHINAFAENRDVVTGAGLFFIAYAISMFVMRSYLGKLQDRRGDNSVIYFGLVFFVISFIVLSLSTANWHVVVAGVLAGLGYGTLMPAAQAVSVGVVDKSEFGSAFSTLFLFVDLGHGFGPVILGAVVSAIGYGSMYAVLVGVGVIAGIYYLFTHARTERAKHGVVKHVETMVLAQ

SEQ ID NO: 54 - DNA, 1242 bp, synthetic construct
  source 1..1242: mol_type = other DNA; note = C. st F354H NT
gtgcacacaaccgaagaggtcaaactctttacgccgacgtttatcatggggtgggtcgccaacttcctgcagttcttggtgttctacttcctcatcaccacgatggcgctctacgcaaccaaggaattcagcgcatcggaaaccgaagcaggctttgccgccagtgcgattgttatcggtgcggtcttttcccgtttggtttccggatacattattgaccgcttcggtcgccgcaaaattgtggtggtctccgtcatcgcgaccactattgcgtgcgcgctatatatcccgatcgattctttggggctgctctacgctgaccgcttcttccacggtgtagcttatgcctttgcgtgcaccgcgattatggcgatggtccaggaactcattccttctgcacgccgctccgaaggcactggctacctggctttgggtaccaccgtttcggctgctatcggaccagcgctagcgctatttttgctgggttctttcaactacgaagtcctcttcgttgtcgtcctcggcatttcgattgtctctttgatcgcttcgctagtcatctatttccgcacctccgacccagagccagagctggatgaaaacggcaatgctgctgagcccattaagttcagcttcaagtccatcattaaccctaaagtcttgccgattggcctcttcatgctgctggtagcctttgcctactccggcgtgatcgcacatatcaacgcttttgctgaaaaccgcgacgttgttactggcgcaggcctattctttatcgcttacgccatctccatgttcgtgatgcgctcctaccttggtaaattgcaagaccgccggggcgataacagcgttatctactttggtctcgtattctttgttatctcatttatcgtgctctcgctttctaccgccaactggcatgtcgttgtcgctggcgtgctagcaggtctgggctacggcaccttgatgccagctgctcaagcagtatctgttggtgttgtcgacaagagcgagttcggctcagcattttccaccttgttccttttcgttgacctcggccacggcttcggcccagtcatccttggtgcagtggtttccgcgattggctacggttcgatgtatgcagtgctcgtcggcgtcggcgttattgctggcatctactacctgttcacccacgcacgcaccgagcgcgcaaagcacggcgtagtcaagcatgtagaaaccatggttctggctcaataa

SEQ ID NO: 55 - protein, 413 aa, synthetic construct
  source 1..413: note = C. st I259T AA
MHTTEEVKLFTPTFIMGWVANFLQFLVFYFLITTMALYATKEFSASETEAGFAASAIVIGAVFSRLVSGYIIDRFGRRKIVVVSVIATTIACALYIPIDSLGLLYADRFFHGVAYAFACTAIMAMVQELIPSARRSEGTGYLALGTTVSAAIGPALALFLLGSFNYEVLFVVVLGISIVSLIASLVIYFRTSDPEPELDENGNAAEPIKFSFKSIINPKVLPIGLFMLLVAFAYSGVIAHINAFAENRDVVTGAGLFFTAYAISMFVMRSYLGKLQDRRGDNSVIYFGLVFFVISFIVLSLSTANWHVVVAGVLAGLGYGTLMPAAQAVSVGVVDKSEFGSAFSTLFLFVDLGFGFGPVILGAVVSAIGYGSMYAVLVGVGVIAGIYYLFTHARTERAKHGVVKHVETMVLAQ

SEQ ID NO: 56 - DNA, 1242 bp, synthetic construct
  source 1..1242: mol_type = other DNA; note = C. st I259T NT
gtgcacacaaccgaagaggtcaaactctttacgccgacgtttatcatggggtgggtcgccaacttcctgcagttcttggtgttctacttcctcatcaccacgatggcgctctacgcaaccaaggaattcagcgcatcggaaaccgaagcaggctttgccgccagtgcgattgttatcggtgcggtcttttcccgtttggtttccggatacattattgaccgcttcggtcgccgcaaaattgtggtggtctccgtcatcgcgaccactattgcgtgcgcgctatatatcccgatcgattctttggggctgctctacgctgaccgcttcttccacggtgtagcttatgcctttgcgtgcaccgcgattatggcgatggtccaggaactcattccttctgcacgccgctccgaaggcactggctacctggctttgggtaccaccgtttcggctgctatcggaccagcgctagcgctatttttgctgggttctttcaactacgaagtcctcttcgttgtcgtcctcggcatttcgattgtctctttgatcgcttcgctagtcatctatttccgcacctccgacccagagccagagctggatgaaaacggcaatgctgctgagcccattaagttcagcttcaagtccatcattaaccctaaagtcttgccgattggcctcttcatgctgctggtagcctttgcctactccggcgtgatcgcacatatcaacgcttttgctgaaaaccgcgacgttgttactggcgcaggcctattctttaccgcttacgccatctccatgttcgtgatgcgctcctaccttggtaaattgcaagaccgccggggcgataacagcgttatctactttggtctcgtattctttgttatctcatttatcgtgctctcgctttctaccgccaactggcatgtcgttgtcgctggcgtgctagcaggtctgggctacggcaccttgatgccagctgctcaagcagtatctgttggtgttgtcgacaagagcgagttcggctcagcattttccaccttgttccttttcgttgacctcggcttcggcttcggcccagtcatccttggtgcagtggtttccgcgattggctacggttcgatgtatgcagtgctcgtcggcgtcggcgttattgctggcatctactacctgttcacccacgcacgcaccgagcgcgcaaagcacggcgtagtcaagcatgtagaaaccatggttctggctcaataa

SEQ ID NO: 57 - protein, 413 aa, synthetic construct
  source 1..413: note = C. st I259S AA
MHTTEEVKLFTPTFIMGWVANFLQFLVFYFLITTMALYATKEFSASETEAGFAASAIVIGAVFSRLVSGYIIDRFGRRKIVVVSVIATTIACALYIPIDSLGLLYADRFFHGVAYAFACTAIMAMVQELIPSARRSEGTGYLALGTTVSAAIGPALALFLLGSFNYEVLFVVVLGISIVSLIASLVIYFRTSDPEPELDENGNAAEPIKFSFKSIINPKVLPIGLFMLLVAFAYSGVIAHINAFAENRDVVTGAGLFFSAYAISMFVMRSYLGKLQDRRGDNSVIYFGLVFFVISFIVLSLSTANWHVVVAGVLAGLGYGTLMPAAQAVSVGVVDKSEFGSAFSTLFLFVDLGFGFGPVILGAVVSAIGYGSMYAVLVGVGVIAGIYYLFTHARTERAKHGVVKHVETMVLAQ

SEQ ID NO: 58 - DNA, 1242 bp, synthetic construct
  source 1..1242: mol_type = other DNA; note = C. st I259S NT
gtgcacacaaccgaagaggtcaaactctttacgccgacgtttatcatggggtgggtcgccaacttcctgcagttcttggtgttctacttcctcatcaccacgatggcgctctacgcaaccaaggaattcagcgcatcggaaaccgaagcaggctttgccgccagtgcgattgttatcggtgcggtcttttcccgtttggtttccggatacattattgaccgcttcggtcgccgcaaaattgtggtggtctccgtcatcgcgaccactattgcgtgcgcgctatatatcccgatcgattctttggggctgctctacgctgaccgcttcttccacggtgtagcttatgcctttgcgtgcaccgcgattatggcgatggtccaggaactcattccttctgcacgccgctccgaaggcactggctacctggctttgggtaccaccgtttcggctgctatcggaccagcgctagcgctatttttgctgggttctttcaactacgaagtcctcttcgttgtcgtcctcggcatttcgattgtctctttgatcgcttcgctagtcatctatttccgcacctccgacccagagccagagctggatgaaaacggcaatgctgctgagcccattaagttcagcttcaagtccatcattaaccctaaagtcttgccgattggcctcttcatgctgctggtagcctttgcctactccggcgtgatcgcacatatcaacgcttttgctgaaaaccgcgacgttgttactggcgcaggcctattcttttccgcttacgccatctccatgttcgtgatgcgctcctaccttggtaaattgcaagaccgccggggcgataacagcgttatctactttggtctcgtattctttgttatctcatttatcgtgctctcgctttctaccgccaactggcatgtcgttgtcgctggcgtgctagcaggtctgggctacggcaccttgatgccagctgctcaagcagtatctgttggtgttgtcgacaagagcgagttcggctcagcattttccaccttgttccttttcgttgacctcggcttcggcttcggcccagtcatccttggtgcagtggtttccgcgattggctacggttcgatgtatgcagtgctcgtcggcgtcggcgttattgctggcatctactacctgttcacccacgcacgcaccgagcgcgcaaagcacggcgtagtcaagcatgtagaaaccatggttctggctcaataa

SEQ ID NO: 59 - protein, 413 aa, synthetic construct
  source 1..413: note = C. st I259F AA
MHTTEEVKLFTPTFIMGWVANFLQFLVFYFLITTMALYATKEFSASETEAGFAASAIVIGAVFSRLVSGYIIDRFGRRKIVVVSVIATTIACALYIPIDSLGLLYADRFFHGVAYAFACTAIMAMVQELIPSARRSEGTGYLALGTTVSAAIGPALALFLLGSFNYEVLFVVVLGISIVSLIASLVIYFRTSDPEPELDENGNAAEPIKFSFKSIINPKVLPIGLFMLLVAFAYSGVIAHINAFAENRDVVTGAGLFFFAYAISMFVMRSYLGKLQDRRGDNSVIYFGLVFFVISFIVLSLSTANWHVVVAGVLAGLGYGTLMPAAQAVSVGVVDKSEFGSAFSTLFLFVDLGFGFGPVILGAVVSAIGYGSMYAVLVGVGVIAGIYYLFTHARTERAKHGVVKHVETMVLAQ

SEQ ID NO: 60 - DNA, 1242 bp, synthetic construct
  source 1..1242: mol_type = other DNA; note = C. st I259F NT
gtgcacacaaccgaagaggtcaaactctttacgccgacgtttatcatggggtgggtcgccaacttcctgcagttcttggtgttctacttcctcatcaccacgatggcgctctacgcaaccaaggaattcagcgcatcggaaaccgaagcaggctttgccgccagtgcgattgttatcggtgcggtcttttcccgtttggtttccggatacattattgaccgcttcggtcgccgcaaaattgtggtggtctccgtcatcgcgaccactattgcgtgcgcgctatatatcccgatcgattctttggggctgctctacgctgaccgcttcttccacggtgtagcttatgcctttgcgtgcaccgcgattatggcgatggtccaggaactcattccttctgcacgccgctccgaaggcactggctacctggctttgggtaccaccgtttcggctgctatcggaccagcgctagcgctatttttgctgggttctttcaactacgaagtcctcttcgttgtcgtcctcggcatttcgattgtctctttgatcgcttcgctagtcatctatttccgcacctccgacccagagccagagctggatgaaaacggcaatgctgctgagcccattaagttcagcttcaagtccatcattaaccctaaagtcttgccgattggcctcttcatgctgctggtagcctttgcctactccggcgtgatcgcacatatcaacgcttttgctgaaaaccgcgacgttgttactggcgcaggcctattctttttcgcttacgccatctccatgttcgtgatgcgctcctaccttggtaaattgcaagaccgccggggcgataacagcgttatctactttggtctcgtattctttgttatctcatttatcgtgctctcgctttctaccgccaactggcatgtcgttgtcgctggcgtgctagcaggtctgggctacggcaccttgatgccagctgctcaagcagtatctgttggtgttgtcgacaagagcgagttcggctcagcattttccaccttgttccttttcgttgacctcggcttcggcttcggcccagtcatccttggtgcagtggtttccgcgattggctacggttcgatgtatgcagtgctcgtcggcgtcggcgttattgctggcatctactacctgttcacccacgcacgcaccgagcgcgcaaagcacggcgtagtcaagcatgtagaaaccatggttctggctcaataa

SEQ ID NO: 61 - protein, 413 aa, synthetic construct
  source 1..413: note = C. st I259Y AA
MHTTEEVKLFTPTFIMGWVANFLQFLVFYFLITTMALYATKEFSASETEAGFAASAIVIGAVFSRLVSGYIIDRFGRRKIVVVSVIATTIACALYIPIDSLGLLYADRFFHGVAYAFACTAIMAMVQELIPSARRSEGTGYLALGTTVSAAIGPALALFLLGSFNYEVLFVVVLGISIVSLIASLVIYFRTSDPEPELDENGNAAEPIKFSFKSIINPKVLPIGLFMLLVAFAYSGVIAHINAFAENRDVVTGAGLFFYAYAISMFVMRSYLGKLQDRRGDNSVIYFGLVFFVISFIVLSLSTANWHVVVAGVLAGLGYGTLMPAAQAVSVGVVDKSEFGSAFSTLFLFVDLGFGFGPVILGAVVSAIGYGSMYAVLVGVGVIAGIYYLFTHARTERAKHGVVKHVETMVLAQ

SEQ ID NO: 62 - DNA, 1242 bp, synthetic construct
  source 1..1242: mol_type = other DNA; note = C. st I259Y NT
gtgcacacaaccgaagaggtcaaactctttacgccgacgtttatcatggggtgggtcgccaacttcctgcagttcttggtgttctacttcctcatcaccacgatggcgctctacgcaaccaaggaattcagcgcatcggaaaccgaagcaggctttgccgccagtgcgattgttatcggtgcggtcttttcccgtttggtttccggatacattattgaccgcttcggtcgccgcaaaattgtggtggtctccgtcatcgcgaccactattgcgtgcgcgctatatatcccgatcgattctttggggctgctctacgctgaccgcttcttccacggtgtagcttatgcctttgcgtgcaccgcgattatggcgatggtccaggaactcattccttctgcacgccgctccgaaggcactggctacctggctttgggtaccaccgtttcggctgctatcggaccagcgctagcgctatttttgctgggttctttcaactacgaagtcctcttcgttgtcgtcctcggcatttcgattgtctctttgatcgcttcgctagtcatctatttccgcacctccgacccagagccagagctggatgaaaacggcaatgctgctgagcccattaagttcagcttcaagtccatcattaaccctaaagtcttgccgattggcctcttcatgctgctggtagcctttgcctactccggcgtgatcgcacatatcaacgcttttgctgaaaaccgcgacgttgttactggcgcaggcctattcttttacgcttacgccatctccatgttcgtgatgcgctcctaccttggtaaattgcaagaccgccggggcgataacagcgttatctactttggtctcgtattctttgttatctcatttatcgtgctctcgctttctaccgccaactggcatgtcgttgtcgctggcgtgctagcaggtctgggctacggcaccttgatgccagctgctcaagcagtatctgttggtgttgtcgacaagagcgagttcggctcagcattttccaccttgttccttttcgttgacctcggcttcggcttcggcccagtcatccttggtgcagtggtttccgcgattggctacggttcgatgtatgcagtgctcgtcggcgtcggcgttattgctggcatctactacctgttcacccacgcacgcaccgagcgcgcaaagcacggcgtagtcaagcatgtagaaaccatggttctggctcaataa

SEQ ID NO: 63 - protein, 413 aa, synthetic construct
  source 1..413: note = C. st I259C AA
MHTTEEVKLFTPTFIMGWVANFLQFLVFYFLITTMALYATKEFSASETEAGFAASAIVIGAVFSRLVSGYIIDRFGRRKIVVVSVIATTIACALYIPIDSLGLLYADRFFHGVAYAFACTAIMAMVQELIPSARRSEGTGYLALGTTVSAAIGPALALFLLGSFNYEVLFVVVLGISIVSLIASLVIYFRTSDPEPELDENGNAAEPIKFSFKSIINPKVLPIGLFMLLVAFAYSGVIAHINAFAENRDVVTGAGLFFCAYAISMFVMRSYLGKLQDRRGDNSVIYFGLVFFVISFIVLSLSTANWHVVVAGVLAGLGYGTLMPAAQAVSVGVVDKSEFGSAFSTLFLFVDLGFGFGPVILGAVVSAIGYGSMYAVLVGVGVIAGIYYLFTHARTERAKHGVVKHVETMVLAQ

SEQ ID NO: 64 - DNA, 1242 bp, synthetic construct
  source 1..1242: mol_type = other DNA; note = C. st I259C NT
gtgcacacaaccgaagaggtcaaactctttacgccgacgtttatcatggggtgggtcgccaacttcctgcagttcttggtgttctacttcctcatcaccacgatggcgctctacgcaaccaaggaattcagcgcatcggaaaccgaagcaggctttgccgccagtgcgattgttatcggtgcggtcttttcccgtttggtttccggatacattattgaccgcttcggtcgccgcaaaattgtggtggtctccgtcatcgcgaccactattgcgtgcgcgctatatatcccgatcgattctttggggctgctctacgctgaccgcttcttccacggtgtagcttatgcctttgcgtgcaccgcgattatggcgatggtccaggaactcattccttctgcacgccgctccgaaggcactggctacctggctttgggtaccaccgtttcggctgctatcggaccagcgctagcgctatttttgctgggttctttcaactacgaagtcctcttcgttgtcgtcctcggcatttcgattgtctctttgatcgcttcgctagtcatctatttccgcacctccgacccagagccagagctggatgaaaacggcaatgctgctgagcccattaagttcagcttcaagtccatcattaaccctaaagtcttgccgattggcctcttcatgctgctggtagcctttgcctactccggcgtgatcgcacatatcaacgcttttgctgaaaaccgcgacgttgttactggcgcaggcctattcttttgcgcttacgccatctccatgttcgtgatgcgctcctaccttggtaaattgcaagaccgccggggcgataacagcgttatctactttggtctcgtattctttgttatctcatttatcgtgctctcgctttctaccgccaactggcatgtcgttgtcgctggcgtgctagcaggtctgggctacggcaccttgatgccagctgctcaagcagtatctgttggtgttgtcgacaagagcgagttcggctcagcattttccaccttgttccttttcgttgacctcggcttcggcttcggcccagtcatccttggtgcagtggtttccgcgattggctacggttcgatgtatgcagtgctcgtcggcgtcggcgttattgctggcatctactacctgttcacccacgcacgcaccgagcgcgcaaagcacggcgtagtcaagcatgtagaaaccatggttctggctcaataa

SEQ ID NO: 65 - protein, 413 aa, synthetic construct
  source 1..413: note = C. st I259L AA
MHTTEEVKLFTPTFIMGWVANFLQFLVFYFLITTMALYATKEFSASETEAGFAASAIVIGAVFSRLVSGYIIDRFGRRKIVVVSVIATTIACALYIPIDSLGLLYADRFFHGVAYAFACTAIMAMVQELIPSARRSEGTGYLALGTTVSAAIGPALALFLLGSFNYEVLFVVVLGISIVSLIASLVIYFRTSDPEPELDENGNAAEPIKFSFKSIINPKVLPIGLFMLLVAFAYSGVIAHINAFAENRDVVTGAGLFFLAYAISMFVMRSYLGKLQDRRGDNSVIYFGLVFFVISFIVLSLSTANWHVVVAGVLAGLGYGTLMPAAQAVSVGVVDKSEFGSAFSTLFLFVDLGFGFGPVILGAVVSAIGYGSMYAVLVGVGVIAGIYYLFTHARTERAKHGVVKHVETMVLAQ

SEQ ID NO: 66 - DNA, 1242 bp, synthetic construct
  source 1..1242: mol_type = other DNA; note = C. st I259L NT
gtgcacacaaccgaagaggtcaaactctttacgccgacgtttatcatggggtgggtcgccaacttcctgcagttcttggtgttctacttcctcatcaccacgatggcgctctacgcaaccaaggaattcagcgcatcggaaaccgaagcaggctttgccgccagtgcgattgttatcggtgcggtcttttcccgtttggtttccggatacattattgaccgcttcggtcgccgcaaaattgtggtggtctccgtcatcgcgaccactattgcgtgcgcgctatatatcccgatcgattctttggggctgctctacgctgaccgcttcttccacggtgtagcttatgcctttgcgtgcaccgcgattatggcgatggtccaggaactcattccttctgcacgccgctccgaaggcactggctacctggctttgggtaccaccgtttcggctgctatcggaccagcgctagcgctatttttgctgggttctttcaactacgaagtcctcttcgttgtcgtcctcggcatttcgattgtctctttgatcgcttcgctagtcatctatttccgcacctccgacccagagccagagctggatgaaaacggcaatgctgctgagcccattaagttcagcttcaagtccatcattaaccctaaagtcttgccgattggcctcttcatgctgctggtagcctttgcctactccggcgtgatcgcacatatcaacgcttttgctgaaaaccgcgacgttgttactggcgcaggcctattctttctggcttacgccatctccatgttcgtgatgcgctcctaccttggtaaattgcaagaccgccggggcgataacagcgttatctactttggtctcgtattctttgttatctcatttatcgtgctctcgctttctaccgccaactggcatgtcgttgtcgctggcgtgctagcaggtctgggctacggcaccttgatgccagctgctcaagcagtatctgttggtgttgtcgacaagagcgagttcggctcagcattttccaccttgttccttttcgttgacctcggcttcggcttcggcccagtcatccttggtgcagtggtttccgcgattggctacggttcgatgtatgcagtgctcgtcggcgtcggcgttattgctggcatctactacctgttcacccacgcacgcaccgagcgcgcaaagcacggcgtagtcaagcatgtagaaaccatggttctggctcaataa

SEQ ID NO: 67 - protein, 413 aa, synthetic construct
  source 1..413: note = C. st I259H AA
MHTTEEVKLFTPTFIMGWVANFLQFLVFYFLITTMALYATKEFSASETEAGFAASAIVIGAVFSRLVSGYIIDRFGRRKIVVVSVIATTIACALYIPIDSLGLLYADRFFHGVAYAFACTAIMAMVQELIPSARRSEGTGYLALGTTVSAAIGPALALFLLGSFNYEVLFVVVLGISIVSLIASLVIYFRTSDPEPELDENGNAAEPIKFSFKSIINPKVLPIGLFMLLVAFAYSGVIAHINAFAENRDVVTGAGLFFHAYAISMFVMRSYLGKLQDRRGDNSVIYFGLVFFVISFIVLSLSTANWHVVVAGVLAGLGYGTLMPAAQAVSVGVVDKSEFGSAFSTLFLFVDLGFGFGPVILGAVVSAIGYGSMYAVLVGVGVIAGIYYLFTHARTERAKHGVVKHVETMVLAQ

SEQ ID NO: 68 - DNA, 1242 bp, synthetic construct
  source 1..1242: mol_type = other DNA; note = C. st I259H NT
gtgcacacaaccgaagaggtcaaactctttacgccgacgtttatcatggggtgggtcgccaacttcctgcagttcttggtgttctacttcctcatcaccacgatggcgctctacgcaaccaaggaattcagcgcatcggaaaccgaagcaggctttgccgccagtgcgattgttatcggtgcggtcttttcccgtttggtttccggatacattattgaccgcttcggtcgccgcaaaattgtggtggtctccgtcatcgcgaccactattgcgtgcgcgctatatatcccgatcgattctttggggctgctctacgctgaccgcttcttccacggtgtagcttatgcctttgcgtgcaccgcgattatggcgatggtccaggaactcattccttctgcacgccgctccgaaggcactggctacctggctttgggtaccaccgtttcggctgctatcggaccagcgctagcgctatttttgctgggttctttcaactacgaagtcctcttcgttgtcgtcctcggcatttcgattgtctctttgatcgcttcgctagtcatctatttccgcacctccgacccagagccagagctggatgaaaacggcaatgctgctgagcccattaagttcagcttcaagtccatcattaaccctaaagtcttgccgattggcctcttcatgctgctggtagcctttgcctactccggcgtgatcgcacatatcaacgcttttgctgaaaaccgcgacgttgttactggcgcaggcctattctttcacgcttacgccatctccatgttcgtgatgcgctcctaccttggtaaattgcaagaccgccggggcgataacagcgttatctactttggtctcgtattctttgttatctcatttatcgtgctctcgctttctaccgccaactggcatgtcgttgtcgctggcgtgctagcaggtctgggctacggcaccttgatgccagctgctcaagcagtatctgttggtgttgtcgacaagagcgagttcggctcagcattttccaccttgttccttttcgttgacctcggcttcggcttcggcccagtcatccttggtgcagtggtttccgcgattggctacggttcgatgtatgcagtgctcgtcggcgtcggcgttattgctggcatctactacctgttcacccacgcacgcaccgagcgcgcaaagcacggcgtagtcaagcatgtagaaaccatggttctggctcaataa

SEQ ID NO: 69 - protein, 413 aa, synthetic construct
  source 1..413: note = C. st I259V AA
MHTTEEVKLFTPTFIMGWVANFLQFLVFYFLITTMALYATKEFSASETEAGFAASAIVIGAVFSRLVSGYIIDRFGRRKIVVVSVIATTIACALYIPIDSLGLLYADRFFHGVAYAFACTAIMAMVQELIPSARRSEGTGYLALGTTVSAAIGPALALFLLGSFNYEVLFVVVLGISIVSLIASLVIYFRTSDPEPELDENGNAAEPIKFSFKSIINPKVLPIGLFMLLVAFAYSGVIAHINAFAENRDVVTGAGLFFVAYAISMFVMRSYLGKLQDRRGDNSVIYFGLVFFVISFIVLSLSTANWHVVVAGVLAGLGYGTLMPAAQAVSVGVVDKSEFGSAFSTLFLFVDLGFGFGPVILGAVVSAIGYGSMYAVLVGVGVIAGIYYLFTHARTERAKHGVVKHVETMVLAQ

SEQ ID NO: 70 - DNA, 1242 bp, synthetic construct
  source 1..1242: mol_type = other DNA; note = C. st I259V NT
gtgcacacaaccgaagaggtcaaactctttacgccgacgtttatcatggggtgggtcgccaacttcctgcagttcttggtgttctacttcctcatcaccacgatggcgctctacgcaaccaaggaattcagcgcatcggaaaccgaagcaggctttgccgccagtgcgattgttatcggtgcggtcttttcccgtttggtttccggatacattattgaccgcttcggtcgccgcaaaattgtggtggtctccgtcatcgcgaccactattgcgtgcgcgctatatatcccgatcgattctttggggctgctctacgctgaccgcttcttccacggtgtagcttatgcctttgcgtgcaccgcgattatggcgatggtccaggaactcattccttctgcacgccgctccgaaggcactggctacctggctttgggtaccaccgtttcggctgctatcggaccagcgctagcgctatttttgctgggttctttcaactacgaagtcctcttcgttgtcgtcctcggcatttcgattgtctctttgatcgcttcgctagtcatctatttccgcacctccgacccagagccagagctggatgaaaacggcaatgctgctgagcccattaagttcagcttcaagtccatcattaaccctaaagtcttgccgattggcctcttcatgctgctggtagcctttgcctactccggcgtgatcgcacatatcaacgcttttgctgaaaaccgcgacgttgttactggcgcaggcctattctttgtggcttacgccatctccatgttcgtgatgcgctcctaccttggtaaattgcaagaccgccggggcgataacagcgttatctactttggtctcgtattctttgttatctcatttatcgtgctctcgctttctaccgccaactggcatgtcgttgtcgctggcgtgctagcaggtctgggctacggcaccttgatgccagctgctcaagcagtatctgttggtgttgtcgacaagagcgagttcggctcagcattttccaccttgttccttttcgttgacctcggcttcggcttcggcccagtcatccttggtgcagtggtttccgcgattggctacggttcgatgtatgcagtgctcgtcggcgtcggcgttattgctggcatctactacctgttcacccacgcacgcaccgagcgcgcaaagcacggcgtagtcaagcatgtagaaaccatggttctggctcaataa

SEQ ID NO: 71 - protein, 413 aa, synthetic construct
  source 1..413: note = C. st I259D AA
MHTTEEVKLFTPTFIMGWVANFLQFLVFYFLITTMALYATKEFSASETEAGFAASAIVIGAVFSRLVSGYIIDRFGRRKIVVVSVIATTIACALYIPIDSLGLLYADRFFHGVAYAFACTAIMAMVQELIPSARRSEGTGYLALGTTVSAAIGPALALFLLGSFNYEVLFVVVLGISIVSLIASLVIYFRTSDPEPELDENGNAAEPIKFSFKSIINPKVLPIGLFMLLVAFAYSGVIAHINAFAENRDVVTGAGLFFDAYAISMFVMRSYLGKLQDRRGDNSVIYFGLVFFVISFIVLSLSTANWHVVVAGVLAGLGYGTLMPAAQAVSVGVVDKSEFGSAFSTLFLFVDLGFGFGPVILGAVVSAIGYGSMYAVLVGVGVIAGIYYLFTHARTERAKHGVVKHVETMVLAQ

SEQ ID NO: 72 - DNA, 1242 bp, synthetic construct
  source 1..1242: mol_type = other DNA; note = C. st I259D NT
gtgcacacaaccgaagaggtcaaactctttacgccgacgtttatcatggggtgggtcgccaacttcctgcagttcttggtgttctacttcctcatcaccacgatggcgctctacgcaaccaaggaattcagcgcatcggaaaccgaagcaggctttgccgccagtgcgattgttatcggtgcggtcttttcccgtttggtttccggatacattattgaccgcttcggtcgccgcaaaattgtggtggtctccgtcatcgcgaccactattgcgtgcgcgctatatatcccgatcgattctttggggctgctctacgctgaccgcttcttccacggtgtagcttatgcctttgcgtgcaccgcgattatggcgatggtccaggaactcattccttctgcacgccgctccgaaggcactggctacctggctttgggtaccaccgtttcggctgctatcggaccagcgctagcgctatttttgctgggttctttcaactacgaagtcctcttcgttgtcgtcctcggcatttcgattgtctctttgatcgcttcgctagtcatctatttccgcacctccgacccagagccagagctggatgaaaacggcaatgctgctgagcccattaagttcagcttcaagtccatcattaaccctaaagtcttgccgattggcctcttcatgctgctggtagcctttgcctactccggcgtgatcgcacatatcaacgcttttgctgaaaaccgcgacgttgttactggcgcaggcctattctttgatgcttacgccatctccatgttcgtgatgcgctcctaccttggtaaattgcaagaccgccggggcgataacagcgttatctactttggtctcgtattctttgttatctcatttatcgtgctctcgctttctaccgccaactggcatgtcgttgtcgctggcgtgctagcaggtctgggctacggcaccttgatgccagctgctcaagcagtatctgttggtgttgtcgacaagagcgagttcggctcagcattttccaccttgttccttttcgttgacctcggcttcggcttcggcccagtcatccttggtgcagtggtttccgcgattggctacggttcgatgtatgcagtgctcgtcggcgtcggcgttattgctggcatctactacctgttcacccacgcacgcaccgagcgcgcaaagcacggcgtagtcaagcatgtagaaaccatggttctggctcaataa

SEQ ID NO: 73 - protein, 413 aa, synthetic construct
  source 1..413: note = C. st I259G AA
MHTTEEVKLFTPTFIMGWVANFLQFLVFYFLITTMALYATKEFSASETEAGFAASAIVIGAVFSRLVSGYIIDRFGRRKIVVVSVIATTIACALYIPIDSLGLLYADRFFHGVAYAFACTAIMAMVQELIPSARRSEGTGYLALGTTVSAAIGPALALFLLGSFNYEVLFVVVLGISIVSLIASLVIYFRTSDPEPELDENGNAAEPIKFSFKSIINPKVLPIGLFMLLVAFAYSGVIAHINAFAENRDVVTGAGLFFGAYAISMFVMRSYLGKLQDRRGDNSVIYFGLVFFVISFIVLSLSTANWHVVVAGVLAGLGYGTLMPAAQAVSVGVVDKSEFGSAFSTLFLFVDLGFGFGPVILGAVVSAIGYGSMYAVLVGVGVIAGIYYLFTHARTERAKHGVVKHVETMVLAQ

SEQ ID NO: 74 - DNA, 1242 bp, synthetic construct
  source 1..1242: mol_type = other DNA; note = C. st I259G NT
gtgcacacaaccgaagaggtcaaactctttacgccgacgtttatcatggggtgggtcgccaacttcctgcagttcttggtgttctacttcctcatcaccacgatggcgctctacgcaaccaaggaattcagcgcatcggaaaccgaagcaggctttgccgccagtgcgattgttatcggtgcggtcttttcccgtttggtttccggatacattattgaccgcttcggtcgccgcaaaattgtggtggtctccgtcatcgcgaccactattgcgtgcgcgctatatatcccgatcgattctttggggctgctctacgctgaccgcttcttccacggtgtagcttatgcctttgcgtgcaccgcgattatggcgatggtccaggaactcattccttctgcacgccgctccgaaggcactggctacctggctttgggtaccaccgtttcggctgctatcggaccagcgctagcgctatttttgctgggttctttcaactacgaagtcctcttcgttgtcgtcctcggcatttcgattgtctctttgatcgcttcgctagtcatctatttccgcacctccgacccagagccagagctggatgaaaacggcaatgctgctgagcccattaagttcagcttcaagtccatcattaaccctaaagtcttgccgattggcctcttcatgctgctggtagcctttgcctactccggcgtgatcgcacatatcaacgcttttgctgaaaaccgcgacgttgttactggcgcaggcctattctttggcgcttacgccatctccatgttcgtgatgcgctcctaccttggtaaattgcaagaccgccggggcgataacagcgttatctactttggtctcgtattctttgttatctcatttatcgtgctctcgctttctaccgccaactggcatgtcgttgtcgctggcgtgctagcaggtctgggctacggcaccttgatgccagctgctcaagcagtatctgttggtgttgtcgacaagagcgagttcggctcagcattttccaccttgttccttttcgttgacctcggcttcggcttcggcccagtcatccttggtgcagtggtttccgcgattggctacggttcgatgtatgcagtgctcgtcggcgtcggcgttattgctggcatctactacctgttcacccacgcacgcaccgagcgcgcaaagcacggcgtagtcaagcatgtagaaaccatggttctggctcaataa

SEQ ID NO: 75 - protein, 413 aa, synthetic construct
  source 1..413: note = C. st I259P AA
MHTTEEVKLFTPTFIMGWVANFLQFLVFYFLITTMALYATKEFSASETEAGFAASAIVIGAVFSRLVSGYIIDRFGRRKIVVVSVIATTIACALYIPIDSLGLLYADRFFHGVAYAFACTAIMAMVQELIPSARRSEGTGYLALGTTVSAAIGPALALFLLGSFNYEVLFVVVLGISIVSLIASLVIYFRTSDPEPELDENGNAAEPIKFSFKSIINPKVLPIGLFMLLVAFAYSGVIAHINAFAENRDVVTGAGLFFPAYAISMFVMRSYLGKLQDRRGDNSVIYFGLVFFVISFIVLSLSTANWHVVVAGVLAGLGYGTLMPAAQAVSVGVVDKSEFGSAFSTLFLFVDLGFGFGPVILGAVVSAIGYGSMYAVLVGVGVIAGIYYLFTHARTERAKHGVVKHVETMVLAQ

SEQ ID NO: 76 - DNA, 1242 bp, synthetic construct
  source 1..1242: mol_type = other DNA; note = C. st I259P NT
gtgcacacaaccgaagaggtcaaactctttacgccgacgtttatcatggggtgggtcgccaacttcctgcagttcttggtgttctacttcctcatcaccacgatggcgctctacgcaaccaaggaattcagcgcatcggaaaccgaagcaggctttgccgccagtgcgattgttatcggtgcggtcttttcccgtttggtttccggatacattattgaccgcttcggtcgccgcaaaattgtggtggtctccgtcatcgcgaccactattgcgtgcgcgctatatatcccgatcgattctttggggctgctctacgctgaccgcttcttccacggtgtagcttatgcctttgcgtgcaccgcgattatggcgatggtccaggaactcattccttctgcacgccgctccgaaggcactggctacctggctttgggtaccaccgtttcggctgctatcggaccagcgctagcgctatttttgctgggttctttcaactacgaagtcctcttcgttgtcgtcctcggcatttcgattgtctctttgatcgcttcgctagtcatctatttccgcacctccgacccagagccagagctggatgaaaacggcaatgctgctgagcccattaagttcagcttcaagtccatcattaaccctaaagtcttgccgattggcctcttcatgctgctggtagcctttgcctactccggcgtgatcgcacatatcaacgcttttgctgaaaaccgcgacgttgttactggcgcaggcctattctttccagcttacgccatctccatgttcgtgatgcgctcctaccttggtaaattgcaagaccgccggggcgataacagcgttatctactttggtctcgtattctttgttatctcatttatcgtgctctcgctttctaccgccaactggcatgtcgttgtcgctggcgtgctagcaggtctgggctacggcaccttgatgccagctgctcaagcagtatctgttggtgttgtcgacaagagcgagttcggctcagcattttccaccttgttccttttcgttgacctcggcttcggcttcggcccagtcatccttggtgcagtggtttccgcgattggctacggttcgatgtatgcagtgctcgtcggcgtcggcgttattgctggcatctactacctgttcacccacgcacgcaccgagcgcgcaaagcacggcgtagtcaagcatgtagaaaccatggttctggctcaataa

SEQ ID NO: 77 - protein, 413 aa, synthetic construct
  source 1..413: note = C. st I259A AA
MHTTEEVKLFTPTFIMGWVANFLQFLVFYFLITTMALYATKEFSASETEAGFAASAIVIGAVFSRLVSGYIIDRFGRRKIVVVSVIATTIACALYIPIDSLGLLYADRFFHGVAYAFACTAIMAMVQELIPSARRSEGTGYLALGTTVSAAIGPALALFLLGSFNYEVLFVVVLGISIVSLIASLVIYFRTSDPEPELDENGNAAEPIKFSFKSIINPKVLPIGLFMLLVAFAYSGVIAHINAFAENRDVVTGAGLFFAAYAISMFVMRSYLGKLQDRRGDNSVIYFGLVFFVISFIVLSLSTANWHVVVAGVLAGLGYGTLMPAAQAVSVGVVDKSEFGSAFSTLFLFVDLGFGFGPVILGAVVSAIGYGSMYAVLVGVGVIAGIYYLFTHARTERAKHGVVKHVETMVLAQ

SEQ ID NO: 78 - DNA, 1242 bp, synthetic construct
  source 1..1242: mol_type = other DNA; note = C. st I259A NT
gtgcacacaaccgaagaggtcaaactctttacgccgacgtttatcatggggtgggtcgccaacttcctgcagttcttggtgttctacttcctcatcaccacgatggcgctctacgcaaccaaggaattcagcgcatcggaaaccgaagcaggctttgccgccagtgcgattgttatcggtgcggtcttttcccgtttggtttccggatacattattgaccgcttcggtcgccgcaaaattgtggtggtctccgtcatcgcgaccactattgcgtgcgcgctatatatcccgatcgattctttggggctgctctacgctgaccgcttcttccacggtgtagcttatgcctttgcgtgcaccgcgattatggcgatggtccaggaactcattccttctgcacgccgctccgaaggcactggctacctggctttgggtaccaccgtttcggctgctatcggaccagcgctagcgctatttttgctgggttctttcaactacgaagtcctcttcgttgtcgtcctcggcatttcgattgtctctttgatcgcttcgctagtcatctatttccgcacctccgacccagagccagagctggatgaaaacggcaatgctgctgagcccattaagttcagcttcaagtccatcattaaccctaaagtcttgccgattggcctcttcatgctgctggtagcctttgcctactccggcgtgatcgcacatatcaacgcttttgctgaaaaccgcgacgttgttactggcgcaggcctattctttgcagcttacgccatctccatgttcgtgatgcgctcctaccttggtaaattgcaagaccgccggggcgataacagcgttatctactttggtctcgtattctttgttatctcatttatcgtgctctcgctttctaccgccaactggcatgtcgttgtcgctggcgtgctagcaggtctgggctacggcaccttgatgccagctgctcaagcagtatctgttggtgttgtcgacaagagcgagttcggctcagcattttccaccttgttccttttcgttgacctcggcttcggcttcggcccagtcatccttggtgcagtggtttccgcgattggctacggttcgatgtatgcagtgctcgtcggcgtcggcgttattgctggcatctactacctgttcacccacgcacgcaccgagcgcgcaaagcacggcgtagtcaagcatgtagaaaccatggttctggctcaataa

SEQ ID NO: 79 - protein, 413 aa, synthetic construct
  source 1..413: note = C. st I259E AA
MHTTEEVKLFTPTFIMGWVANFLQFLVFYFLITTMALYATKEFSASETEAGFAASAIVIGAVFSRLVSGYIIDRFGRRKIVVVSVIATTIACALYIPIDSLGLLYADRFFHGVAYAFACTAIMAMVQELIPSARRSEGTGYLALGTTVSAAIGPALALFLLGSFNYEVLFVVVLGISIVSLIASLVIYFRTSDPEPELDENGNAAEPIKFSFKSIINPKVLPIGLFMLLVAFAYSGVIAHINAFAENRDVVTGAGLFFEAYAISMFVMRSYLGKLQDRRGDNSVIYFGLVFFVISFIVLSLSTANWHVVVAGVLAGLGYGTLMPAAQAVSVGVVDKSEFGSAFSTLFLFVDLGFGFGPVILGAVVSAIGYGSMYAVLVGVGVIAGIYYLFTHARTERAKHGVVKHVETMVLAQ

SEQ ID NO: 80 - DNA, 1242 bp, synthetic construct
  source 1..1242: mol_type = other DNA; note = C. st I259E NT
gtgcacacaaccgaagaggtcaaactctttacgccgacgtttatcatggggtgggtcgccaacttcctgcagttcttggtgttctacttcctcatcaccacgatggcgctctacgcaaccaaggaattcagcgcatcggaaaccgaagcaggctttgccgccagtgcgattgttatcggtgcggtcttttcccgtttggtttccggatacattattgaccgcttcggtcgccgcaaaattgtggtggtctccgtcatcgcgaccactattgcgtgcgcgctatatatcccgatcgattctttggggctgctctacgctgaccgcttcttccacggtgtagcttatgcctttgcgtgcaccgcgattatggcgatggtccaggaactcattccttctgcacgccgctccgaaggcactggctacctggctttgggtaccaccgtttcggctgctatcggaccagcgctagcgctatttttgctgggttctttcaactacgaagtcctcttcgttgtcgtcctcggcatttcgattgtctctttgatcgcttcgctagtcatctatttccgcacctccgacccagagccagagctggatgaaaacggcaatgctgctgagcccattaagttcagcttcaagtccatcattaaccctaaagtcttgccgattggcctcttcatgctgctggtagcctttgcctactccggcgtgatcgcacatatcaacgcttttgctgaaaaccgcgacgttgttactggcgcaggcctattctttgaagcttacgccatctccatgttcgtgatgcgctcctaccttggtaaattgcaagaccgccggggcgataacagcgttatctactttggtctcgtattctttgttatctcatttatcgtgctctcgctttctaccgccaactggcatgtcgttgtcgctggcgtgctagcaggtctgggctacggcaccttgatgccagctgctcaagcagtatctgttggtgttgtcgacaagagcgagttcggctcagcattttccaccttgttccttttcgttgacctcggcttcggcttcggcccagtcatccttggtgcagtggtttccgcgattggctacggttcgatgtatgcagtgctcgtcggcgtcggcgttattgctggcatctactacctgttcacccacgcacgcaccgagcgcgcaaagcacggcgtagtcaagcatgtagaaaccatggttctggctcaataa

SEQ ID NO: 81 - protein, 413 aa, synthetic construct
  source 1..413: note = C. st I259M AA
MHTTEEVKLFTPTFIMGWVANFLQFLVFYFLITTMALYATKEFSASETEAGFAASAIVIGAVFSRLVSGYIIDRFGRRKIVVVSVIATTIACALYIPIDSLGLLYADRFFHGVAYAFACTAIMAMVQELIPSARRSEGTGYLALGTTVSAAIGPALALFLLGSFNYEVLFVVVLGISIVSLIASLVIYFRTSDPEPELDENGNAAEPIKFSFKSIINPKVLPIGLFMLLVAFAYSGVIAHINAFAENRDVVTGAGLFFMAYAISMFVMRSYLGKLQDRRGDNSVIYFGLVFFVISFIVLSLSTANWHVVVAGVLAGLGYGTLMPAAQAVSVGVVDKSEFGSAFSTLFLFVDLGFGFGPVILGAVVSAIGYGSMYAVLVGVGVIAGIYYLFTHARTERAKHGVVKHVETMVLAQ

SEQ ID NO: 82 - DNA, 1242 bp, synthetic construct
  source 1..1242: mol_type = other DNA; note = C. st I259M NT
gtgcacacaaccgaagaggtcaaactctttacgccgacgtttatcatggggtgggtcgccaacttcctgcagttcttggtgttctacttcctcatcaccacgatggcgctctacgcaaccaaggaattcagcgcatcggaaaccgaagcaggctttgccgccagtgcgattgttatcggtgcggtcttttcccgtttggtttccggatacattattgaccgcttcggtcgccgcaaaattgtggtggtctccgtcatcgcgaccactattgcgtgcgcgctatatatcccgatcgattctttggggctgctctacgctgaccgcttcttccacggtgtagcttatgcctttgcgtgcaccgcgattatggcgatggtccaggaactcattccttctgcacgccgctccgaaggcactggctacctggctttgggtaccaccgtttcggctgctatcggaccagcgctagcgctatttttgctgggttctttcaactacgaagtcctcttcgttgtcgtcctcggcatttcgattgtctctttgatcgcttcgctagtcatctatttccgcacctccgacccagagccagagctggatgaaaacggcaatgctgctgagcccattaagttcagcttcaagtccatcattaaccctaaagtcttgccgattggcctcttcatgctgctggtagcctttgcctactccggcgtgatcgcacatatcaacgcttttgctgaaaaccgcgacgttgttactggcgcaggcctattctttatggcttacgccatctccatgttcgtgatgcgctcctaccttggtaaattgcaagaccgccggggcgataacagcgttatctactttggtctcgtattctttgttatctcatttatcgtgctctcgctttctaccgccaactggcatgtcgttgtcgctggcgtgctagcaggtctgggctacggcaccttgatgccagctgctcaagcagtatctgttggtgttgtcgacaagagcgagttcggctcagcattttccaccttgttccttttcgttgacctcggcttcggcttcggcccagtcatccttggtgcagtggtttccgcgattggctacggttcgatgtatgcagtgctcgtcggcgtcggcgttattgctggcatctactacctgttcacccacgcacgcaccgagcgcgcaaagcacggcgtagtcaagcatgtagaaaccatggttctggctcaataa

SEQ ID NO: 83 - protein, 413 aa, synthetic construct
  source 1..413: note = C. st I259W AA
MHTTEEVKLFTPTFIMGWVANFLQFLVFYFLITTMALYATKEFSASETEAGFAASAIVIGAVFSRLVSGYIIDRFGRRKIVVVSVIATTIACALYIPIDSLGLLYADRFFHGVAYAFACTAIMAMVQELIPSARRSEGTGYLALGTTVSAAIGPALALFLLGSFNYEVLFVVVLGISIVSLIASLVIYFRTSDPEPELDENGNAAEPIKFSFKSIINPKVLPIGLFMLLVAFAYSGVIAHINAFAENRDVVTGAGLFFWAYAISMFVMRSYLGKLQDRRGDNSVIYFGLVFFVISFIVLSLSTANWHVVVAGVLAGLGYGTLMPAAQAVSVGVVDKSEFGSAFSTLFLFVDLGFGFGPVILGAVVSAIGYGSMYAVLVGVGVIAGIYYLFTHARTERAKHGVVKHVETMVLAQ

SEQ ID NO: 84 - DNA, 1242 bp, synthetic construct
  source 1..1242: mol_type = other DNA; note = C. st I259W NT
gtgcacacaaccgaagaggtcaaactctttacgccgacgtttatcatggggtgggtcgccaacttcctgcagttcttggtgttctacttcctcatcaccacgatggcgctctacgcaaccaaggaattcagcgcatcggaaaccgaagcaggctttgccgccagtgcgattgttatcggtgcggtcttttcccgtttggtttccggatacattattgaccgcttcggtcgccgcaaaattgtggtggtctccgtcatcgcgaccactattgcgtgcgcgctatatatcccgatcgattctttggggctgctctacgctgaccgcttcttccacggtgtagcttatgcctttgcgtgcaccgcgattatggcgatggtccaggaactcattccttctgcacgccgctccgaaggcactggctacctggctttgggtaccaccgtttcggctgctatcggaccagcgctagcgctatttttgctgggttctttcaactacgaagtcctcttcgttgtcgtcctcggcatttcgattgtctctttgatcgcttcgctagtcatctatttccgcacctccgacccagagccagagctggatgaaaacggcaatgctgctgagcccattaagttcagcttcaagtccatcattaaccctaaagtcttgccgattggcctcttcatgctgctggtagcctttgcctactccggcgtgatcgcacatatcaacgcttttgctgaaaaccgcgacgttgttactggcgcaggcctattcttttgggcttacgccatctccatgttcgtgatgcgctcctaccttggtaaattgcaagaccgccggggcgataacagcgttatctactttggtctcgtattctttgttatctcatttatcgtgctctcgctttctaccgccaactggcatgtcgttgtcgctggcgtgctagcaggtctgggctacggcaccttgatgccagctgctcaagcagtatctgttggtgttgtcgacaagagcgagttcggctcagcattttccaccttgttccttttcgttgacctcggcttcggcttcggcccagtcatccttggtgcagtggtttccgcgattggctacggttcgatgtatgcagtgctcgtcggcgtcggcgttattgctggcatctactacctgttcacccacgcacgcaccgagcgcgcaaagcacggcgtagtcaagcatgtagaaaccatggttctggctcaataa

SEQ ID NO: 85 - protein, 413 aa, synthetic construct
  source 1..413: note = C. st I259Q AA
MHTTEEVKLFTPTFIMGWVANFLQFLVFYFLITTMALYATKEFSASETEAGFAASAIVIGAVFSRLVSGYIIDRFGRRKIVVVSVIATTIACALYIPIDSLGLLYADRFFHGVAYAFACTAIMAMVQELIPSARRSEGTGYLALGTTVSAAIGPALALFLLGSFNYEVLFVVVLGISIVSLIASLVIYFRTSDPEPELDENGNAAEPIKFSFKSIINPKVLPIGLFMLLVAFAYSGVIAHINAFAENRDVVTGAGLFFQAYAISMFVMRSYLGKLQDRRGDNSVIYFGLVFFVISFIVLSLSTANWHVVVAGVLAGLGYGTLMPAAQAVSVGVVDKSEFGSAFSTLFLFVDLGFGFGPVILGAVVSAIGYGSMYAVLVGVGVIAGIYYLFTHARTERAKHGVVKHVETMVLAQ

SEQ ID NO: 86 - DNA, 1242 bp, synthetic construct
  source 1..1242: mol_type = other DNA; note = C. st I259Q NT
gtgcacacaaccgaagaggtcaaactctttacgccgacgtttatcatggggtgggtcgccaacttcctgcagttcttggtgttctacttcctcatcaccacgatggcgctctacgcaaccaaggaattcagcgcatcggaaaccgaagcaggctttgccgccagtgcgattgttatcggtgcggtcttttcccgtttggtttccggatacattattgaccgcttcggtcgccgcaaaattgtggtggtctccgtcatcgcgaccactattgcgtgcgcgctatatatcccgatcgattctttggggctgctctacgctgaccgcttcttccacggtgtagcttatgcctttgcgtgcaccgcgattatggcgatggtccaggaactcattccttctgcacgccgctccgaaggcactggctacctggctttgggtaccaccgtttcggctgctatcggaccagcgctagcgctatttttgctgggttctttcaactacgaagtcctcttcgttgtcgtcctcggcatttcgattgtctctttgatcgcttcgctagtcatctatttccgcacctccgacccagagccagagctggatgaaaacggcaatgctgctgagcccattaagttcagcttcaagtccatcattaaccctaaagtcttgccgattggcctcttcatgctgctggtagcctttgcctactccggcgtgatcgcacatatcaacgcttttgctgaaaaccgcgacgttgttactggcgcaggcctattctttcaggcttacgccatctccatgttcgtgatgcgctcctaccttggtaaattgcaagaccgccggggcgataacagcgttatctactttggtctcgtattctttgttatctcatttatcgtgctctcgctttctaccgccaactggcatgtcgttgtcgctggcgtgctagcaggtctgggctacggcaccttgatgccagctgctcaagcagtatctgttggtgttgtcgacaagagcgagttcggctcagcattttccaccttgttccttttcgttgacctcggcttcggcttcggcccagtcatccttggtgcagtggtttccgcgattggctacggttcgatgtatgcagtgctcgtcggcgtcggcgttattgctggcatctactacctgttcacccacgcacgcaccgagcgcgcaaagcacggcgtagtcaagcatgtagaaaccatggttctggctcaataa

SEQ ID NO: 87 - protein, 413 aa, synthetic construct
  source 1..413: note = C. st I259K AA
MHTTEEVKLFTPTFIMGWVANFLQFLVFYFLITTMALYATKEFSASETEAGFAASAIVIGAVFSRLVSGYIIDRFGRRKIVVVSVIATTIACALYIPIDSLGLLYADRFFHGVAYAFACTAIMAMVQELIPSARRSEGTGYLALGTTVSAAIGPALALFLLGSFNYEVLFVVVLGISIVSLIASLVIYFRTSDPEPELDENGNAAEPIKFSFKSIINPKVLPIGLFMLLVAFAYSGVIAHINAFAENRDVVTGAGLFFKAYAISMFVMRSYLGKLQDRRGDNSVIYFGLVFFVISFIVLSLSTANWHVVVAGVLAGLGYGTLMPAAQAVSVGVVDKSEFGSAFSTLFLFVDLGFGFGPVILGAVVSAIGYGSMYAVLVGVGVIAGIYYLFTHARTERAKHGVVKHVETMVLAQ

SEQ ID NO: 88 - DNA, 1242 bp, synthetic construct
  source 1..1242: mol_type = other DNA; note = C. st I259K NT
gtgcacacaaccgaagaggtcaaactctttacgccgacgtttatcatggggtgggtcgccaacttcctgcagttcttggtgttctacttcctcatcaccacgatggcgctctacgcaaccaaggaattcagcgcatcggaaaccgaagcaggctttgccgccagtgcgattgttatcggtgcggtcttttcccgtttggtttccggatacattattgaccgcttcggtcgccgcaaaattgtggtggtctccgtcatcgcgaccactattgcgtgcgcgctatatatcccgatcgattctttggggctgctctacgctgaccgcttcttccacggtgtagcttatgcctttgcgtgcaccgcgattatggcgatggtccaggaactcattccttctgcacgccgctccgaaggcactggctacctggctttgggtaccaccgtttcggctgctatcggaccagcgctagcgctatttttgctgggttctttcaactacgaagtcctcttcgttgtcgtcctcggcatttcgattgtctctttgatcgcttcgctagtcatctatttccgcacctccgacccagagccagagctggatgaaaacggcaatgctgctgagcccattaagttcagcttcaagtccatcattaaccctaaagtcttgccgattggcctcttcatgctgctggtagcctttgcctactccggcgtgatcgcacatatcaacgcttttgctgaaaaccgcgacgttgttactggcgcaggcctattctttaaggcttacgccatctccatgttcgtgatgcgctcctaccttggtaaattgcaagaccgccggggcgataacagcgttatctactttggtctcgtattctttgttatctcatttatcgtgctctcgctttctaccgccaactggcatgtcgttgtcgctggcgtgctagcaggtctgggctacggcaccttgatgccagctgctcaagcagtatctgttggtgttgtcgacaagagcgagttcggctcagcattttccaccttgttccttttcgttgacctcggcttcggcttcggcccagtcatccttggtgcagtggtttccgcgattggctacggttcgatgtatgcagtgctcgtcggcgtcggcgttattgctggcatctactacctgttcacccacgcacgcaccgagcgcgcaaagcacggcgtagtcaagcatgtagaaaccatggttctggctcaataa

SEQ ID NO: 89 - protein, 413 aa, synthetic construct
  source 1..413: note = C. st I259R AA
MHTTEEVKLFTPTFIMGWVANFLQFLVFYFLITTMALYATKEFSASETEAGFAASAIVIGAVFSRLVSGYIIDRFGRRKIVVVSVIATTIACALYIPIDSLGLLYADRFFHGVAYAFACTAIMAMVQELIPSARRSEGTGYLALGTTVSAAIGPALALFLLGSFNYEVLFVVVLGISIVSLIASLVIYFRTSDPEPELDENGNAAEPIKFSFKSIINPKVLPIGLFMLLVAFAYSGVIAHINAFAENRDVVTGAGLFFRAYAISMFVMRSYLGKLQDRRGDNSVIYFGLVFFVISFIVLSLSTANWHVVVAGVLAGLGYGTLMPAAQAVSVGVVDKSEFGSAFSTLFLFVDLGFGFGPVILGAVVSAIGYGSMYAVLVGVGVIAGIYYLFTHARTERAKHGVVKHVETMVLAQ

SEQ ID NO: 90 - DNA, 1242 bp, synthetic construct
  source 1..1242: mol_type = other DNA; note = C. st I259R NT
gtgcacacaaccgaagaggtcaaactctttacgccgacgtttatcatggggtgggtcgccaacttcctgcagttcttggtgttctacttcctcatcaccacgatggcgctctacgcaaccaaggaattcagcgcatcggaaaccgaagcaggctttgccgccagtgcgattgttatcggtgcggtcttttcccgtttggtttccggatacattattgaccgcttcggtcgccgcaaaattgtggtggtctccgtcatcgcgaccactattgcgtgcgcgctatatatcccgatcgattctttggggctgctctacgctgaccgcttcttccacggtgtagcttatgcctttgcgtgcaccgcgattatggcgatggtccaggaactcattccttctgcacgccgctccgaaggcactggctacctggctttgggtaccaccgtttcggctgctatcggaccagcgctagcgctatttttgctgggttctttcaactacgaagtcctcttcgttgtcgtcctcggcatttcgattgtctctttgatcgcttcgctagtcatctatttccgcacctccgacccagagccagagctggatgaaaacggcaatgctgctgagcccattaagttcagcttcaagtccatcattaaccctaaagtcttgccgattggcctcttcatgctgctggtagcctttgcctactccggcgtgatcgcacatatcaacgcttttgctgaaaaccgcgacgttgttactggcgcaggcctattctttagagcttacgccatctccatgttcgtgatgcgctcctaccttggtaaattgcaagaccgccggggcgataacagcgttatctactttggtctcgtattctttgttatctcatttatcgtgctctcgctttctaccgccaactggcatgtcgttgtcgctggcgtgctagcaggtctgggctacggcaccttgatgccagctgctcaagcagtatctgttggtgttgtcgacaagagcgagttcggctcagcattttccaccttgttccttttcgttgacctcggcttcggcttcggcccagtcatccttggtgcagtggtttccgcgattggctacggttcgatgtatgcagtgctcgtcggcgtcggcgttattgctggcatctactacctgttcacccacgcacgcaccgagcgcgcaaagcacggcgtagtcaagcatgtagaaaccatggttctggctcaataa

SEQ ID NO: 91 - protein, 413 aa, synthetic construct
  source 1..413: note = C. st I259N AA
MHTTEEVKLFTPTFIMGWVANFLQFLVFYFLITTMALYATKEFSASETEAGFAASAIVIGAVFSRLVSGYIIDRFGRRKIVVVSVIATTIACALYIPIDSLGLLYADRFFHGVAYAFACTAIMAMVQELIPSARRSEGTGYLALGTTVSAAIGPALALFLLGSFNYEVLFVVVLGISIVSLIASLVIYFRTSDPEPELDENGNAAEPIKFSFKSIINPKVLPIGLFMLLVAFAYSGVIAHINAFAENRDVVTGAGLFFNAYAISMFVMRSYLGKLQDRRGDNSVIYFGLVFFVISFIVLSLSTANWHVVVAGVLAGLGYGTLMPAAQAVSVGVVDKSEFGSAFSTLFLFVDLGFGFGPVILGAVVSAIGYGSMYAVLVGVGVIAGIYYLFTHARTERAKHGVVKHVETMVLAQ

SEQ ID NO: 92 - DNA, 1242 bp, synthetic construct
  source 1..1242: mol_type = other DNA; note = C. st I259N NT
gtgcacacaaccgaagaggtcaaactctttacgccgacgtttatcatggggtgggtcgccaacttcctgcagttcttggtgttctacttcctcatcaccacgatggcgctctacgcaaccaaggaattcagcgcatcggaaaccgaagcaggctttgccgccagtgcgattgttatcggtgcggtcttttcccgtttggtttccggatacattattgaccgcttcggtcgccgcaaaattgtggtggtctccgtcatcgcgaccactattgcgtgcgcgctatatatcccgatcgattctttggggctgctctacgctgaccgcttcttccacggtgtagcttatgcctttgcgtgcaccgcgattatggcgatggtccaggaactcattccttctgcacgccgctccgaaggcactggctacctggctttgggtaccaccgtttcggctgctatcggaccagcgctagcgctatttttgctgggttctttcaactacgaagtcctcttcgttgtcgtcctcggcatttcgattgtctctttgatcgcttcgctagtcatctatttccgcacctccgacccagagccagagctggatgaaaacggcaatgctgctgagcccattaagttcagcttcaagtccatcattaaccctaaagtcttgccgattggcctcttcatgctgctggtagcctttgcctactccggcgtgatcgcacatatcaacgcttttgctgaaaaccgcgacgttgttactggcgcaggcctattctttaacgcttacgccatctccatgttcgtgatgcgctcctaccttggtaaattgcaagaccgccggggcgataacagcgttatctactttggtctcgtattctttgttatctcatttatcgtgctctcgctttctaccgccaactggcatgtcgttgtcgctggcgtgctagcaggtctgggctacggcaccttgatgccagctgctcaagcagtatctgttggtgttgtcgacaagagcgagttcggctcagcattttccaccttgttccttttcgttgacctcggcttcggcttcggcccagtcatccttggtgcagtggtttccgcgattggctacggttcgatgtatgcagtgctcgtcggcgtcggcgttattgctggcatctactacctgttcacccacgcacgcaccgagcgcgcaaagcacggcgtagtcaagcatgtagaaaccatggttctggctcaataa

SEQ ID NO: 93 - protein, 413 aa, synthetic construct
  source 1..413: note = C. st V310A AA
MHTTEEVKLFTPTFIMGWVANFLQFLVFYFLITTMALYATKEFSASETEAGFAASAIVIGAVFSRLVSGYIIDRFGRRKIVVVSVIATTIACALYIPIDSLGLLYADRFFHGVAYAFACTAIMAMVQELIPSARRSEGTGYLALGTTVSAAIGPALALFLLGSFNYEVLFVVVLGISIVSLIASLVIYFRTSDPEPELDENGNAAEPIKFSFKSIINPKVLPIGLFMLLVAFAYSGVIAHINAFAENRDVVTGAGLFFIAYAISMFVMRSYLGKLQDRRGDNSVIYFGLVFFVISFIVLSLSTANWHVVAAGVLAGLGYGTLMPAAQAVSVGVVDKSEFGSAFSTLFLFVDLGFGFGPVILGAVVSAIGYGSMYAVLVGVGVIAGIYYLFTHARTERAKHGVVKHVETMVLAQ

SEQ ID NO: 94 - DNA, 1242 bp, synthetic construct
  source 1..1242: mol_type = other DNA; note = C. st V310A NT
gtgcacacaaccgaagaggtcaaactctttacgccgacgtttatcatggggtgggtcgccaacttcctgcagttcttggtgttctacttcctcatcaccacgatggcgctctacgcaaccaaggaattcagcgcatcggaaaccgaagcaggctttgccgccagtgcgattgttatcggtgcggtcttttcccgtttggtttccggatacattattgaccgcttcggtcgccgcaaaattgtggtggtctccgtcatcgcgaccactattgcgtgcgcgctatatatcccgatcgattctttggggctgctctacgctgaccgcttcttccacggtgtagcttatgcctttgcgtgcaccgcgattatggcgatggtccaggaactcattccttctgcacgccgctccgaaggcactggctacctggctttgggtaccaccgtttcggctgctatcggaccagcgctagcgctatttttgctgggttctttcaactacgaagtcctcttcgttgtcgtcctcggcatttcgattgtctctttgatcgcttcgctagtcatctatttccgcacctccgacccagagccagagctggatgaaaacggcaatgctgctgagcccattaagttcagcttcaagtccatcattaaccctaaagtcttgccgattggcctcttcatgctgctggtagcctttgcctactccggcgtgatcgcacatatcaacgcttttgctgaaaaccgcgacgttgttactggcgcaggcctattctttatcgcttacgccatctccatgttcgtgatgcgctcctaccttggtaaattgcaagaccgccggggcgataacagcgttatctactttggtctcgtattctttgttatctcatttatcgtgctctcgctttctaccgccaactggcatgtcgttgccgctggcgtgctagcaggtctgggctacggcaccttgatgccagctgctcaagcagtatctgttggtgttgtcgacaagagcgagttcggctcagcattttccaccttgttccttttcgttgacctcggcttcggcttcggcccagtcatccttggtgcagtggtttccgcgattggctacggttcgatgtatgcagtgctcgtcggcgtcggcgttattgctggcatctactacctgttcacccacgcacgcaccgagcgcgcaaagcacggcgtagtcaagcatgtagaaaccatggttctggctcaataa

SEQ ID NO: 95 - protein, 413 aa, synthetic construct
  source 1..413: note = C. st V310F AA
MHTTEEVKLFTPTFIMGWVANFLQFLVFYFLITTMALYATKEFSASETEAGFAASAIVIGAVFSRLVSGYIIDRFGRRKIVVVSVIATTIACALYIPIDSLGLLYADRFFHGVAYAFACTAIMAMVQELIPSARRSEGTGYLALGTTVSAAIGPALALFLLGSFNYEVLFVVVLGISIVSLIASLVIYFRTSDPEPELDENGNAAEPIKFSFKSIINPKVLPIGLFMLLVAFAYSGVIAHINAFAENRDVVTGAGLFFIAYAISMFVMRSYLGKLQDRRGDNSVIYFGLVFFVISFIVLSLSTANWHVVFAGVLAGLGYGTLMPAAQAVSVGVVDKSEFGSAFSTLFLFVDLGFGFGPVILGAVVSAIGYGSMYAVLVGVGVIAGIYYLFTHARTERAKHGVVKHVETMVLAQ

SEQ ID NO: 96 - DNA, 1242 bp, synthetic construct
  source 1..1242: mol_type = other DNA; note = C. st V310F NT
gtgcacacaaccgaagaggtcaaactctttacgccgacgtttatcatggggtgggtcgccaacttcctgcagttcttggtgttctacttcctcatcaccacgatggcgctctacgcaaccaaggaattcagcgcatcggaaaccgaagcaggctttgccgccagtgcgattgttatcggtgcggtcttttcccgtttggtttccggatacattattgaccgcttcggtcgccgcaaaattgtggtggtctccgtcatcgcgaccactattgcgtgcgcgctatatatcccgatcgattctttggggctgctctacgctgaccgcttcttccacggtgtagcttatgcctttgcgtgcaccgcgattatggcgatggtccaggaactcattccttctgcacgccgctccgaaggcactggctacctggctttgggtaccaccgtttcggctgctatcggaccagcgctagcgctatttttgctgggttctttcaactacgaagtcctcttcgttgtcgtcctcggcatttcgattgtctctttgatcgcttcgctagtcatctatttccgcacctccgacccagagccagagctggatgaaaacggcaatgctgctgagcccattaagttcagcttcaagtccatcattaaccctaaagtcttgccgattggcctcttcatgctgctggtagcctttgcctactccggcgtgatcgcacatatcaacgcttttgctgaaaaccgcgacgttgttactggcgcaggcctattctttatcgcttacgccatctccatgttcgtgatgcgctcctaccttggtaaattgcaagaccgccggggcgataacagcgttatctactttggtctcgtattctttgttatctcatttatcgtgctctcgctttctaccgccaactggcatgtcgttttcgctggcgtgctagcaggtctgggctacggcaccttgatgccagctgctcaagcagtatctgttggtgttgtcgacaagagcgagttcggctcagcattttccaccttgttccttttcgttgacctcggcttcggcttcggcccagtcatccttggtgcagtggtttccgcgattggctacggttcgatgtatgcagtgctcgtcggcgtcggcgttattgctggcatctactacctgttcacccacgcacgcaccgagcgcgcaaagcacggcgtagtcaagcatgtagaaaccatggttctggctcaataa

SEQ ID NO: 97 - protein, 413 aa, synthetic construct
  source 1..413: note = C. st V310C AA
MHTTEEVKLFTPTFIMGWVANFLQFLVFYFLITTMALYATKEFSASETEAGFAASAIVIGAVFSRLVSGYIIDRFGRRKIVVVSVIATTIACALYIPIDSLGLLYADRFFHGVAYAFACTAIMAMVQELIPSARRSEGTGYLALGTTVSAAIGPALALFLLGSFNYEVLFVVVLGISIVSLIASLVIYFRTSDPEPELDENGNAAEPIKFSFKSIINPKVLPIGLFMLLVAFAYSGVIAHINAFAENRDVVTGAGLFFIAYAISMFVMRSYLGKLQDRRGDNSVIYFGLVFFVISFIVLSLSTANWHVVCAGVLAGLGYGTLMPAAQAVSVGVVDKSEFGSAFSTLFLFVDLGFGFGPVILGAVVSAIGYGSMYAVLVGVGVIAGIYYLFTHARTERAKHGVVKHVETMVLAQ

SEQ ID NO: 98 - DNA, 1242 bp, synthetic construct
  source 1..1242: mol_type = other DNA; note = C. st V310C NT
gtgcacacaaccgaagaggtcaaactctttacgccgacgtttatcatggggtgggtcgccaacttcctgcagttcttggtgttctacttcctcatcaccacgatggcgctctacgcaaccaaggaattcagcgcatcggaaaccgaagcaggctttgccgccagtgcgattgttatcggtgcggtcttttcccgtttggtttccggatacattattgaccgcttcggtcgccgcaaaattgtggtggtctccgtcatcgcgaccactattgcgtgcgcgctatatatcccgatcgattctttggggctgctctacgctgaccgcttcttccacggtgtagcttatgcctttgcgtgcaccgcgattatggcgatggtccaggaactcattccttctgcacgccgctccgaaggcactggctacctggctttgggtaccaccgtttcggctgctatcggaccagcgctagcgctatttttgctgggttctttcaactacgaagtcctcttcgttgtcgtcctcggcatttcgattgtctctttgatcgcttcgctagtcatctatttccgcacctccgacccagagccagagctggatgaaaacggcaatgctgctgagcccattaagttcagcttcaagtccatcattaaccctaaagtcttgccgattggcctcttcatgctgctggtagcctttgcctactccggcgtgatcgcacatatcaacgcttttgctgaaaaccgcgacgttgttactggcgcaggcctattctttatcgcttacgccatctccatgttcgtgatgcgctcctaccttggtaaattgcaagaccgccggggcgataacagcgttatctactttggtctcgtattctttgttatctcatttatcgtgctctcgctttctaccgccaactggcatgtcgtttgcgctggcgtgctagcaggtctgggctacggcaccttgatgccagctgctcaagcagtatctgttggtgttgtcgacaagagcgagttcggctcagcattttccaccttgttccttttcgttgacctcggcttcggcttcggcccagtcatccttggtgcagtggtttccgcgattggctacggttcgatgtatgcagtgctcgtcggcgtcggcgttattgctggcatctactacctgttcacccacgcacgcaccgagcgcgcaaagcacggcgtagtcaagcatgtagaaaccatggttctggctcaataa

SEQ ID NO: 99 - protein, 413 aa, synthetic construct
  source 1..413: note = C. st V310L AA
MHTTEEVKLFTPTFIMGWVANFLQFLVFYFLITTMALYATKEFSASETEAGFAASAIVIGAVFSRLVSGYIIDRFGRRKIVVVSVIATTIACALYIPIDSLGLLYADRFFHGVAYAFACTAIMAMVQELIPSARRSEGTGYLALGTTVSAAIGPALALFLLGSFNYEVLFVVVLGISIVSLIASLVIYFRTSDPEPELDENGNAAEPIKFSFKSIINPKVLPIGLFMLLVAFAYSGVIAHINAFAENRDVVTGAGLFFIAYAISMFVMRSYLGKLQDRRGDNSVIYFGLVFFVISFIVLSLSTANWHVVLAGVLAGLGYGTLMPAAQAVSVGVVDKSEFGSAFSTLFLFVDLGFGFGPVILGAVVSAIGYGSMYAVLVGVGVIAGIYYLFTHARTERAKHGVVKHVETMVLAQ

SEQ ID NO: 100 - DNA, 1242 bp, synthetic construct
  source 1..1242: mol_type = other DNA; note = C. st V310L NT
gtgcacacaaccgaagaggtcaaactctttacgccgacgtttatcatggggtgggtcgccaacttcctgcagttcttggtgttctacttcctcatcaccacgatggcgctctacgcaaccaaggaattcagcgcatcggaaaccgaagcaggctttgccgccagtgcgattgttatcggtgcggtcttttcccgtttggtttccggatacattattgaccgcttcggtcgccgcaaaattgtggtggtctccgtcatcgcgaccactattgcgtgcgcgctatatatcccgatcgattctttggggctgctctacgctgaccgcttcttccacggtgtagcttatgcctttgcgtgcaccgcgattatggcgatggtccaggaactcattccttctgcacgccgctccgaaggcactggctacctggctttgggtaccaccgtttcggctgctatcggaccagcgctagcgctatttttgctgggttctttcaactacgaagtcctcttcgttgtcgtcctcggcatttcgattgtctctttgatcgcttcgctagtcatctatttccgcacctccgacccagagccagagctggatgaaaacggcaatgctgctgagcccattaagttcagcttcaagtccatcattaaccctaaagtcttgccgattggcctcttcatgctgctggtagcctttgcctactccggcgtgatcgcacatatcaacgcttttgctgaaaaccgcgacgttgttactggcgcaggcctattctttatcgcttacgccatctccatgttcgtgatgcgctcctaccttggtaaattgcaagaccgccggggcgataacagcgttatctactttggtctcgtattctttgttatctcatttatcgtgctctcgctttctaccgccaactggcatgtcgttctggctggcgtgctagcaggtctgggctacggcaccttgatgccagctgctcaagcagtatctgttggtgttgtcgacaagagcgagttcggctcagcattttccaccttgttccttttcgttgacctcggcttcggcttcggcccagtcatccttggtgcagtggtttccgcgattggctacggttcgatgtatgcagtgctcgtcggcgtcggcgttattgctggcatctactacctgttcacccacgcacgcaccgagcgcgcaaagcacggcgtagtcaagcatgtagaaaccatggttctggctcaataa

SEQ ID NO: 101 - protein, 413 aa, synthetic construct
  source 1..413: note = C. st V310H AA
MHTTEEVKLFTPTFIMGWVANFLQFLVFYFLITTMALYATKEFSASETEAGFAASAIVIGAVFSRLVSGYIIDRFGRRKIVVVSVIATTIACALYIPIDSLGLLYADRFFHGVAYAFACTAIMAMVQELIPSARRSEGTGYLALGTTVSAAIGPALALFLLGSFNYEVLFVVVLGISIVSLIASLVIYFRTSDPEPELDENGNAAEPIKFSFKSIINPKVLPIGLFMLLVAFAYSGVIAHINAFAENRDVVTGAGLFFIAYAISMFVMRSYLGKLQDRRGDNSVIYFGLVFFVISFIVLSLSTANWHVVHAGVLAGLGYGTLMPAAQAVSVGVVDKSEFGSAFSTLFLFVDLGFGFGPVILGAVVSAIGYGSMYAVLVGVGVIAGIYYLFTHARTERAKHGVVKHVETMVLAQ

SEQ ID NO: 102 - DNA, 1242 bp, synthetic construct
  source 1..1242: mol_type = other DNA; note = C. st V310H NT
gtgcacacaaccgaagaggtcaaactctttacgccgacgtttatcatggggtgggtcgccaacttcctgcagttcttggtgttctacttcctcatcaccacgatggcgctctacgcaaccaaggaattcagcgcatcggaaaccgaagcaggctttgccgccagtgcgattgttatcggtgcggtcttttcccgtttggtttccggatacattattgaccgcttcggtcgccgcaaaattgtggtggtctccgtcatcgcgaccactattgcgtgcgcgctatatatcccgatcgattctttggggctgctctacgctgaccgcttcttccacggtgtagcttatgcctttgcgtgcaccgcgattatggcgatggtccaggaactcattccttctgcacgccgctccgaaggcactggctacctggctttgggtaccaccgtttcggctgctatcggaccagcgctagcgctatttttgctgggttctttcaactacgaagtcctcttcgttgtcgtcctcggcatttcgattgtctctttgatcgcttcgctagtcatctatttccgcacctccgacccagagccagagctggatgaaaacggcaatgctgctgagcccattaagttcagcttcaagtccatcattaaccctaaagtcttgccgattggcctcttcatgctgctggtagcctttgcctactccggcgtgatcgcacatatcaacgcttttgctgaaaaccgcgacgttgttactggcgcaggcctattctttatcgcttacgccatctccatgttcgtgatgcgctcctaccttggtaaattgcaagaccgccggggcgataacagcgttatctactttggtctcgtattctttgttatctcatttatcgtgctctcgctttctaccgccaactggcatgtcgttcacgctggcgtgctagcaggtctgggctacggcaccttgatgccagctgctcaagcagtatctgttggtgttgtcgacaagagcgagttcggctcagcattttccaccttgttccttttcgttgacctcggcttcggcttcggcccagtcatccttggtgcagtggtttccgcgattggctacggttcgatgtatgcagtgctcgtcggcgtcggcgttattgctggcatctactacctgttcacccacgcacgcaccgagcgcgcaaagcacggcgtagtcaagcatgtagaaaccatggttctggctcaataa

SEQ ID NO: 103 - protein, 413 aa, synthetic construct
  source 1..413: note = C. st V310R AA
MHTTEEVKLFTPTFIMGWVANFLQFLVFYFLITTMALYATKEFSASETEAGFAASAIVIGAVFSRLVSGYIIDRFGRRKIVVVSVIATTIACALYIPIDSLGLLYADRFFHGVAYAFACTAIMAMVQELIPSARRSEGTGYLALGTTVSAAIGPALALFLLGSFNYEVLFVVVLGISIVSLIASLVIYFRTSDPEPELDENGNAAEPIKFSFKSIINPKVLPIGLFMLLVAFAYSGVIAHINAFAENRDVVTGAGLFFIAYAISMFVMRSYLGKLQDRRGDNSVIYFGLVFFVISFIVLSLSTANWHVVRAGVLAGLGYGTLMPAAQAVSVGVVDKSEFGSAFSTLFLFVDLGFGFGPVILGAVVSAIGYGSMYAVLVGVGVIAGIYYLFTHARTERAKHGVVKHVETMVLAQ

SEQ ID NO: 104 - DNA, 1242 bp, synthetic construct
  source 1..1242: mol_type = other DNA; note = C. st V310R NT
gtgcacacaaccgaagaggtcaaactctttacgccgacgtttatcatggggtgggtcgccaacttcctgcagttcttggtgttctacttcctcatcaccacgatggcgctctacgcaaccaaggaattcagcgcatcggaaaccgaagcaggctttgccgccagtgcgattgttatcggtgcggtcttttcccgtttggtttccggatacattattgaccgcttcggtcgccgcaaaattgtggtggtctccgtcatcgcgaccactattgcgtgcgcgctatatatcccgatcgattctttggggctgctctacgctgaccgcttcttccacggtgtagcttatgcctttgcgtgcaccgcgattatggcgatggtccaggaactcattccttctgcacgccgctccgaaggcactggctacctggctttgggtaccaccgtttcggctgctatcggaccagcgctagcgctatttttgctgggttctttcaactacgaagtcctcttcgttgtcgtcctcggcatttcgattgtctctttgatcgcttcgctagtcatctatttccgcacctccgacccagagccagagctggatgaaaacggcaatgctgctgagcccattaagttcagcttcaagtccatcattaaccctaaagtcttgccgattggcctcttcatgctgctggtagcctttgcctactccggcgtgatcgcacatatcaacgcttttgctgaaaaccgcgacgttgttactggcgcaggcctattctttatcgcttacgccatctccatgttcgtgatgcgctcctaccttggtaaattgcaagaccgccggggcgataacagcgttatctactttggtctcgtattctttgttatctcatttatcgtgctctcgctttctaccgccaactggcatgtcgttagagctggcgtgctagcaggtctgggctacggcaccttgatgccagctgctcaagcagtatctgttggtgttgtcgacaagagcgagttcggctcagcattttccaccttgttccttttcgttgacctcggcttcggcttcggcccagtcatccttggtgcagtggtttccgcgattggctacggttcgatgtatgcagtgctcgtcggcgtcggcgttattgctggcatctactacctgttcacccacgcacgcaccgagcgcgcaaagcacggcgtagtcaagcatgtagaaaccatggttctggctcaataa

SEQ ID NO: 105 - protein, 413 aa, synthetic construct
  source 1..413: note = C. st V310I AA
MHTTEEVKLFTPTFIMGWVANFLQFLVFYFLITTMALYATKEFSASETEAGFAASAIVIGAVFSRLVSGYIIDRFGRRKIVVVSVIATTIACALYIPIDSLGLLYADRFFHGVAYAFACTAIMAMVQELIPSARRSEGTGYLALGTTVSAAIGPALALFLLGSFNYEVLFVVVLGISIVSLIASLVIYFRTSDPEPELDENGNAAEPIKFSFKSIINPKVLPIGLFMLLVAFAYSGVIAHINAFAENRDVVTGAGLFFIAYAISMFVMRSYLGKLQDRRGDNSVIYFGLVFFVISFIVLSLSTANWHVVIAGVLAGLGYGTLMPAAQAVSVGVVDKSEFGSAFSTLFLFVDLGFGFGPVILGAVVSAIGYGSMYAVLVGVGVIAGIYYLFTHARTERAKHGVVKHVETMVLAQ

SEQ ID NO: 106 - DNA, 1242 bp, synthetic construct
  source 1..1242: mol_type = other DNA; note = C. st V310I NT
gtgcacacaaccgaagaggtcaaactctttacgccgacgtttatcatggggtgggtcgccaacttcctgcagttcttggtgttctacttcctcatcaccacgatggcgctctacgcaaccaaggaattcagcgcatcggaaaccgaagcaggctttgccgccagtgcgattgttatcggtgcggtcttttcccgtttggtttccggatacattattgaccgcttcggtcgccgcaaaattgtggtggtctccgtcatcgcgaccactattgcgtgcgcgctatatatcccgatcgattctttggggctgctctacgctgaccgcttcttccacggtgtagcttatgcctttgcgtgcaccgcgattatggcgatggtccaggaactcattccttctgcacgccgctccgaaggcactggctacctggctttgggtaccaccgtttcggctgctatcggaccagcgctagcgctatttttgctgggttctttcaactacgaagtcctcttcgttgtcgtcctcggcatttcgattgtctctttgatcgcttcgctagtcatctatttccgcacctccgacccagagccagagctggatgaaaacggcaatgctgctgagcccattaagttcagcttcaagtccatcattaaccctaaagtcttgccgattggcctcttcatgctgctggtagcctttgcctactccggcgtgatcgcacatatcaacgcttttgctgaaaaccgcgacgttgttactggcgcaggcctattctttatcgcttacgccatctccatgttcgtgatgcgctcctaccttggtaaattgcaagaccgccggggcgataacagcgttatctactttggtctcgtattctttgttatctcatttatcgtgctctcgctttctaccgccaactggcatgtcgttatcgctggcgtgctagcaggtctgggctacggcaccttgatgccagctgctcaagcagtatctgttggtgttgtcgacaagagcgagttcggctcagcattttccaccttgttccttttcgttgacctcggcttcggcttcggcccagtcatccttggtgcagtggtttccgcgattggctacggttcgatgtatgcagtgctcgtcggcgtcggcgttattgctggcatctactacctgttcacccacgcacgcaccgagcgcgcaaagcacggcgtagtcaagcatgtagaaaccatggttctggctcaataa

SEQ ID NO: 107 - protein, 413 aa, synthetic construct
  source 1..413: note = C. st V310N AA
MHTTEEVKLFTPTFIMGWVANFLQFLVFYFLITTMALYATKEFSASETEAGFAASAIVIGAVFSRLVSGYIIDRFGRRKIVVVSVIATTIACALYIPIDSLGLLYADRFFHGVAYAFACTAIMAMVQELIPSARRSEGTGYLALGTTVSAAIGPALALFLLGSFNYEVLFVVVLGISIVSLIASLVIYFRTSDPEPELDENGNAAEPIKFSFKSIINPKVLPIGLFMLLVAFAYSGVIAHINAFAENRDVVTGAGLFFIAYAISMFVMRSYLGKLQDRRGDNSVIYFGLVFFVISFIVLSLSTANWHVVNAGVLAGLGYGTLMPAAQAVSVGVVDKSEFGSAFSTLFLFVDLGFGFGPVILGAVVSAIGYGSMYAVLVGVGVIAGIYYLFTHARTERAKHGVVKHVETMVLAQ

SEQ ID NO: 108 - DNA, 1242 bp, synthetic construct
  source 1..1242: mol_type = other DNA; note = C. st V310N NT
gtgcacacaaccgaagaggtcaaactctttacgccgacgtttatcatggggtgggtcgccaacttcctgcagttcttggtgttctacttcctcatcaccacgatggcgctctacgcaaccaaggaattcagcgcatcggaaaccgaagcaggctttgccgccagtgcgattgttatcggtgcggtcttttcccgtttggtttccggatacattattgaccgcttcggtcgccgcaaaattgtggtggtctccgtcatcgcgaccactattgcgtgcgcgctatatatcccgatcgattctttggggctgctctacgctgaccgcttcttccacggtgtagcttatgcctttgcgtgcaccgcgattatggcgatggtccaggaactcattccttctgcacgccgctccgaaggcactggctacctggctttgggtaccaccgtttcggctgctatcggaccagcgctagcgctatttttgctgggttctttcaactacgaagtcctcttcgttgtcgtcctcggcatttcgattgtctctttgatcgcttcgctagtcatctatttccgcacctccgacccagagccagagctggatgaaaacggcaatgctgctgagcccattaagttcagcttcaagtccatcattaaccctaaagtcttgccgattggcctcttcatgctgctggtagcctttgcctactccggcgtgatcgcacatatcaacgcttttgctgaaaaccgcgacgttgttactggcgcaggcctattctttatcgcttacgccatctccatgttcgtgatgcgctcctaccttggtaaattgcaagaccgccggggcgataacagcgttatctactttggtctcgtattctttgttatctcatttatcgtgctctcgctttctaccgccaactggcatgtcgttaacgctggcgtgctagcaggtctgggctacggcaccttgatgccagctgctcaagcagtatctgttggtgttgtcgacaagagcgagttcggctcagcattttccaccttgttccttttcgttgacctcggcttcggcttcggcccagtcatccttggtgcagtggtttccgcgattggctacggttcgatgtatgcagtgctcgtcggcgtcggcgttattgctggcatctactacctgttcacccacgcacgcaccgagcgcgcaaagcacggcgtagtcaagcatgtagaaaccatggttctggctcaataa

SEQ ID NO: 109 - protein, 413 aa, synthetic construct
  source 1..413: note = C. st V310D AA
MHTTEEVKLFTPTFIMGWVANFLQFLVFYFLITTMALYATKEFSASETEAGFAASAIVIGAVFSRLVSGYIIDRFGRRKIVVVSVIATTIACALYIPIDSLGLLYADRFFHGVAYAFACTAIMAMVQELIPSARRSEGTGYLALGTTVSAAIGPALALFLLGSFNYEVLFVVVLGISIVSLIASLVIYFRTSDPEPELDENGNAAEPIKFSFKSIINPKVLPIGLFMLLVAFAYSGVIAHINAFAENRDVVTGAGLFFIAYAISMFVMRSYLGKLQDRRGDNSVIYFGLVFFVISFIVLSLSTANWHVVDAGVLAGLGYGTLMPAAQAVSVGVVDKSEFGSAFSTLFLFVDLGFGFGPVILGAVVSAIGYGSMYAVLVGVGVIAGIYYLFTHARTERAKHGVVKHVETMVLAQ

SEQ ID NO: 110 - DNA, 1242 bp, synthetic construct
  source 1..1242: mol_type = other DNA; note = C. st V310D NT
gtgcacacaaccgaagaggtcaaactctttacgccgacgtttatcatggggtgggtcgccaacttcctgcagttcttggtgttctacttcctcatcaccacgatggcgctctacgcaaccaaggaattcagcgcatcggaaaccgaagcaggctttgccgccagtgcgattgttatcggtgcggtcttttcccgtttggtttccggatacattattgaccgcttcggtcgccgcaaaattgtggtggtctccgtcatcgcgaccactattgcgtgcgcgctatatatcccgatcgattctttggggctgctctacgctgaccgcttcttccacggtgtagcttatgcctttgcgtgcaccgcgattatggcgatggtccaggaactcattccttctgcacgccgctccgaaggcactggctacctggctttgggtaccaccgtttcggctgctatcggaccagcgctagcgctatttttgctgggttctttcaactacgaagtcctcttcgttgtcgtcctcggcatttcgattgtctctttgatcgcttcgctagtcatctatttccgcacctccgacccagagccagagctggatgaaaacggcaatgctgctgagcccattaagttcagcttcaagtccatcattaaccctaaagtcttgccgattggcctcttcatgctgctggtagcctttgcctactccggcgtgatcgcacatatcaacgcttttgctgaaaaccgcgacgttgttactggcgcaggcctattctttatcgcttacgccatctccatgttcgtgatgcgctcctaccttggtaaattgcaagaccgccggggcgataacagcgttatctactttggtctcgtattctttgttatctcatttatcgtgctctcgctttctaccgccaactggcatgtcgttgatgctggcgtgctagcaggtctgggctacggcaccttgatgccagctgctcaagcagtatctgttggtgttgtcgacaagagcgagttcggctcagcattttccaccttgttccttttcgttgacctcggcttcggcttcggcccagtcatccttggtgcagtggtttccgcgattggctacggttcgatgtatgcagtgctcgtcggcgtcggcgttattgctggcatctactacctgttcacccacgcacgcaccgagcgcgcaaagcacggcgtagtcaagcatgtagaaaccatggttctggctcaataa

SEQ ID NO: 111 - protein, 413 aa, synthetic construct
  source 1..413: note = C. st V310G AA
MHTTEEVKLFTPTFIMGWVANFLQFLVFYFLITTMALYATKEFSASETEAGFAASAIVIGAVFSRLVSGYIIDRFGRRKIVVVSVIATTIACALYIPIDSLGLLYADRFFHGVAYAFACTAIMAMVQELIPSARRSEGTGYLALGTTVSAAIGPALALFLLGSFNYEVLFVVVLGISIVSLIASLVIYFRTSDPEPELDENGNAAEPIKFSFKSIINPKVLPIGLFMLLVAFAYSGVIAHINAFAENRDVVTGAGLFFIAYAISMFVMRSYLGKLQDRRGDNSVIYFGLVFFVISFIVLSLSTANWHVVGAGVLAGLGYGTLMPAAQAVSVGVVDKSEFGSAFSTLFLFVDLGFGFGPVILGAVVSAIGYGSMYAVLVGVGVIAGIYYLFTHARTERAKHGVVKHVETMVLAQ

SEQ ID NO: 112 - DNA, 1242 bp, synthetic construct
  source 1..1242: mol_type = other DNA; note = C. st V310G NT
gtgcacacaaccgaagaggtcaaactctttacgccgacgtttatcatggggtgggtcgccaacttcctgcagttcttggtgttctacttcctcatcaccacgatggcgctctacgcaaccaaggaattcagcgcatcggaaaccgaagcaggctttgccgccagtgcgattgttatcggtgcggtcttttcccgtttggtttccggatacattattgaccgcttcggtcgccgcaaaattgtggtggtctccgtcatcgcgaccactattgcgtgcgcgctatatatcccgatcgattctttggggctgctctacgctgaccgcttcttccacggtgtagcttatgcctttgcgtgcaccgcgattatggcgatggtccaggaactcattccttctgcacgccgctccgaaggcactggctacctggctttgggtaccaccgtttcggctgctatcggaccagcgctagcgctatttttgctgggttctttcaactacgaagtcctcttcgttgtcgtcctcggcatttcgattgtctctttgatcgcttcgctagtcatctatttccgcacctccgacccagagccagagctggatgaaaacggcaatgctgctgagcccattaagttcagcttcaagtccatcattaaccctaaagtcttgccgattggcctcttcatgctgctggtagcctttgcctactccggcgtgatcgcacatatcaacgcttttgctgaaaaccgcgacgttgttactggcgcaggcctattctttatcgcttacgccatctccatgttcgtgatgcgctcctaccttggtaaattgcaagaccgccggggcgataacagcgttatctactttggtctcgtattctttgttatctcatttatcgtgctctcgctttctaccgccaactggcatgtcgttggcgctggcgtgctagcaggtctgggctacggcaccttgatgccagctgctcaagcagtatctgttggtgttgtcgacaagagcgagttcggctcagcattttccaccttgttccttttcgttgacctcggcttcggcttcggcccagtcatccttggtgcagtggtttccgcgattggctacggttcgatgtatgcagtgctcgtcggcgtcggcgttattgctggcatctactacctgttcacccacgcacgcaccgagcgcgcaaagcacggcgtagtcaagcatgtagaaaccatggttctggctcaataa

SEQ ID NO: 113 - protein, 413 aa, synthetic construct
  source 1..413: note = C. st V310P AA
MHTTEEVKLFTPTFIMGWVANFLQFLVFYFLITTMALYATKEFSASETEAGFAASAIVIGAVFSRLVSGYIIDRFGRRKIVVVSVIATTIACALYIPIDSLGLLYADRFFHGVAYAFACTAIMAMVQELIPSARRSEGTGYLALGTTVSAAIGPALALFLLGSFNYEVLFVVVLGISIVSLIASLVIYFRTSDPEPELDENGNAAEPIKFSFKSIINPKVLPIGLFMLLVAFAYSGVIAHINAFAENRDVVTGAGLFFIAYAISMFVMRSYLGKLQDRRGDNSVIYFGLVFFVISFIVLSLSTANWHVVPAGVLAGLGYGTLMPAAQAVSVGVVDKSEFGSAFSTLFLFVDLGFGFGPVILGAVVSAIGYGSMYAVLVGVGVIAGIYYLFTHARTERAKHGVVKHVETMVLAQ

SEQ ID NO: 114 - DNA, 1242 bp, synthetic construct
  source 1..1242: mol_type = other DNA; note = C. st V310P NT
gtgcacacaaccgaagaggtcaaactctttacgccgacgtttatcatggggtgggtcgccaacttcctgcagttcttggtgttctacttcctcatcaccacgatggcgctctacgcaaccaaggaattcagcgcatcggaaaccgaagcaggctttgccgccagtgcgattgttatcggtgcggtcttttcccgtttggtttccggatacattattgaccgcttcggtcgccgcaaaattgtggtggtctccgtcatcgcgaccactattgcgtgcgcgctatatatcccgatcgattctttggggctgctctacgctgaccgcttcttccacggtgtagcttatgcctttgcgtgcaccgcgattatggcgatggtccaggaactcattccttctgcacgccgctccgaaggcactggctacctggctttgggtaccaccgtttcggctgctatcggaccagcgctagcgctatttttgctgggttctttcaactacgaagtcctcttcgttgtcgtcctcggcatttcgattgtctctttgatcgcttcgctagtcatctatttccgcacctccgacccagagccagagctggatgaaaacggcaatgctgctgagcccattaagttcagcttcaagtccatcattaaccctaaagtcttgccgattggcctcttcatgctgctggtagcctttgcctactccggcgtgatcgcacatatcaacgcttttgctgaaaaccgcgacgttgttactggcgcaggcctattctttatcgcttacgccatctccatgttcgtgatgcgctcctaccttggtaaattgcaagaccgccggggcgataacagcgttatctactttggtctcgtattctttgttatctcatttatcgtgctctcgctttctaccgccaactggcatgtcgttccagctggcgtgctagcaggtctgggctacggcaccttgatgccagctgctcaagcagtatctgttggtgttgtcgacaagagcgagttcggctcagcattttccaccttgttccttttcgttgacctcggcttcggcttcggcccagtcatccttggtgcagtggtttccgcgattggctacggttcgatgtatgcagtgctcgtcggcgtcggcgttattgctggcatctactacctgttcacccacgcacgcaccgagcgcgcaaagcacggcgtagtcaagcatgtagaaaccatggttctggctcaataa

SEQ ID NO: 115 - protein, 413 aa, synthetic construct
  source 1..413: note = C. st V310E AA
MHTTEEVKLFTPTFIMGWVANFLQFLVFYFLITTMALYATKEFSASETEAGFAASAIVIGAVFSRLVSGYIIDRFGRRKIVVVSVIATTIACALYIPIDSLGLLYADRFFHGVAYAFACTAIMAMVQELIPSARRSEGTGYLALGTTVSAAIGPALALFLLGSFNYEVLFVVVLGISIVSLIASLVIYFRTSDPEPELDENGNAAEPIKFSFKSIINPKVLPIGLFMLLVAFAYSGVIAHINAFAENRDVVTGAGLFFIAYAISMFVMRSYLGKLQDRRGDNSVIYFGLVFFVISFIVLSLSTANWHVVEAGVLAGLGYGTLMPAAQAVSVGVVDKSEFGSAFSTLFLFVDLGFGFGPVILGAVVSAIGYGSMYAVLVGVGVIAGIYYLFTHARTERAKHGVVKHVETMVLAQ

SEQ ID NO: 116 - DNA, 1242 bp, synthetic construct
  source 1..1242: mol_type = other DNA; note = C. st V310E NT
gtgcacacaaccgaagaggtcaaactctttacgccgacgtttatcatggggtgggtcgccaacttcctgcagttcttggtgttctacttcctcatcaccacgatggcgctctacgcaaccaaggaattcagcgcatcggaaaccgaagcaggctttgccgccagtgcgattgttatcggtgcggtcttttcccgtttggtttccggatacattattgaccgcttcggtcgccgcaaaattgtggtggtctccgtcatcgcgaccactattgcgtgcgcgctatatatcccgatcgattctttggggctgctctacgctgaccgcttcttccacggtgtagcttatgcctttgcgtgcaccgcgattatggcgatggtccaggaactcattccttctgcacgccgctccgaaggcactggctacctggctttgggtaccaccgtttcggctgctatcggaccagcgctagcgctatttttgctgggttctttcaactacgaagtcctcttcgttgtcgtcctcggcatttcgattgtctctttgatcgcttcgctagtcatctatttccgcacctccgacccagagccagagctggatgaaaacggcaatgctgctgagcccattaagttcagcttcaagtccatcattaaccctaaagtcttgccgattggcctcttcatgctgctggtagcctttgcctactccggcgtgatcgcacatatcaacgcttttgctgaaaaccgcgacgttgttactggcgcaggcctattctttatcgcttacgccatctccatgttcgtgatgcgctcctaccttggtaaattgcaagaccgccggggcgataacagcgttatctactttggtctcgtattctttgttatctcatttatcgtgctctcgctttctaccgccaactggcatgtcgttgaagctggcgtgctagcaggtctgggctacggcaccttgatgccagctgctcaagcagtatctgttggtgttgtcgacaagagcgagttcggctcagcattttccaccttgttccttttcgttgacctcggcttcggcttcggcccagtcatccttggtgcagtggtttccgcgattggctacggttcgatgtatgcagtgctcgtcggcgtcggcgttattgctggcatctactacctgttcacccacgcacgcaccgagcgcgcaaagcacggcgtagtcaagcatgtagaaaccatggttctggctcaataa

SEQ ID NO: 117 - protein, 413 aa, synthetic construct
  source 1..413: note = C. st V310M AA
MHTTEEVKLFTPTFIMGWVANFLQFLVFYFLITTMALYATKEFSASETEAGFAASAIVIGAVFSRLVSGYIIDRFGRRKIVVVSVIATTIACALYIPIDSLGLLYADRFFHGVAYAFACTAIMAMVQELIPSARRSEGTGYLALGTTVSAAIGPALALFLLGSFNYEVLFVVVLGISIVSLIASLVIYFRTSDPEPELDENGNAAEPIKFSFKSIINPKVLPIGLFMLLVAFAYSGVIAHINAFAENRDVVTGAGLFFIAYAISMFVMRSYLGKLQDRRGDNSVIYFGLVFFVISFIVLSLSTANWHVVMAGVLAGLGYGTLMPAAQAVSVGVVDKSEFGSAFSTLFLFVDLGFGFGPVILGAVVSAIGYGSMYAVLVGVGVIAGIYYLFTHARTERAKHGVVKHVETMVLAQ

SEQ ID NO: 118 - DNA, 1242 bp, synthetic construct
  source 1..1242: mol_type = other DNA; note = C. st V310M NT
gtgcacacaaccgaagaggtcaaactctttacgccgacgtttatcatggggtgggtcgccaacttcctgcagttcttggtgttctacttcctcatcaccacgatggcgctctacgcaaccaaggaattcagcgcatcggaaaccgaagcaggctttgccgccagtgcgattgttatcggtgcggtcttttcccgtttggtttccggatacattattgaccgcttcggtcgccgcaaaattgtggtggtctccgtcatcgcgaccactattgcgtgcgcgctatatatcccgatcgattctttggggctgctctacgctgaccgcttcttccacggtgtagcttatgcctttgcgtgcaccgcgattatggcgatggtccaggaactcattccttctgcacgccgctccgaaggcactggctacctggctttgggtaccaccgtttcggctgctatcggaccagcgctagcgctatttttgctgggttctttcaactacgaagtcctcttcgttgtcgtcctcggcatttcgattgtctctttgatcgcttcgctagtcatctatttccgcacctccgacccagagccagagctggatgaaaacggcaatgctgctgagcccattaagttcagcttcaagtccatcattaaccctaaagtcttgccgattggcctcttcatgctgctggtagcctttgcctactccggcgtgatcgcacatatcaacgcttttgctgaaaaccgcgacgttgttactggcgcaggcctattctttatcgcttacgccatctccatgttcgtgatgcgctcctaccttggtaaattgcaagaccgccggggcgataacagcgttatctactttggtctcgtattctttgttatctcatttatcgtgctctcgctttctaccgccaactggcatgtcgttatggctggcgtgctagcaggtctgggctacggcaccttgatgccagctgctcaagcagtatctgttggtgttgtcgacaagagcgagttcggctcagcattttccaccttgttccttttcgttgacctcggcttcggcttcggcccagtcatccttggtgcagtggtttccgcgattggctacggttcgatgtatgcagtgctcgtcggcgtcggcgttattgctggcatctactacctgttcacccacgcacgcaccgagcgcgcaaagcacggcgtagtcaagcatgtagaaaccatggttctggctcaataa

SEQ ID NO: 119 - protein, 413 aa, synthetic construct
  source 1..413: note = C. st V310W AA
MHTTEEVKLFTPTFIMGWVANFLQFLVFYFLITTMALYATKEFSASETEAGFAASAIVIGAVFSRLVSGYIIDRFGRRKIVVVSVIATTIACALYIPIDSLGLLYADRFFHGVAYAFACTAIMAMVQELIPSARRSEGTGYLALGTTVSAAIGPALALFLLGSFNYEVLFVVVLGISIVSLIASLVIYFRTSDPEPELDENGNAAEPIKFSFKSIINPKVLPIGLFMLLVAFAYSGVIAHINAFAENRDVVTGAGLFFIAYAISMFVMRSYLGKLQDRRGDNSVIYFGLVFFVISFIVLSLSTANWHVVWAGVLAGLGYGTLMPAAQAVSVGVVDKSEFGSAFSTLFLFVDLGFGFGPVILGAVVSAIGYGSMYAVLVGVGVIAGIYYLFTHARTERAKHGVVKHVETMVLAQ

SEQ ID NO: 120 - DNA, 1242 bp, synthetic construct
  source 1..1242: mol_type = other DNA; note = C. st V310W NT
gtgcacacaaccgaagaggtcaaactctttacgccgacgtttatcatggggtgggtcgccaacttcctgcagttcttggtgttctacttcctcatcaccacgatggcgctctacgcaaccaaggaattcagcgcatcggaaaccgaagcaggctttgccgccagtgcgattgttatcggtgcggtcttttcccgtttggtttccggatacattattgaccgcttcggtcgccgcaaaattgtggtggtctccgtcatcgcgaccactattgcgtgcgcgctatatatcccgatcgattctttggggctgctctacgctgaccgcttcttccacggtgtagcttatgcctttgcgtgcaccgcgattatggcgatggtccaggaactcattccttctgcacgccgctccgaaggcactggctacctggctttgggtaccaccgtttcggctgctatcggaccagcgctagcgctatttttgctgggttctttcaactacgaagtcctcttcgttgtcgtcctcggcatttcgattgtctctttgatcgcttcgctagtcatctatttccgcacctccgacccagagccagagctggatgaaaacggcaatgctgctgagcccattaagttcagcttcaagtccatcattaaccctaaagtcttgccgattggcctcttcatgctgctggtagcctttgcctactccggcgtgatcgcacatatcaacgcttttgctgaaaaccgcgacgttgttactggcgcaggcctattctttatcgcttacgccatctccatgttcgtgatgcgctcctaccttggtaaattgcaagaccgccggggcgataacagcgttatctactttggtctcgtattctttgttatctcatttatcgtgctctcgctttctaccgccaactggcatgtcgtttgggctggcgtgctagcaggtctgggctacggcaccttgatgccagctgctcaagcagtatctgttggtgttgtcgacaagagcgagttcggctcagcattttccaccttgttccttttcgttgacctcggcttcggcttcggcccagtcatccttggtgcagtggtttccgcgattggctacggttcgatgtatgcagtgctcgtcggcgtcggcgttattgctggcatctactacctgttcacccacgcacgcaccgagcgcgcaaagcacggcgtagtcaagcatgtagaaaccatggttctggctcaataa

SEQ ID NO: 121 - protein, 413 aa, synthetic construct
  source 1..413: note = C. st V310S AA
MHTTEEVKLFTPTFIMGWVANFLQFLVFYFLITTMALYATKEFSASETEAGFAASAIVIGAVFSRLVSGYIIDRFGRRKIVVVSVIATTIACALYIPIDSLGLLYADRFFHGVAYAFACTAIMAMVQELIPSARRSEGTGYLALGTTVSAAIGPALALFLLGSFNYEVLFVVVLGISIVSLIASLVIYFRTSDPEPELDENGNAAEPIKFSFKSIINPKVLPIGLFMLLVAFAYSGVIAHINAFAENRDVVTGAGLFFIAYAISMFVMRSYLGKLQDRRGDNSVIYFGLVFFVISFIVLSLSTANWHVVSAGVLAGLGYGTLMPAAQAVSVGVVDKSEFGSAFSTLFLFVDLGFGFGPVILGAVVSAIGYGSMYAVLVGVGVIAGIYYLFTHARTERAKHGVVKHVETMVLAQ

SEQ ID NO: 122 - DNA, 1242 bp, synthetic construct
  source 1..1242: mol_type = other DNA; note = C. st V310S NT
gtgcacacaaccgaagaggtcaaactctttacgccgacgtttatcatggggtgggtcgccaacttcctgcagttcttggtgttctacttcctcatcaccacgatggcgctctacgcaaccaaggaattcagcgcatcggaaaccgaagcaggctttgccgccagtgcgattgttatcggtgcggtcttttcccgtttggtttccggatacattattgaccgcttcggtcgccgcaaaattgtggtggtctccgtcatcgcgaccactattgcgtgcgcgctatatatcccgatcgattctttggggctgctctacgctgaccgcttcttccacggtgtagcttatgcctttgcgtgcaccgcgattatggcgatggtccaggaactcattccttctgcacgccgctccgaaggcactggctacctggctttgggtaccaccgtttcggctgctatcggaccagcgctagcgctatttttgctgggttctttcaactacgaagtcctcttcgttgtcgtcctcggcatttcgattgtctctttgatcgcttcgctagtcatctatttccgcacctccgacccagagccagagctggatgaaaacggcaatgctgctgagcccattaagttcagcttcaagtccatcattaaccctaaagtcttgccgattggcctcttcatgctgctggtagcctttgcctactccggcgtgatcgcacatatcaacgcttttgctgaaaaccgcgacgttgttactggcgcaggcctattctttatcgcttacgccatctccatgttcgtgatgcgctcctaccttggtaaattgcaagaccgccggggcgataacagcgttatctactttggtctcgtattctttgttatctcatttatcgtgctctcgctttctaccgccaactggcatgtcgtttccgctggcgtgctagcaggtctgggctacggcaccttgatgccagctgctcaagcagtatctgttggtgttgtcgacaagagcgagttcggctcagcattttccaccttgttccttttcgttgacctcggcttcggcttcggcccagtcatccttggtgcagtggtttccgcgattggctacggttcgatgtatgcagtgctcgtcggcgtcggcgttattgctggcatctactacctgttcacccacgcacgcaccgagcgcgcaaagcacggcgtagtcaagcatgtagaaaccatggttctggctcaataa

SEQ ID NO: 123 - protein, 413 aa, synthetic construct
  source 1..413: note = C. st V310T AA
MHTTEEVKLFTPTFIMGWVANFLQFLVFYFLITTMALYATKEFSASETEAGFAASAIVIGAVFSRLVSGYIIDRFGRRKIVVVSVIATTIACALYIPIDSLGLLYADRFFHGVAYAFACTAIMAMVQELIPSARRSEGTGYLALGTTVSAAIGPALALFLLGSFNYEVLFVVVLGISIVSLIASLVIYFRTSDPEPELDENGNAAEPIKFSFKSIINPKVLPIGLFMLLVAFAYSGVIAHINAFAENRDVVTGAGLFFIAYAISMFVMRSYLGKLQDRRGDNSVIYFGLVFFVISFIVLSLSTANWHVVTAGVLAGLGYGTLMPAAQAVSVGVVDKSEFGSAFSTLFLFVDLGFGFGPVILGAVVSAIGYGSMYAVLVGVGVIAGIYYLFTHARTERAKHGVVKHVETMVLAQ

SEQ ID NO: 124 - DNA, 1242 bp, synthetic construct
  source 1..1242: mol_type = other DNA; note = C. st V310T NT
gtgcacacaaccgaagaggtcaaactctttacgccgacgtttatcatggggtgggtcgccaacttcctgcagttcttggtgttctacttcctcatcaccacgatggcgctctacgcaaccaaggaattcagcgcatcggaaaccgaagcaggctttgccgccagtgcgattgttatcggtgcggtcttttcccgtttggtttccggatacattattgaccgcttcggtcgccgcaaaattgtggtggtctccgtcatcgcgaccactattgcgtgcgcgctatatatcccgatcgattctttggggctgctctacgctgaccgcttcttccacggtgtagcttatgcctttgcgtgcaccgcgattatggcgatggtccaggaactcattccttctgcacgccgctccgaaggcactggctacctggctttgggtaccaccgtttcggctgctatcggaccagcgctagcgctatttttgctgggttctttcaactacgaagtcctcttcgttgtcgtcctcggcatttcgattgtctctttgatcgcttcgctagtcatctatttccgcacctccgacccagagccagagctggatgaaaacggcaatgctgctgagcccattaagttcagcttcaagtccatcattaaccctaaagtcttgccgattggcctcttcatgctgctggtagcctttgcctactccggcgtgatcgcacatatcaacgcttttgctgaaaaccgcgacgttgttactggcgcaggcctattctttatcgcttacgccatctccatgttcgtgatgcgctcctaccttggtaaattgcaagaccgccggggcgataacagcgttatctactttggtctcgtattctttgttatctcatttatcgtgctctcgctttctaccgccaactggcatgtcgttaccgctggcgtgctagcaggtctgggctacggcaccttgatgccagctgctcaagcagtatctgttggtgttgtcgacaagagcgagttcggctcagcattttccaccttgttccttttcgttgacctcggcttcggcttcggcccagtcatccttggtgcagtggtttccgcgattggctacggttcgatgtatgcagtgctcgtcggcgtcggcgttattgctggcatctactacctgttcacccacgcacgcaccgagcgcgcaaagcacggcgtagtcaagcatgtagaaaccatggttctggctcaataa

SEQ ID NO: 125 - protein, 413 aa, synthetic construct
  source 1..413: note = C. st V310Q AA
MHTTEEVKLFTPTFIMGWVANFLQFLVFYFLITTMALYATKEFSASETEAGFAASAIVIGAVFSRLVSGYIIDRFGRRKIVVVSVIATTIACALYIPIDSLGLLYADRFFHGVAYAFACTAIMAMVQELIPSARRSEGTGYLALGTTVSAAIGPALALFLLGSFNYEVLFVVVLGISIVSLIASLVIYFRTSDPEPELDENGNAAEPIKFSFKSIINPKVLPIGLFMLLVAFAYSGVIAHINAFAENRDVVTGAGLFFIAYAISMFVMRSYLGKLQDRRGDNSVIYFGLVFFVISFIVLSLSTANWHVVQAGVLAGLGYGTLMPAAQAVSVGVVDKSEFGSAFSTLFLFVDLGFGFGPVILGAVVSAIGYGSMYAVLVGVGVIAGIYYLFTHARTERAKHGVVKHVETMVLAQ

SEQ ID NO: 126 - DNA, 1242 bp, synthetic construct
  source 1..1242: mol_type = other DNA; note = C. st V310Q NT
gtgcacacaaccgaagaggtcaaactctttacgccgacgtttatcatggggtgggtcgccaacttcctgcagttcttggtgttctacttcctcatcaccacgatggcgctctacgcaaccaaggaattcagcgcatcggaaaccgaagcaggctttgccgccagtgcgattgttatcggtgcggtcttttcccgtttggtttccggatacattattgaccgcttcggtcgccgcaaaattgtggtggtctccgtcatcgcgaccactattgcgtgcgcgctatatatcccgatcgattctttggggctgctctacgctgaccgcttcttccacggtgtagcttatgcctttgcgtgcaccgcgattatggcgatggtccaggaactcattccttctgcacgccgctccgaaggcactggctacctggctttgggtaccaccgtttcggctgctatcggaccagcgctagcgctatttttgctgggttctttcaactacgaagtcctcttcgttgtcgtcctcggcatttcgattgtctctttgatcgcttcgctagtcatctatttccgcacctccgacccagagccagagctggatgaaaacggcaatgctgctgagcccattaagttcagcttcaagtccatcattaaccctaaagtcttgccgattggcctcttcatgctgctggtagcctttgcctactccggcgtgatcgcacatatcaacgcttttgctgaaaaccgcgacgttgttactggcgcaggcctattctttatcgcttacgccatctccatgttcgtgatgcgctcctaccttggtaaattgcaagaccgccggggcgataacagcgttatctactttggtctcgtattctttgttatctcatttatcgtgctctcgctttctaccgccaactggcatgtcgttcaggctggcgtgctagcaggtctgggctacggcaccttgatgccagctgctcaagcagtatctgttggtgttgtcgacaagagcgagttcggctcagcattttccaccttgttccttttcgttgacctcggcttcggcttcggcccagtcatccttggtgcagtggtttccgcgattggctacggttcgatgtatgcagtgctcgtcggcgtcggcgttattgctggcatctactacctgttcacccacgcacgcaccgagcgcgcaaagcacggcgtagtcaagcatgtagaaaccatggttctggctcaataa

SEQ ID NO: 127 - protein, 413 aa, synthetic construct
  source 1..413: note = C. st V310K AA
MHTTEEVKLFTPTFIMGWVANFLQFLVFYFLITTMALYATKEFSASETEAGFAASAIVIGAVFSRLVSGYIIDRFGRRKIVVVSVIATTIACALYIPIDSLGLLYADRFFHGVAYAFACTAIMAMVQELIPSARRSEGTGYLALGTTVSAAIGPALALFLLGSFNYEVLFVVVLGISIVSLIASLVIYFRTSDPEPELDENGNAAEPIKFSFKSIINPKVLPIGLFMLLVAFAYSGVIAHINAFAENRDVVTGAGLFFIAYAISMFVMRSYLGKLQDRRGDNSVIYFGLVFFVISFIVLSLSTANWHVVKAGVLAGLGYGTLMPAAQAVSVGVVDKSEFGSAFSTLFLFVDLGFGFGPVILGAVVSAIGYGSMYAVLVGVGVIAGIYYLFTHARTERAKHGVVKHVETMVLAQ

SEQ ID NO: 128 - DNA, 1242 bp, synthetic construct
  source 1..1242: mol_type = other DNA; note = C. st V310K NT
gtgcacacaaccgaagaggtcaaactctttacgccgacgtttatcatggggtgggtcgccaacttcctgcagttcttggtgttctacttcctcatcaccacgatggcgctctacgcaaccaaggaattcagcgcatcggaaaccgaagcaggctttgccgccagtgcgattgttatcggtgcggtcttttcccgtttggtttccggatacattattgaccgcttcggtcgccgcaaaattgtggtggtctccgtcatcgcgaccactattgcgtgcgcgctatatatcccgatcgattctttggggctgctctacgctgaccgcttcttccacggtgtagcttatgcctttgcgtgcaccgcgattatggcgatggtccaggaactcattccttctgcacgccgctccgaaggcactggctacctggctttgggtaccaccgtttcggctgctatcggaccagcgctagcgctatttttgctgggttctttcaactacgaagtcctcttcgttgtcgtcctcggcatttcgattgtctctttgatcgcttcgctagtcatctatttccgcacctccgacccagagccagagctggatgaaaacggcaatgctgctgagcccattaagttcagcttcaagtccatcattaaccctaaagtcttgccgattggcctcttcatgctgctggtagcctttgcctactccggcgtgatcgcacatatcaacgcttttgctgaaaaccgcgacgttgttactggcgcaggcctattctttatcgcttacgccatctccatgttcgtgatgcgctcctaccttggtaaattgcaagaccgccggggcgataacagcgttatctactttggtctcgtattctttgttatctcatttatcgtgctctcgctttctaccgccaactggcatgtcgttaaggctggcgtgctagcaggtctgggctacggcaccttgatgccagctgctcaagcagtatctgttggtgttgtcgacaagagcgagttcggctcagcattttccaccttgttccttttcgttgacctcggcttcggcttcggcccagtcatccttggtgcagtggtttccgcgattggctacggttcgatgtatgcagtgctcgtcggcgtcggcgttattgctggcatctactacctgttcacccacgcacgcaccgagcgcgcaaagcacggcgtagtcaagcatgtagaaaccatggttctggctcaataa

SEQ ID NO: 129 - protein, 413 aa, synthetic construct
  source 1..413: note = C. st V310Y AA
MHTTEEVKLFTPTFIMGWVANFLQFLVFYFLITTMALYATKEFSASETEAGFAASAIVIGAVFSRLVSGYIIDRFGRRKIVVVSVIATTIACALYIPIDSLGLLYADRFFHGVAYAFACTAIMAMVQELIPSARRSEGTGYLALGTTVSAAIGPALALFLLGSFNYEVLFVVVLGISIVSLIASLVIYFRTSDPEPELDENGNAAEPIKFSFKSIINPKVLPIGLFMLLVAFAYSGVIAHINAFAENRDVVTGAGLFFIAYAISMFVMRSYLGKLQDRRGDNSVIYFGLVFFVISFIVLSLSTANWHVVYAGVLAGLGYGTLMPAAQAVSVGVVDKSEFGSAFSTLFLFVDLGFGFGPVILGAVVSAIGYGSMYAVLVGVGVIAGIYYLFTHARTERAKHGVVKHVETMVLAQ

SEQ ID NO: 130 - DNA, 1242 bp, synthetic construct
  source 1..1242: mol_type = other DNA; note = C. st V310Y NT
gtgcacacaaccgaagaggtcaaactctttacgccgacgtttatcatggggtgggtcgccaacttcctgcagttcttggtgttctacttcctcatcaccacgatggcgctctacgcaaccaaggaattcagcgcatcggaaaccgaagcaggctttgccgccagtgcgattgttatcggtgcggtcttttcccgtttggtttccggatacattattgaccgcttcggtcgccgcaaaattgtggtggtctccgtcatcgcgaccactattgcgtgcgcgctatatatcccgatcgattctttggggctgctctacgctgaccgcttcttccacggtgtagcttatgcctttgcgtgcaccgcgattatggcgatggtccaggaactcattccttctgcacgccgctccgaaggcactggctacctggctttgggtaccaccgtttcggctgctatcggaccagcgctagcgctatttttgctgggttctttcaactacgaagtcctcttcgttgtcgtcctcggcatttcgattgtctctttgatcgcttcgctagtcatctatttccgcacctccgacccagagccagagctggatgaaaacggcaatgctgctgagcccattaagttcagcttcaagtccatcattaaccctaaagtcttgccgattggcctcttcatgctgctggtagcctttgcctactccggcgtgatcgcacatatcaacgcttttgctgaaaaccgcgacgttgttactggcgcaggcctattctttatcgcttacgccatctccatgttcgtgatgcgctcctaccttggtaaattgcaagaccgccggggcgataacagcgttatctactttggtctcgtattctttgttatctcatttatcgtgctctcgctttctaccgccaactggcatgtcgtttacgctggcgtgctagcaggtctgggctacggcaccttgatgccagctgctcaagcagtatctgttggtgttgtcgacaagagcgagttcggctcagcattttccaccttgttccttttcgttgacctcggcttcggcttcggcccagtcatccttggtgcagtggtttccgcgattggctacggttcgatgtatgcagtgctcgtcggcgtcggcgttattgctggcatctactacctgttcacccacgcacgcaccgagcgcgcaaagcacggcgtagtcaagcatgtagaaaccatggttctggctcaataa

SEQ ID NO: 131 - protein, 413 aa, synthetic construct
  source 1..413: note = C. st I238T AA
MHTTEEVKLFTPTFIMGWVANFLQFLVFYFLITTMALYATKEFSASETEAGFAASAIVIGAVFSRLVSGYIIDRFGRRKIVVVSVIATTIACALYIPIDSLGLLYADRFFHGVAYAFACTAIMAMVQELIPSARRSEGTGYLALGTTVSAAIGPALALFLLGSFNYEVLFVVVLGISIVSLIASLVIYFRTSDPEPELDENGNAAEPIKFSFKSIINPKVLPIGLFMLLVAFAYSGVTAHINAFAENRDVVTGAGLFFIAYAISMFVMRSYLGKLQDRRGDNSVIYFGLVFFVISFIVLSLSTANWHVVVAGVLAGLGYGTLMPAAQAVSVGVVDKSEFGSAFSTLFLFVDLGFGFGPVILGAVVSAIGYGSMYAVLVGVGVIAGIYYLFTHARTERAKHGVVKHVETMVLAQ

SEQ ID NO: 132 - DNA, 1242 bp, synthetic construct
  source 1..1242: mol_type = other DNA; note = C. st I238T NT
gtgcacacaaccgaagaggtcaaactctttacgccgacgtttatcatggggtgggtcgccaacttcctgcagttcttggtgttctacttcctcatcaccacgatggcgctctacgcaaccaaggaattcagcgcatcggaaaccgaagcaggctttgccgccagtgcgattgttatcggtgcggtcttttcccgtttggtttccggatacattattgaccgcttcggtcgccgcaaaattgtggtggtctccgtcatcgcgaccactattgcgtgcgcgctatatatcccgatcgattctttggggctgctctacgctgaccgcttcttccacggtgtagcttatgcctttgcgtgcaccgcgattatggcgatggtccaggaactcattccttctgcacgccgctccgaaggcactggctacctggctttgggtaccaccgtttcggctgctatcggaccagcgctagcgctatttttgctgggttctttcaactacgaagtcctcttcgttgtcgtcctcggcatttcgattgtctctttgatcgcttcgctagtcatctatttccgcacctccgacccagagccagagctggatgaaaacggcaatgctgctgagcccattaagttcagcttcaagtccatcattaaccctaaagtcttgccgattggcctcttcatgctgctggtagcctttgcctactccggcgtgaccgcacatatcaacgcttttgctgaaaaccgcgacgttgttactggcgcaggcctattctttatcgcttacgccatctccatgttcgtgatgcgctcctaccttggtaaattgcaagaccgccggggcgataacagcgttatctactttggtctcgtattctttgttatctcatttatcgtgctctcgctttctaccgccaactggcatgtcgttgtcgctggcgtgctagcaggtctgggctacggcaccttgatgccagctgctcaagcagtatctgttggtgttgtcgacaagagcgagttcggctcagcattttccaccttgttccttttcgttgacctcggcttcggcttcggcccagtcatccttggtgcagtggtttccgcgattggctacggttcgatgtatgcagtgctcgtcggcgtcggcgttattgctggcatctactacctgttcacccacgcacgcaccgagcgcgcaaagcacggcgtagtcaagcatgtagaaaccatggttctggctcaataa

SEQ ID NO: 133 - protein, 406 aa, synthetic construct
  source 1..406: note = C. gl 13032 I231T AA
MSVAEEGKLFTPTFVMGWFANLFQFLVFYFLITTMALYAIKEFQASEVEAGFASSSIVIGAVFSRFFSGYIIDRFGRRKIVLISVLVTTIACALYLPIESLPLLYANRFLHGVGYAFAATAIMAMVQELIPASRRSEGTGYLALGTTVSAALGPALALFVLGTFDYDMLFIVVLATSVISLIAVVFMYFKTSDPEPSGEPAKFSFKSIMNPKIIPIGIFILLICFAYSGVIAYINAFAEERDLITGAGLFFIAYAVSMFVMRSFLGKLQDRRGDNVVIYFGLFFFVISLTTLSFATSNWHVVLSGVIAGLGYGTLMPAVQSIAVGVVDKTEFGTAFSTLFLFVDLGFGFGPIILGAVSAAIGFGPMYAALAGVGVIAGIFYLFTHARTDRAKNGFVKHPEPVALVS

SEQ ID NO: 134 - DNA, 1221 bp, synthetic construct
  source 1..1221: mol_type = other DNA; note = C. gl 13032 I231T NT
atgtccgtagctgaagaagggaaactttttacaccaacgtttgtcatgggatggtttgccaaccttttccagttcctggtgttctacttcctcatcaccaccatggctttgtacgccatcaaggaatttcaagcctctgaagtagaagctggcttcgcatccagctcaattgttatcggcgcagtcttttccaggtttttctccggctatattattgaccgttttggtcgacgcaagattgtgctcatctcagtcctagtcactaccattgcgtgtgccttgtaccttcccatcgaatcattgccattgctatacgcaaacaggttcctccacggtgttggatacgcttttgctgccaccgcgatcatggcaatggtccaggagctcattccagcgtcacgacgttccgaaggtactggttacctggcattgggcactaccgtttctgcagcacttggaccagccctagcactttttgtcctaggaacatttgattacgacatgctgtttatcgtggtcttggcaacctcggtcatctctttgatcgccgtcgtgttcatgtactttaagaccagcgaccctgagccttctggggaaccagccaagttcagcttcaaatctattatgaacccaaagatcatccccatcggcatctttatcttgcttatttgctttgcttactctggcgtcaccgcctacatcaacgcatttgctgaagaacgcgatctgattacgggtgctggattgttcttcattgcctacgcagtatcaatgtttgtgatgcgcagcttccttggcaaactgcaggaccgtcgcggagacaacgtcgttatttactttggattgttcttcttcgttatttccttgacgattttgtcctttgccacttccaactggcacgttgtgttgtccggagtcattgcaggtctgggatacggcactttgatgccagcagtgcagtccatcgctgttggtgtagtagacaaaaccgaattcggtacggccttctccactttgttcctgtttgtggacttaggttttggctttggacctattatcctgggagcagtttctgcggcaattggtttcggacctatgtatgcagcactggcaggtgtgggtgtgattgccggaatcttctacctgttcacacacgctcgcaccgatcgagctaagaatggctttgttaaacacccagagcctgtcgctttagttagctag

SEQ ID NO: 135 - protein, 406 aa, synthetic construct
  source 1..406: note = C. gl 13032 F347S AA
MSVAEEGKLFTPTFVMGWFANLFQFLVFYFLITTMALYAIKEFQASEVEAGFASSSIVIGAVFSRFFSGYIIDRFGRRKIVLISVLVTTIACALYLPIESLPLLYANRFLHGVGYAFAATAIMAMVQELIPASRRSEGTGYLALGTTVSAALGPALALFVLGTFDYDMLFIVVLATSVISLIAVVFMYFKTSDPEPSGEPAKFSFKSIMNPKIIPIGIFILLICFAYSGVIAYINAFAEERDLITGAGLFFIAYAVSMFVMRSFLGKLQDRRGDNVVIYFGLFFFVISLTILSFATSNWHVVLSGVIAGLGYGTLMPAVQSIAVGVVDKTEFGTAFSTLFLFVDLGSGFGPIILGAVSAAIGFGPMYAALAGVGVIAGIFYLFTHARTDRAKNGFVKHPEPVALVS

SEQ ID NO: 136 - DNA, 1221 bp, synthetic construct
  source 1..1221: mol_type = other DNA; note = C. gl 13032 F347S NT
atgtccgtagctgaagaagggaaactttttacaccaacgtttgtcatgggatggtttgccaaccttttccagttcctggtgttctacttcctcatcaccaccatggctttgtacgccatcaaggaatttcaagcctctgaagtagaagctggcttcgcatccagctcaattgttatcggcgcagtcttttccaggtttttctccggctatattattgaccgttttggtcgacgcaagattgtgctcatctcagtcctagtcactaccattgcgtgtgccttgtaccttcccatcgaatcattgccattgctatacgcaaacaggttcctccacggtgttggatacgcttttgctgccaccgcgatcatggcaatggtccaggagctcattccagcgtcacgacgttccgaaggtactggttacctggcattgggcactaccgtttctgcagcacttggaccagccctagcactttttgtcctaggaacatttgattacgacatgctgtttatcgtggtcttggcaacctcggtcatctctttgatcgccgtcgtgttcatgtactttaagaccagcgaccctgagccttctggggaaccagccaagttcagcttcaaatctattatgaacccaaagatcatccccatcggcatctttatcttgcttatttgctttgcttactctggcgtcattgcctacatcaacgcatttgctgaagaacgcgatctgattacgggtgctggattgttcttcattgcctacgcagtatcaatgtttgtgatgcgcagcttccttggcaaactgcaggaccgtcgcggagacaacgtcgttatttactttggattgttcttcttcgttatttccttgacgattttgtcctttgccacttccaactggcacgttgtgttgtccggagtcattgcaggtctgggatacggcactttgatgccagcagtgcagtccatcgctgttggtgtagtagacaaaaccgaattcggtacggccttctccactttgttcctgtttgtggacttaggttccggctttggacctattatcctgggagcagtttctgcggcaattggtttcggacctatgtatgcagcactggcaggtgtgggtgtgattgccggaatcttctacctgttcacacacgctcgcaccgatcgagctaagaatggctttgttaaacacccagagcctgtcgctttagttagctag

SEQ ID NO: 137 - protein, 391 aa, synthetic construct
  source 1..391: note = C. gl 13869 I216T AA
MGWFANLFQFLVFYFLITTMALYAIKEFQASEVEAGFASSSIVIGAVFSRFFSGYIIDRFGRRKIVLISVLVTTIACALYLPIESLPLLYANRFLHGVGYAFAATAIMAMVQELIPASRRSEGTGYLALGTTVSAALGPALALFVLGTFDYDMLFIVVLATSIISLIAVVFMYFKTSDPEPSGEPAKFSFKSIMNPKIIPIGIFILLICFAYSGVTAYINAFAEERDLITGAGLFFIAYAVSMFVMRSFLGKLQDRRGDNVVIYFGLFFFVISLVILSFATSNWHVVLSGVIAGLGYGTLMPAVQSIAVGVVDKTEFGTAFSTLFLFVDLGFGFGPIILGAVSAAIGFGPMYAALAGVGVIAGIFYLFTHARTDRAKNGFVKHPEPVALVS

SEQ ID NO: 138 - DNA, 1176 bp, synthetic construct
  source 1..1176: mol_type = other DNA; note = C. gl 13869 I216T NT
atgggatggtttgccaacctgttccaattcttggtgttctacttcctcatcaccaccatggctttgtatgccatcaaggaatttcaggcctctgaagtagaagcaggatttgcatccagctcaattgttatcggcgcagtcttttccaggtttttctccggctatattattgaccgttttggtcgacgcaagattgtgctcatctcagtcctcgtcactaccattgcgtgtgccttgtaccttcccatcgaatcattgccattgctatacgcaaacaggttcctccacggtgttggatacgcttttgctgccaccgcgatcatggcaatggtccaggagctcattccagcgtcacgacgttccgaaggtactggttacctggcattgggcaccaccgtttctgcagcacttggaccagccctagcactttttgtcctaggaacatttgattacgacatgctgtttatcgtggtcttggcaacctccatcatctctttgattgccgtcgtattcatgtactttaagaccagcgaccctgagccttctggggaaccagccaagttcagcttcaaatctattatgaacccaaagatcatccccatcggcatctttatcttgcttatttgctttgcttactctggcgtcaccgcctacatcaacgcatttgctgaagaacgcgatctgattacgggtgctggattgttcttcattgcctacgcagtatcaatgtttgtgatgcgcagcttccttggcaaactgcaggaccgtcgcggagacaacgtcgttatttactttggattgttcttcttcgttatttccttggtgattttgtcctttgccacttccaactggcacgttgtgttgtccggggtcattgcaggtctgggatacggcactttgatgccagcagtgcagtccatcgctgttggtgtagtagacaaaaccgaattcggtacggccttctccactttgttcctgtttgtggacttaggttttggctttggacctattatcctgggagcggtttctgcggcaattggtttcggacctatgtatgcagcactggcaggtgtgggtgtgattgccggaatcttctacctgttcacacacgctcgcaccgatcgagctaagaatggctttgttaaacacccagagcctgtcgctttagttagctag

SEQ ID NO: 139 - protein, 391 aa, synthetic construct
  source 1..391: note = C. gl 13869 F332S AA
MGWFANLFQFLVFYFLITTMALYAIKEFQASEVEAGFASSSIVIGAVFSRFFSGYIIDRFGRRKIVLISVLVTTIACALYLPIESLPLLYANRFLHGVGYAFAATAIMAMVQELIPASRRSEGTGYLALGTTVSAALGPALALFVLGTFDYDMLFIVVLATSIISLIAVVFMYFKTSDPEPSGEPAKFSFKSIMNPKIIPIGIFILLICFAYSGVIAYINAFAEERDLITGAGLFFIAYAVSMFVMRSFLGKLQDRRGDNVVIYFGLFFFVISLVILSFATSNWHVVLSGVIAGLGYGTLMPAVQSIAVGVVDKTEFGTAFSTLFLFVDLGSGFGPIILGAVSAAIGFGPMYAALAGVGVIAGIFYLFTHARTDRAKNGFVKHPEPVALVS

SEQ ID NO: 140 - DNA, 1176 bp, synthetic construct
  source 1..1176: mol_type = other DNA; note = C. gl 13869 F332S NT
atgggatggtttgccaacctgttccaattcttggtgttctacttcctcatcaccaccatggctttgtatgccatcaaggaatttcaggcctctgaagtagaagcaggatttgcatccagctcaattgttatcggcgcagtcttttccaggtttttctccggctatattattgaccgttttggtcgacgcaagattgtgctcatctcagtcctcgtcactaccattgcgtgtgccttgtaccttcccatcgaatcattgccattgctatacgcaaacaggttcctccacggtgttggatacgcttttgctgccaccgcgatcatggcaatggtccaggagctcattccagcgtcacgacgttccgaaggtactggttacctggcattgggcaccaccgtttctgcagcacttggaccagccctagcactttttgtcctaggaacatttgattacgacatgctgtttatcgtggtcttggcaacctccatcatctctttgattgccgtcgtattcatgtactttaagaccagcgaccctgagccttctggggaaccagccaagttcagcttcaaatctattatgaacccaaagatcatccccatcggcatctttatcttgcttatttgctttgcttactctggcgtcattgcctacatcaacgcatttgctgaagaacgcgatctgattacgggtgctggattgttcttcattgcctacgcagtatcaatgtttgtgatgcgcagcttccttggcaaactgcaggaccgtcgcggagacaacgtcgttatttactttggattgttcttcttcgttatttccttggtgattttgtcctttgccacttccaactggcacgttgtgttgtccggggtcattgcaggtctgggatacggcactttgatgccagcagtgcagtccatcgctgttggtgtagtagacaaaaccgaattcggtacggccttctccactttgttcctgtttgtggacttaggttccggctttggacctattatcctgggagcggtttctgcggcaattggtttcggacctatgtatgcagcactggcaggtgtgggtgtgattgccggaatcttctacctgttcacacacgctcgcaccgatcgagctaagaatggctttgttaaacacccagagcctgtcgctttagttagctag

SEQ ID NO: 141 - DNA, 60 bp, synthetic construct
  source 1..60: mol_type = other DNA; note = xmpE CF
agctatgaccatgattacgccaagcttggtaccgagctcgttatcatggggtgggtcgcc

SEQ ID NO: 142 - DNA, 60 bp, synthetic construct
  source 1..60: mol_type = other DNA; note = xmpE CR
tgaattgtaatacgactcactatagggcgaattgggccctttattgagccagaaccatgg

SEQ ID NO: 143 - DNA, 20 bp, synthetic construct
  source 1..20: mol_type = other DNA; note = xmpE seq F
ggaatccgctgtcatgatct

SEQ ID NO: 144 - DNA, 20 bp, synthetic construct
  source 1..20: mol_type = other DNA; note = xmpE seq R
tcgcagttcacgcactaaag

SEQ ID NO: 145 - DNA, 30 bp, synthetic construct
  source 1..30: mol_type = other DNA; note = pDCM2-xmpE(F354C)
cgttgacctcggctgcggcttcggcccagt

SEQ ID NO: 146 - DNA, 30 bp, synthetic construct
  source 1..30: mol_type = other DNA; note = pDCM2-xmpE(F354C)
actgggccgaagccgcagccgaggtcaacg

SEQ ID NO: 147 - DNA, 30 bp, synthetic construct
  source 1..30: mol_type = other DNA; note = pDCM2-xmpE(F354R)
cgttgacctcggcagaggcttcggcccagt

SEQ ID NO: 148 - DNA, 30 bp, synthetic construct
  source 1..30: mol_type = other DNA; note = pDCM2-xmpE(F354R)
actgggccgaagcctctgccgaggtcaacg

SEQ ID NO: 149 - DNA, 30 bp, synthetic construct
  source 1..30: mol_type = other DNA; note = pDCM2-xmpE(F354I)
cgttgacctcggcatcggcttcggcccagt

SEQ ID NO: 150 - DNA, 30 bp, synthetic construct
  source 1..30: mol_type = other DNA; note = pDCM2-xmpE(F354I)
actgggccgaagccgatgccgaggtcaacg

SEQ ID NO: 151 - DNA, 30 bp, synthetic construct
  source 1..30: mol_type = other DNA; note = pDCM2-xmpE(F354V)
cgttgacctcggcgtgggcttcggcccagt

SEQ ID NO: 152 - DNA, 30 bp, synthetic construct
  source 1..30: mol_type = other DNA; note = pDCM2-xmpE(F354V)
actgggccgaagcccacgccgaggtcaacg

SEQ ID NO: 153 - DNA, 30 bp, synthetic construct
  source 1..30: mol_type = other DNA; note = pDCM2-xmpE(F354D)
cgttgacctcggcgatggcttcggcccagt

SEQ ID NO: 154 - DNA, 30 bp, synthetic construct
  source 1..30: mol_type = other DNA; note = pDCM2-xmpE(F354D)
actgggccgaagccatcgccgaggtcaacg

SEQ ID NO: 155 - DNA, 30 bp, synthetic construct
  source 1..30: mol_type = other DNA; note = pDCM2-xmpE(F354G)
cgttgacctcggcggcggcttcggcccagt

SEQ ID NO: 156 - DNA, 30 bp, synthetic construct
  source 1..30: mol_type = other DNA; note = pDCM2-xmpE(F354G)
actgggccgaagccgccgccgaggtcaacg

SEQ ID NO: 157 - DNA, 30 bp, synthetic construct
  source 1..30: mol_type = other DNA; note = pDCM2-xmpE(F354P)
cgttgacctcggcccaggcttcggcccagt

SEQ ID NO: 158 - DNA, 30 bp, synthetic construct
  source 1..30: mol_type = other DNA; note = pDCM2-xmpE(F354P)
actgggccgaagcctgggccgaggtcaacg

SEQ ID NO: 159 - DNA, 30 bp, synthetic construct
  source 1..30: mol_type = other DNA; note = pDCM2-xmpE(F354A)
cgttgacctcggcgcaggcttcggcccagt

SEQ ID NO: 160 - DNA, 30 bp, synthetic construct
  source 1..30: mol_type = other DNA; note = pDCM2-xmpE(F354A)
actgggccgaagcctgcgccgaggtcaacg

SEQ ID NO: 161 - DNA, 30 bp, synthetic construct
  source 1..30: mol_type = other DNA; note = pDCM2-xmpE(F354E)
cgttgacctcggcgaaggcttcggcccagt

SEQ ID NO: 162 - DNA, 30 bp, synthetic construct
  source 1..30: mol_type = other DNA; note = pDCM2-xmpE(F354E)
actgggccgaagccttcgccgaggtcaacg

SEQ ID NO: 163 - DNA, 30 bp, synthetic construct
  source 1..30: mol_type = other DNA; note = pDCM2-xmpE(F354M)
cgttgacctcggcatgggcttcggcccagt

SEQ ID NO: 164 - DNA, 30 bp, synthetic construct
  source 1..30: mol_type = other DNA; note = pDCM2-xmpE(F354M)
actgggccgaagcccatgccgaggtcaacg

SEQ ID NO: 165 - DNA, 30 bp, synthetic construct
  source 1..30: mol_type = other DNA; note = pDCM2-xmpE(F354W)
cgttgacctcggctggggcttcggcccagt

SEQ ID NO: 166 - DNA, 30 bp, synthetic construct
  source 1..30: mol_type = other DNA; note = pDCM2-xmpE(F354W)
actgggccgaagccccagccgaggtcaacg

SEQ ID NO: 167 - DNA, 30 bp, synthetic construct
  source 1..30: mol_type = other DNA; note = pDCM2-xmpE(F354T)
cgttgacctcggcaccggcttcggcccagt

SEQ ID NO: 168 - DNA, 30 bp, synthetic construct
  source 1..30: mol_type = other DNA; note = pDCM2-xmpE(F354T)
actgggccgaagccggtgccgaggtcaacg

SEQ ID NO: 169 - DNA, 30 bp, synthetic construct
  source 1..30: mol_type = other DNA; note = pDCM2-xmpE(F354Q)
cgttgacctcggccagggcttcggcccagt

SEQ ID NO: 170 - DNA, 30 bp, synthetic construct
  source 1..30: mol_type = other DNA; note = pDCM2-xmpE(F354Q)
actgggccgaagccctggccgaggtcaacg

SEQ ID NO: 171 - DNA, 30 bp, synthetic construct
  source 1..30: mol_type = other DNA; note = pDCM2-xmpE(F354K)
cgttgacctcggcaagggcttcggcccagt

SEQ ID NO: 172 - DNA, 30 bp, synthetic construct
  source 1..30: mol_type = other DNA; note = pDCM2-xmpE(F354K)
actgggccgaagcccttgccgaggtcaacg

SEQ ID NO: 173 - DNA, 30 bp, synthetic construct
  source 1..30: mol_type = other DNA; note = pDCM2-xmpE(F354L)
cgttgacctcggcctgggcttcggcccagt

SEQ ID NO: 174 - DNA, 30 bp, synthetic construct
  source 1..30: mol_type = other DNA; note = pDCM2-xmpE(F354L)
actgggccgaagcccaggccgaggtcaacg

SEQ ID NO: 175 - DNA, 30 bp, synthetic construct
  source 1..30: mol_type = other DNA; note = pDCM2-xmpE(F354H)
cgttgacctcggccacggcttcggcccagt

SEQ ID NO: 176 - DNA, 30 bp, synthetic construct
  source 1..30: mol_type = other DNA; note = pDCM2-xmpE(F354H)
actgggccgaagccgtggccgaggtcaacg

SEQ ID NO: 177 - DNA, 33 bp, synthetic construct
  source 1..33: mol_type = other DNA; note = pDCM2-xmpE(I259F)
cgcaggcctattctttttcgcttacgccatctc

SEQ ID NO: 178 - DNA, 33 bp, synthetic construct
  source 1..33: mol_type = other DNA; note = pDCM2-xmpE(I259F)
gagatggcgtaagcgaaaaagaataggcctgcg

SEQ ID NO: 179 - DNA, 33 bp, synthetic construct
  source 1..33: mol_type = other DNA; note = pDCM2-xmpE(I259Y)
cgcaggcctattcttttacgcttacgccatctc

SEQ ID NO: 180 - DNA, 33 bp, synthetic construct
  source 1..33: mol_type = other DNA; note = pDCM2-xmpE(I259Y)
gagatggcgtaagcgtaaaagaataggcctgcg

SEQ ID NO: 181 - DNA, 33 bp, synthetic construct
  source 1..33: mol_type = other DNA; note = pDCM2-xmpE(I259C)
cgcaggcctattcttttgcgcttacgccatctc

SEQ ID NO: 182 - DNA, 33 bp, synthetic construct
  source 1..33: mol_type = other DNA; note = pDCM2-xmpE(I259C)
gagatggcgtaagcgcaaaagaataggcctgcg

SEQ ID NO: 183 - DNA, 33 bp, synthetic construct
  source 1..33: mol_type = other DNA; note = pDCM2-xmpE(I259L)
cgcaggcctattctttctggcttacgccatctc

SEQ ID NO: 184 - DNA, 33 bp, synthetic construct
  source 1..33: mol_type = other DNA; note = pDCM2-xmpE(I259L)
gagatggcgtaagccagaaagaataggcctgcg

SEQ ID NO: 185 - DNA, 33 bp, synthetic construct
  source 1..33: mol_type = other DNA; note = pDCM2-xmpE(I259H)
cgcaggcctattctttcacgcttacgccatctc

SEQ ID NO: 186 - DNA, 33 bp, synthetic construct
  source 1..33: mol_type = other DNA; note = pDCM2-xmpE(I259H)
gagatggcgtaagcgtgaaagaataggcctgcg

SEQ ID NO: 187 - DNA, 33 bp, synthetic construct
  source 1..33: mol_type = other DNA; note = pDCM2-xmpE(I259V)
cgcaggcctattctttgtggcttacgccatctc

SEQ ID NO: 188 - DNA, 33 bp, synthetic construct
  source 1..33: mol_type = other DNA; note = pDCM2-xmpE(I259V)
gagatggcgtaagccacaaagaataggcctgcg

SEQ ID NO: 189 - DNA, 33 bp, synthetic construct
  source 1..33: mol_type = other DNA; note = pDCM2-xmpE(I259D)
cgcaggcctattctttgatgcttacgccatctc

SEQ ID NO: 190 - DNA, 33 bp, synthetic construct
  source 1..33: mol_type = other DNA; note = pDCM2-xmpE(I259D)
gagatggcgtaagcatcaaagaataggcctgcg

SEQ ID NO: 191 - DNA, 33 bp, synthetic construct
  source 1..33: mol_type = other DNA; note = pDCM2-xmpE(I259G)
cgcaggcctattctttggcgcttacgccatctc

SEQ ID NO: 192 - DNA, 33 bp, synthetic construct
  source 1..33: mol_type = other DNA; note = pDCM2-xmpE(I259G)
gagatggcgtaagcgccaaagaataggcctgcg

SEQ ID NO: 193 - DNA, 33 bp, synthetic construct
  source 1..33: mol_type = other DNA; note = pDCM2-xmpE(I259P)
cgcaggcctattctttccagcttacgccatctc

SEQ ID NO: 194 - DNA, 33 bp, synthetic construct
  source 1..33: mol_type = other DNA; note = pDCM2-xmpE(I259P)
gagatggcgtaagctggaaagaataggcctgcg

SEQ ID NO: 195 - DNA, 33 bp, synthetic construct
  source 1..33: mol_type = other DNA; note = pDCM2-xmpE(I259A)
cgcaggcctattctttgcagcttacgccatctc

SEQ ID NO: 196 - DNA, 33 bp, synthetic construct
  source 1..33: mol_type = other DNA; note = pDCM2-xmpE(I259A)
gagatggcgtaagctgcaaagaataggcctgcg

SEQ ID NO: 197 - DNA, 33 bp, synthetic construct
  source 1..33: mol_type = other DNA; note = pDCM2-xmpE(I259E)
cgcaggcctattctttgaagcttacgccatctc

SEQ ID NO: 198 - DNA, 33 bp, synthetic construct
  source 1..33: mol_type = other DNA; note = pDCM2-xmpE(I259E)
gagatggcgtaagcttcaaagaataggcctgcg

SEQ ID NO: 199 - DNA, 33 bp, synthetic construct
  source 1..33: mol_type = other DNA; note = pDCM2-xmpE(I259M)
cgcaggcctattctttatggcttacgccatctc

SEQ ID NO: 200 - DNA, 33 bp, synthetic construct
  source 1..33: mol_type = other DNA; note = pDCM2-xmpE(I259M)
gagatggcgtaagccataaagaataggcctgcg

SEQ ID NO: 201 - DNA, 33 bp, synthetic construct
  source 1..33: mol_type = other DNA; note = pDCM2-xmpE(I259W)
cgcaggcctattcttttgggcttacgccatctc

SEQ ID NO: 202 - DNA, 33 bp, synthetic construct
  source 1..33: mol_type = other DNA; note = pDCM2-xmpE(I259W)
gagatggcgtaagcccaaaagaataggcctgcg

SEQ ID NO: 203 - DNA, 33 bp, synthetic construct
  source 1..33: mol_type = other DNA; note = pDCM2-xmpE(I259Q)
cgcaggcctattctttcaggcttacgccatctc

SEQ ID NO: 204 - DNA, 33 bp, synthetic construct
  source 1..33: mol_type = other DNA; note = pDCM2-xmpE(I259Q)
gagatggcgtaagcctgaaagaataggcctgcg

SEQ ID NO: 205 - DNA, 33 bp, synthetic construct
  source 1..33: mol_type = other DNA; note = pDCM2-xmpE(I259K)
cgcaggcctattctttaaggcttacgccatctc

SEQ ID NO: 206 - DNA, 33 bp, synthetic construct
  source 1..33: mol_type = other DNA; note = pDCM2-xmpE(I259K)
gagatggcgtaagccttaaagaataggcctgcg

SEQ ID NO: 207 - DNA, 33 bp, synthetic construct
  source 1..33: mol_type = other DNA; note = pDCM2-xmpE(I259R)
cgcaggcctattctttagagcttacgccatctc

SEQ ID NO: 208 - DNA, 33 bp, synthetic construct
  source 1..33: mol_type = other DNA; note = pDCM2-xmpE(I259R)
gagatggcgtaagctctaaagaataggcctgcg

SEQ ID NO: 209 - DNA, 33 bp, synthetic construct
  source 1..33: mol_type = other DNA; note = pDCM2-xmpE(I259N)
cgcaggcctattctttaacgcttacgccatctc

SEQ ID NO: 210 - DNA, 33 bp, synthetic construct
  source 1..33: mol_type = other DNA; note = pDCM2-xmpE(I259N)
gagatggcgtaagcgttaaagaataggcctgcg

SEQ ID NO: 211 - DNA, 33 bp, synthetic construct
  source 1..33: mol_type = other DNA; note = pDCM2-xmpE(V310F)
caactggcatgtcgttttcgctggcgtgctagc

SEQ ID NO: 212 - DNA, 33 bp, synthetic construct
  source 1..33: mol_type = other DNA; note = pDCM2-xmpE(V310F)
gctagcacgccagcgaaaacgacatgccagttg

SEQ ID NO: 213 - DNA, 33 bp, synthetic construct
  source 1..33: mol_type = other DNA; note = pDCM2-xmpE(V310C)
caactggcatgtcgtttgcgctggcgtgctagc

SEQ ID NO: 214 - DNA, 33 bp, synthetic construct
  source 1..33: mol_type = other DNA; note = pDCM2-xmpE(V310C)
gctagcacgccagcgcaaacgacatgccagttg

SEQ ID NO: 215 - DNA, 33 bp, synthetic construct
  source 1..33: mol_type = other DNA; note = pDCM2-xmpE(V310L)
caactggcatgtcgttctggctggcgtgctagc

SEQ ID NO: 216 - DNA, 33 bp, synthetic construct
  source 1..33: mol_type = other DNA; note = pDCM2-xmpE(V310L)
gctagcacgccagccagaacgacatgccagttg

SEQ ID NO: 217 - DNA, 33 bp, synthetic construct
  source 1..33: mol_type = other DNA; note = pDCM2-xmpE(V310H)
caactggcatgtcgttcacgctggcgtgctagc

SEQ ID NO: 218 - DNA, 33 bp, synthetic construct
  source 1..33: mol_type = other DNA; note = pDCM2-xmpE(V310H)
gctagcacgccagcgtgaacgacatgccagttg

SEQ ID NO: 219 - DNA, 33 bp, synthetic construct
  source 1..33: mol_type = other DNA; note = pDCM2-xmpE(V310R)
caactggcatgtcgttagagctggcgtgctagc

SEQ ID NO: 220 - DNA, 33 bp, synthetic construct
  source 1..33: mol_type = other DNA; note = pDCM2-xmpE(V310R)
gctagcacgccagctctaacgacatgccagttg

SEQ ID NO: 221 - DNA, 33 bp, synthetic construct
  source 1..33: mol_type = other DNA; note = pDCM2-xmpE(V310I)
caactggcatgtcgttatcgctggcgtgctagc

SEQ ID NO: 222 - DNA, 33 bp, synthetic construct
  source 1..33: mol_type = other DNA; note = pDCM2-xmpE(V310I)
gctagcacgccagcgataacgacatgccagttg

SEQ ID NO: 223 - DNA, 33 bp, synthetic construct
  source 1..33: mol_type = other DNA; note = pDCM2-xmpE(V310N)
caactggcatgtcgttaacgctggcgtgctagc

SEQ ID NO: 224 - DNA, 33 bp, synthetic construct
  source 1..33: mol_type = other DNA; note = pDCM2-xmpE(V310N)
gctagcacgccagcgttaacgacatgccagttg

SEQ ID NO: 225 - DNA, 33 bp, synthetic construct
  source 1..33: mol_type = other DNA; note = pDCM2-xmpE(V310D)
caactggcatgtcgttgatgctggcgtgctagc

SEQ ID NO: 226 - DNA, 33 bp, synthetic construct
  source 1..33: mol_type = other DNA; note = pDCM2-xmpE(V310D)
gctagcacgccagcatcaacgacatgccagttg

SEQ ID NO: 227 - DNA, 33 bp, synthetic construct
  source 1..33: mol_type = other DNA; note = pDCM2-xmpE(V310G)
caactggcatgtcgttggcgctggcgtgctagc

SEQ ID NO: 228 - DNA, 33 bp, synthetic construct
  source 1..33: mol_type = other DNA; note = pDCM2-xmpE(V310G)
gctagcacgccagcgccaacgacatgccagttg

SEQ ID NO: 229 - DNA, 33 bp, synthetic construct
  source 1..33: mol_type = other DNA; note = pDCM2-xmpE(V310P)
caactggcatgtcgttccagctggcgtgctagc

SEQ ID NO: 230 - DNA, 33 bp, synthetic construct
  source 1..33: mol_type = other DNA; note = pDCM2-xmpE(V310P)
gctagcacgccagctggaacgacatgccagttg

SEQ ID NO: 231 - DNA, 33 bp, synthetic construct
  source 1..33: mol_type = other DNA; note = pDCM2-xmpE(V310E)
caactggcatgtcgttgaagctggcgtgctagc

SEQ ID NO: 232 - DNA, 33 bp, synthetic construct
  source 1..33: mol_type = other DNA; note = pDCM2-xmpE(V310E)
gctagcacgccagcttcaacgacatgccagttg

SEQ ID NO: 233 - DNA, 33 bp, synthetic construct
  source 1..33: mol_type = other DNA; note = pDCM2-xmpE(V310M)
caactggcatgtcgttatggctggcgtgctagc

SEQ ID NO: 234 - DNA, 33 bp, synthetic construct
  source 1..33: mol_type = other DNA; note = pDCM2-xmpE(V310M)
gctagcacgccagccataacgacatgccagttg

SEQ ID NO: 235 - DNA, 33 bp, synthetic construct
  source 1..33: mol_type = other DNA; note = pDCM2-xmpE(V310W)
caactggcatgtcgtttgggctggcgtgctagc

SEQ ID NO: 236 - DNA, 33 bp, synthetic construct
  source 1..33: mol_type = other DNA; note = pDCM2-xmpE(V310W)
gctagcacgccagcccaaacgacatgccagttg

SEQ ID NO: 237 - DNA, 33 bp, synthetic construct
  source 1..33: mol_type = other DNA; note = pDCM2-xmpE(V310S)
caactggcatgtcgtttccgctggcgtgctagc

SEQ ID NO: 238 - DNA, 33 bp, synthetic construct
  source 1..33: mol_type = other DNA; note = pDCM2-xmpE(V310S)
gctagcacgccagcggaaacgacatgccagttg

SEQ ID NO: 239 - DNA, 33 bp, synthetic construct
  source 1..33: mol_type = other DNA; note = pDCM2-xmpE(V310T)
caactggcatgtcgttaccgctggcgtgctagc

SEQ ID NO: 240 - DNA, 33 bp, synthetic construct
  source 1..33: mol_type = other DNA; note = pDCM2-xmpE(V310T)
gctagcacgccagcggtaacgacatgccagttg

SEQ ID NO: 241 - DNA, 33 bp, synthetic construct
  source 1..33: mol_type = other DNA; note = pDCM2-xmpE(V310Q)
caactggcatgtcgttcaggctggcgtgctagc

SEQ ID NO: 242 - DNA, 33 bp, synthetic construct
  source 1..33: mol_type = other DNA; note = pDCM2-xmpE(V310Q)
gctagcacgccagcctgaacgacatgccagttg

SEQ ID NO: 243 - DNA, 33 bp, synthetic construct
  source 1..33: mol_type = other DNA; note = pDCM2-xmpE(V310K)
caactggcatgtcgttaaggctggcgtgctagc

SEQ ID NO: 244 - DNA, 33 bp, synthetic construct
  source 1..33: mol_type = other DNA; note = pDCM2-xmpE(V310K)
gctagcacgccagccttaacgacatgccagttg

SEQ ID NO: 245 - DNA, 33 bp, synthetic construct
  source 1..33: mol_type = other DNA; note = pDCM2-xmpE(V310Y)
caactggcatgtcgtttacgctggcgtgctagc

SEQ ID NO: 246 - DNA, 33 bp, synthetic construct
  source 1..33: mol_type = other DNA; note = pDCM2-xmpE(V310Y)
gctagcacgccagcgtaaacgacatgccagttg

SEQ ID NO: 247 - DNA, 41 bp, synthetic construct
  source 1..41: mol_type = other DNA; note = pDC-xmpE-LA-F
agctcggtacccggggatcctcgcatcgggtaggatctgca

SEQ ID NO: 248 - DNA, 40 bp, synthetic construct
  source 1..40: mol_type = other DNA; note = xmpE-LA-(Cgl13032)-R
ccttcttcagctacggacatgattctccttactgcagtta

SEQ ID NO: 249 - DNA, 40 bp, synthetic construct
  source 1..40: mol_type = other DNA; note = (xmpE-LA)-Cgl13032-F
taactgcagtaaggagaatcatgtccgtagctgaagaagg

SEQ ID NO: 250 - DNA, 40 bp, synthetic construct
  source 1..40: mol_type = other DNA; note = Cgl13032-(xmpE-RA)-R
tcccttggctcaaatatttactagctaactaaagcgacag

SEQ ID NO: 251 - DNA, 40 bp, synthetic construct
  source 1..40: mol_type = other DNA; note = (Cgl13032)-xmpE-RA-F
ctgtcgctttagttagctagtaaatatttgagccaaggga

SEQ ID NO: 252 - DNA, 42 bp, synthetic construct
  source 1..42: mol_type = other DNA; note = pDC-xmpE-RA-R
tgcatgcctgcaggtcgactatgaatgcccacaggaacagca

SEQ ID NO: 253 - DNA, 40 bp, synthetic construct
  source 1..40: mol_type = other DNA; note = xmpE-LA-(Cgl13869)-R
aggttggcaaaccatcccatgattctccttactgcagtta

SEQ ID NO: 254 - DNA, 40 bp, synthetic construct
  source 1..40: mol_type = other DNA; note = (xmpE-LA)-Cgl13869-F
taactgcagtaaggagaatcatgggatggtttgccaacct

SEQ ID NO: 255 - DNA, 40 bp, synthetic construct; identical to SEQ ID NO: 250
  source 1..40: mol_type = other DNA; note = Cgl138692-(xmpE-RA)-R

SEQ ID NO: 256 - DNA, 40 bp, synthetic construct; identical to SEQ ID NO: 251
  source 1..40: mol_type = other DNA; note = (Cgl13869)-xmpE-RA-F

SEQ ID NO: 257 - DNA, 36 bp, synthetic construct
  source 1..36: mol_type = other DNA; note = C. gl 13032 I231T/C. gl 13869 I216T
gcttactctggcgtcaccgcctacatcaacgcattt

SEQ ID NO: 258 - DNA, 36 bp, synthetic construct
  source 1..36: mol_type = other DNA; note = C. gl 13032 I231T/C. gl 13869 I216T
aaatgcgttgatgtaggcggtgacgccagagtaagc

SEQ ID NO: 259 - DNA, 34 bp, synthetic construct
  source 1..34: mol_type = other DNA; note = C. gl 13032 F347S/C. gl 13869 F332S
gtttgtggacttaggttccggctttggacctatt

SEQ ID NO: 260 - DNA, 34 bp, synthetic construct
  source 1..34: mol_type = other DNA; note = C. gl 13032 F347S/C. gl 13869 F332S
aataggtccaaagccggaacctaagtccacaaac